European Patent Specification EP 3 775 274 B1, published December 20, 2023. Title: Detection method of somatic genetic anomalies, combination of capture probes and kit of detection. Applicant: Université de Bourgogne Centre Georges-François Leclerc. The sequence listing filed with the application follows.

SEQUENCE LISTING (1229 sequences)

SEQ ID NO: 1 - DNA, 120 bp, Artificial Sequence
  ALK-E25
cagtctttactcacctgtagatgtctcgggccatcccgaagtctccaatcttggccactcttccagggcctggacaggtcaagaggcagtttctggcagcaatgtctctgggaagaaagg

SEQ ID NO: 2 - DNA, 120 bp, Artificial Sequence
  ALK-E24
ctttgactcaccggtggatgaagtggttttcctccaaatactgacagccacaggcaatgtcccgagccacgtgcagaaggtccagcatggccagggaggagggctggctctgtggggaga

SEQ ID NO: 3 - DNA, 120 bp, Artificial Sequence
  ALK-E23
acaactgcagcaaagactggttctcactcaccgggcgagggcgggtctctcggaggaaggacttgaggtctccccccgccatgagctccagcaggatgaaccggggcagggattgcaggc

SEQ ID NO: 4 - DNA, 120 bp, Artificial Sequence
  ALK-E23
cactcaccgggcgagggcgggtctctcggaggaaggacttgaggtctccccccgccatgagctccagcaggatgaaccggggcagggattgcaggctcaccccaatgcagcgaacaatgt

SEQ ID NO: 5 - DNA, 120 bp, Artificial Sequence
  EGFR-E18
gtcccccccagcttgtggagcctcttacacccagtggagaagctcccaaccaagctctcttgaggatcttgaaggaaactgaattcaaaaagatcaaagtgctgggctccggtgcgttcg

SEQ ID NO: 6 - DNA, 120 bp, Artificial Sequence
  EGFR-E18
ttacacccagtggagaagctcccaaccaagctctcttgaggatcttgaaggaaactgaattcaaaaagatcaaagtgctgggctccggtgcgttcggcacggtgtataaggtaaggtccc

SEQ ID NO: 7 - DNA, 120 bp, Artificial Sequence
  EGFR-E19
ctctgtcatagggactctggatcccagaaggtgagaaagttaaaattcccgtcgctatcaaggaattaagagaagcaacatctccgaaagccaacaaggaaatcctcgatgtgagtttct

SEQ ID NO: 8 - DNA, 120 bp, Artificial Sequence
  EGFR-E20
caggaagcctacgtgatggccagcgtggacaacccccacgtgtgccgcctgctgggcatctgcctcacctccaccgtgcagctcatcacgcagctcatgcccttcggctgcctcctggac

SEQ ID NO: 9 - DNA, 120 bp, Artificial Sequence
  EGFR-E20
accgtgcagctcatcacgcagctcatgcccttcggctgcctcctggactatgtccgggaacacaaagacaatattggctcccagtacctgctcaactggtgtgtgcagatcgcaaaggta

SEQ ID NO: 10 - DNA, 120 bp, Artificial Sequence
  EGFR-E21
tttcagggcatgaactacttggaggaccgtcgcttggtgcaccgcgacctggcagccaggaacgtactggtgaaaacaccgcagcatgtcaagatcacagattttgggctggccaaactg

SEQ ID NO: 11 - DNA, 120 bp, Artificial Sequence
  EGFR-E21
ctggcagccaggaacgtactggtgaaaacaccgcagcatgtcaagatcacagattttgggctggccaaactgctgggtgcggaagagaaagaataccatgcagaaggaggcaaagtaagg

SEQ ID NO: 12 - DNA, 120 bp, Artificial Sequence
  MET-E14
ctgtcttatatgtagtccataaaacccatgagttctgggcactgggtcaaagtctcctggggcccatgatagccgtctttaacaagctctttctttctctctgttttaagatctgggcag

SEQ ID NO: 13 - DNA, 120 bp, Artificial Sequence
  MET-E14
ttttccagaaggtatatttcagtttattgttctgagaaatacctatacatatacctcagtgggttgtgacattgttgtttatttttggttttgcatttatatttttataaaaacctaaag

SEQ ID NO: 14 - DNA, 120 bp, Artificial Sequence
  MET-E17
ctcaggaatcactgacataggagaagtttcccaatttctgaccgagggaatcatcatgaaagattttagtcatcccaatgtcctctcgctcctgggaatctgcctgcgaagtgaagggtc

SEQ ID NO: 15 - DNA, 120 bp, Artificial Sequence
  MET-E17
tcccaatgtcctctcgctcctgggaatctgcctgcgaagtgaagggtctccgctggtggtcctaccatacatgaaacatggagatcttcgaaatttcattcgaaatgagactcatgtaag

SEQ ID NO: 16 - DNA, 120 bp, Artificial Sequence
  MET-E18
actctctttgactgcagaatccaactgtaaaagatcttattggctttggtcttcaagtagccaaaggcatgaaatatcttgcaagcaaaaagtttgtccacagagacttggctgcaagaa

SEQ ID NO: 17 - DNA, 120 bp, Artificial Sequence
  MET-E18
ctgtaaaagatcttattggctttggtcttcaagtagccaaaggcatgaaatatcttgcaagcaaaaagtttgtccacagagacttggctgcaagaaactgtatgtaagtatcagaatctc

SEQ ID NO: 18 - DNA, 120 bp, Artificial Sequence
  MET-E19
gtcctttctgtaggctggatgaaaaattcacagtcaaggttgctgattttggtcttgccagagacatgtatgataaagaatactatagtgtacacaacaaaacaggtgcaaagctgccag

SEQ ID NO: 19 - DNA, 120 bp, Artificial Sequence
  gene MET-E19
ataaagaatactatagtgtacacaacaaaacaggtgcaaagctgccagtgaagtggatggctttggaaagtctgcaaactcaaaagtttaccaccaagtcagatgtggtaatgtattggt

SEQ ID NO: 20 - DNA, 120 bp, Artificial Sequence
  MET-E20
ctagtggtcctttggcgtgctcctctgggagctgatgacaagaggagccccaccttatcctgacgtaaacacctttgatataactgtttacttgttgcaagggagaagactcctacaacc

SEQ ID NO: 21 - DNA, 120 bp, Artificial Sequence
  BRAF-E15
tggatccagacaactgttcaaactgatgggacccactccatcgagatttcactgtagctagaccaaaatcacctatttttactgtgaggtcttcatgaagaaatatatctgaggtgtagt

SEQ ID NO: 22 - DNA, 120 bp, Artificial Sequence
  HER2-E20
caggaagcatacgtgatggctggtgtgggctccccatatgtctcccgccttctgggcatctgcctgacatccacggtgcagctggtgacacagcttatgccctatggctgcctcttagac

SEQ ID NO: 23 - DNA, 120 bp, Artificial Sequence
  HER2-E20
acggtgcagctggtgacacagcttatgccctatggctgcctcttagaccatgtccgggaaaaccgcggacgcctgggctcccaggacctgctgaactggtgtatgcagattgccaaggta

SEQ ID NO: 24 - DNA, 120 bp, Artificial Sequence
  PDGFRA-E12
ttatagaaaccgaggtatgaaattcgctggagggtcattgaatcaatcagcccagatggacatgaatatatttatgtggacccgatgcagctgccttatgactcaagatgggagtttcca

SEQ ID NO: 25 - DNA, 120 bp, Artificial Sequence
  PDGFRA-E12
cgctggagggtcattgaatcaatcagcccagatggacatgaatatatttatgtggacccgatgcagctgccttatgactcaagatgggagtttccaagagatggactagtgcttggtaag

SEQ ID NO: 26 - DNA, 120 bp, Artificial Sequence
  PDGFRA-E14
aacagccacggccagatccagtgaaaaacaagctctcatgtctgaactgaagataatgactcacctggggccacatttgaacattgtaaacttgctgggagcctgcaccaagtcaggtgg

SEQ ID NO: 27 - DNA, 120 bp, Artificial Sequence
  PDGFRA-E18
tttccatgcagtgtgtccaccgtgatctggctgctcgcaacgtcctcctggcacaaggaaaaattgtgaagatctgtgactttggcctggccagagacatcatgcatgattcgaactatg

SEQ ID NO: 28 - DNA, 120 bp, Artificial Sequence
  PDGFRA-E18
atctggctgctcgcaacgtcctcctggcacaaggaaaaattgtgaagatctgtgactttggcctggccagagacatcatgcatgattcgaactatgtgtcgaaaggcagtgtacgtcctc

SEQ ID NO: 29 - DNA, 120 bp, Artificial Sequence
  KIT-E9
cttccctttagatgctctgcttctgtactgccagtggatgtgcagacactaaactcatctgggccaccgtttggaaagctagtggttcagagttctatagattctagtgcattcaagcac

SEQ ID NO: 30 - DNA, 120 bp, Artificial Sequence
  KIT-E9
atagattctagtgcattcaagcacaatggcacggttgaatgtaaggcttacaacgatgtgggcaagacttctgcctattttaactttgcatttaaaggtaacaacaaaggtatatttctt

SEQ ID NO: 31 - DNA, 120 bp, Artificial Sequence
  KIT-E11
tccccacagaaacccatgtatgaagtacagtggaaggttgttgaggagataaatggaaacaattatgtttacatagacccaacacaacttccttatgatcacaaatgggagtttcccaga

SEQ ID NO: 32 - DNA, 120 bp, Artificial Sequence
  KIT-E11
gtacagtggaaggttgttgaggagataaatggaaacaattatgtttacatagacccaacacaacttccttatgatcacaaatgggagtttcccagaaacaggctgagttttggtcagtat

SEQ ID NO: 33 - DNA, 120 bp, Artificial Sequence
  KIT-E13
tttagcgagtgcccatttgacagaacgggaagccctcatgtctgaactcaaagtcctgagttaccttggtaatcacatgaatattgtgaatctacttggagcctgcaccattggaggtaa

SEQ ID NO: 34 - DNA, 120 bp, Artificial Sequence
  KIT-E14
ctatatatctcaccttctttctaaccttttcttatgtgcttttagggcccaccctggtcattacagaatattgttgctatggtgatcttttgaattttttgagaagaaaacgtgattcat

SEQ ID NO: 35 - DNA, 120 bp, Artificial Sequence
  KIT-E14
ttatttgttcaaagcaggaagatcatgcagaagctgcactttataagaatcttctgcattcaaaggagtcttcctggtaagactgatttacataaatagttagctgttgacaggcagttc

SEQ ID NO: 36 - DNA, 120 bp, Artificial Sequence
  KIT-E17
caacctaatagtgtattcacagagacttggcagccagaaatatcctccttactcatggtcggatcacaaagatttgtgattttggtctagccagagacatcaagaatgattctaattatg

SEQ ID NO: 37 - DNA, 120 bp, Artificial Sequence
  KIT-E17
acttggcagccagaaatatcctccttactcatggtcggatcacaaagatttgtgattttggtctagccagagacatcaagaatgattctaattatgtggttaaaggaaacgtgagtaccc

SEQ ID NO: 38 - DNA, 120 bp, Artificial Sequence
  KRAS-E4
ttacctgtcttgtctttgctgatgtttcaataaaaggaattccataacttcttgctaagtcctgagcctgttttgtgtctactgttctagaaggcaaatcacatttatttcctactagga

SEQ ID NO: 39 - DNA, 120 bp, Artificial Sequence
  KRAS-E3
ggcaaatacacaaagaaagccctccccagtcctcatgtactggtccctcattgcactgtactcctcttgacctgctgtgtcgagaatatccaagagacaggtttctccatcaattactac

SEQ ID NO: 40 - DNA, 120 bp, Artificial Sequence
  KRAS-E2
acaagatttacctctattgttggatcatattcgtccacaaaatgattctgaattagctgtatcgtcaaggcactcttgcctacgccaccagctccaactaccacaagtttatattcagtc

SEQ ID NO: 41 - DNA, 120 bp, Artificial Sequence
  NRAS-E4
accatacctgtctggtcttggctgaggtttcaatgaatggaatcccgtaactcttggccagttcgtgggcttgttttgtatcaactgtccttgttggcaaatcacacttgtttcccacta

SEQ ID NO: 42 - DNA, 120 bp, Artificial Sequence
  NRAS-E3
ggcaaatacacagaggaagccttcgcctgtcctcatgtattggtctctcatggcactgtactcttcttgtccagctgtatccagtatgtccaacaaacaggtttcaccatctataaccac

SEQ ID NO: 43 - DNA, 120 bp, Artificial Sequence
  NRAS-E2
ggcctcacctctatggtgggatcatattcatctacaaagtggttctggattagctggattgtcagtgcgcttttcccaacaccacctgctccaaccaccaccagtttgtactcagtcatt

SEQ ID NO: 44 - DNA, 120 bp, Artificial Sequence
  MAP2K1-E2
gaagaagctggaggagctagagcttgatgagcagcagcgaaagcgccttgaggcctttcttacccagaagcagaaggtgggagaactgaaggatgacgactttgagaagatcagtgagct

SEQ ID NO: 45 - DNA, 120 bp, Artificial Sequence
  HER4-E10
cagtttaaaaaattacctgttatctctctgactgtccgaaagacgttcagtttctctgggtctatggcttcaattgcattgtaagggtccctagaaaatcaagaagagatgtagccaaat

SEQ ID NO: 46 - DNA, 120 bp, Artificial Sequence
  HER4-E12
gtacttactacaattttcagcttttctgttgtcccggattactattctctggttgattgtgctgaagagtgttgtccagttaatggtatgataataacacaggttgctgttgtcagtaat

SEQ ID NO: 47 - DNA, 120 bp, Artificial Sequence
  HER4-E12
acacaggttgctgttgtcagtaatatagatgtttcctgcgctgatttccttcagggactggaactgtagagaggtgatgccctgttgcttgaggataagcaaggacaggccactaaggag

SEQ ID NO: 48 - DNA, 120 bp, Artificial Sequence
  TP53-E4
gggggctggtgcaggggccgccggtgtaggagctgctggtgcaggggccacggggggagcagcctctggcattctgggagcttcatctggacctgggtcttcagtgaaccattgttcaat

SEQ ID NO: 49 - DNA, 120 bp, Artificial Sequence
  KDR-E11
taacttcaattttatttcctccctggaagtcctccacacttctccattcttcacaagggtatgggtttgtcactgagacagcttggctataagaaagagataacagcgcatattatgatt

SEQ ID NO: 50 - DNA, 120 bp, Artificial Sequence
  SLC28A1
tgtggctgtctctggacacctcccagcggcctgagcaactggtgtccttcgcaggaatctgcgtgttcgtcgctctcctctttgcctgctcaaagcatcattgcgcagtgagtgctagtt

SEQ ID NO: 51 - DNA, 120 bp, Artificial Sequence
  EIF1AY
ctcctcagagtatgctcaggtaatcaaaatgttgggaaatggacgattggaagcattgtgttttgatggtgtaaagaggttatgccatatcagagggaaattgagaaaaaaggtaggtgt

SEQ ID NO: 52 - DNA, 120 bp, Artificial Sequence
  EIF1AY
ttagcaaagttttaactatgggattatttttaacaaacaattgtgttttctttttcttaaagacaaacacaatgcatacttactgccgaaagcttgacaagattaaaataagtccctcat

SEQ ID NO: 53 - DNA, 120 bp, Artificial Sequence
  EIF1AY
tatttttaacaaacaattgtgttttctttttcttaaagacaaacacaatgcatacttactgccgaaagcttgacaagattaaaataagtccctcatgacaccatcaaagagaatatgcac

SEQ ID NO: 54 - DNA, 120 bp, Artificial Sequence
  EIF1AY
tctttttcttaaagacaaacacaatgcatacttactgccgaaagcttgacaagattaaaataagtccctcatgacaccatcaaagagaatatgcactgttgtaaagcctgagtattttac

SEQ ID NO: 55 - DNA, 120 bp, Artificial Sequence
  EIF1AY
tgcatacttactgccgaaagcttgacaagattaaaataagtccctcatgacaccatcaaagagaatatgcactgttgtaaagcctgagtattttacttggcagctattttcattatttat

SEQ ID NO: 56 - DNA, 120 bp, Artificial Sequence
  EIF1AY
acaagattaaaataagtccctcatgacaccatcaaagagaatatgcactgttgtaaagcctgagtattttacttggcagctattttcattatttatcatattgcattttatgaaaagatt

SEQ ID NO: 57 - DNA, 120 bp, Artificial Sequence
  EIF1AY
gacaccatcaaagagaatatgcactgttgtaaagcctgagtattttacttggcagctattttcattatttatcatattgcattttatgaaaagatttttatataaacatgaagatcttga

SEQ ID NO: 58 - DNA, 120 bp, Artificial Sequence
  EIF1AY
tgttgtaaagcctgagtattttacttggcagctattttcattatttatcatattgcattttatgaaaagatttttatataaacatgaagatcttgatgaaattattggcatttcaggaag

SEQ ID NO: 59 - DNA, 120 bp, Artificial Sequence
  EIF1AY
ttggcagctattttcattatttatcatattgcattttatgaaaagatttttatataaacatgaagatcttgatgaaattattggcatttcaggaagtgctgaaatgttattggaagtgat

SEQ ID NO: 60 - DNA, 120 bp, Artificial Sequence
  EIF1AY
catattgcattttatgaaaagatttttatataaacatgaagatcttgatgaaattattggcatttcaggaagtgctgaaatgttattggaagtgatgaaattattggcatttcaggaagt

SEQ ID NO: 61 - DNA, 120 bp, Artificial Sequence
  EIF1AY
tgcatcttagttcagtcggctcttagagtagtaaccgccagaaaggagtcggaagaggtctcacgaggctgtcatcaccgccatgcccaagaataaaggtactgctgtaagcctctggga

SEQ ID NO: 62 - DNA, 120 bp, Artificial Sequence
  EIF1AY
tcacgaggctgtcatcaccgccatgcccaagaataaaggtactgctgtaagcctctgggactatacctcggcttgctctgccagtaaccccgacgcctgttccaggccgcagtgactgtt

SEQ ID NO: 63 - DNA, 120 bp, Artificial Sequence
  EIF1AY
tatgtagatttttacattaattttttatctactcttttaattaattaggtaaaggaggtaaaaacaggcgcaggggtaaaaatgagaatgaatctgaaaaaagagagttggtgtttaaag

SEQ ID NO: 64 - DNA, 120 bp, Artificial Sequence
  EIF1AY
tttcagtcattacattttaacaaatgtggaccaagatctcaacctttttttttatctcctctcctcagagtatgctcaggtaatcaaaatgttgggaaatggacgattggaagcattgtg

SEQ ID NO: 65 - DNA, 120 bp, Artificial Sequence
  EIF1AY
ttttgatggtgtaaagaggttatgccatatcagagggaaattgagaaaaaaggtaggtgtgtaggttacttttcaataaaaatttgccgcaaaaaatgtctctgctttaaatacatggtc

SEQ ID NO: 66 - DNA, 120 bp, Artificial Sequence
  EIF1AY
tttttatttttaaaataatctgcagtaaatttcttacaggtttggataaatacatcagacattatattggttggtctacgggactatcaggtaaaaataacatttaaagttgtggtatgt

SEQ ID NO: 67 - DNA, 120 bp, Artificial Sequence
  EIF1AY
attatattggttggtctacgggactatcaggtaaaaataacatttaaagttgtggtatgtctgtgtttaagcagttgttaatgtttggaaggtaactatactagcatctttgacccattc

SEQ ID NO: 68 - DNA, 120 bp, Artificial Sequence
  EIF1AY
gtgatattttggtataagacgttttgaaagttatttgtttatttctaaggataacaaagctgatgtaattttaaagtacaatgcagatgaagctagaagcctgaaggcatatggcgagct

SEQ ID NO: 69 - DNA, 120 bp, Artificial Sequence
  EIF1AY
tgatgtaattttaaagtacaatgcagatgaagctagaagcctgaaggcatatggcgagcttccagaacatggtaagatcaaaatgattttatctcctcattatttgatattaatgtttgt

SEQ ID NO: 70 - DNA, 120 bp, Artificial Sequence
  EIF1AY
gactacaggttatataatcagtatgtctgttattttacctttagctaaaatcaatgaaacagacacatttggtcctggagatgatgatgaaatccagtttgacgatattggagatgatga

SEQ ID NO: 71 - DNA, 120 bp, Artificial Sequence
  EIF1AY
agacacatttggtcctggagatgatgatgaaatccagtttgacgatattggagatgatgatgaagacattgatgatgtaagtaaataaacctaacaggtattttgttttatctatgcatt

SEQ ID NO: 72 - DNA, 120 bp, Artificial Sequence
  EIF1AY
cagtttaccactgggagtctttatatgcagtagaatgttgtaataagagttatttttctatggatctgatgttcttttcaattacagatctaaattgaaccaagtgtttttacatgacaa

SEQ ID NO: 73 - DNA, 120 bp, Artificial Sequence
  EIF1AY
tggatctgatgttcttttcaattacagatctaaattgaaccaagtgtttttacatgacaagttctctgaggatggttctacagttgggattttggccatcatcaaccaagaagagaaatt

SEQ ID NO: 74 - DNA, 120 bp, Artificial Sequence
  EIF1AY
aaaacaggcgcaggggtaaaaatgagaatgaatctgaaaaaagagagttggtgtttaaagaggatggacaaggtaagacttttcaacttaggcttctttcattaatatgttttgttgttg

SEQ ID NO: 75 - DNA, 120 bp, Artificial Sequence
  SLC28A1
gtgtgtgggtggggtgggggtgcaatgctgagggtaatggctttctgtctcttgcctgcaggggtctagctcttgctgctttcctgggcctggtcctgtggctgtctctggacacctccc

SEQ ID NO: 76 - DNA, 120 bp, Artificial Sequence
  SLC28A1
atgctgagggtaatggctttctgtctcttgcctgcaggggtctagctcttgctgctttcctgggcctggtcctgtggctgtctctggacacctcccagcggcctgagcaactggtgtcct

SEQ ID NO: 77 - DNA, 120 bp, Artificial Sequence
  SLC28A1
ctcttgcctgcaggggtctagctcttgctgctttcctgggcctggtcctgtggctgtctctggacacctcccagcggcctgagcaactggtgtccttcgcaggaatctgcgtgttcgtcg

SEQ ID NO: 78 - DNA, 120 bp, Artificial Sequence
  SLC28A1
ttgctgctttcctgggcctggtcctgtggctgtctctggacacctcccagcggcctgagcaactggtgtccttcgcaggaatctgcgtgttcgtcgctctcctctttgcctgctcaaagc

SEQ ID NO: 79 - DNA, 120 bp, Artificial Sequence
  SLC28A1
agcggcctgagcaactggtgtccttcgcaggaatctgcgtgttcgtcgctctcctctttgcctgctcaaagcatcattgcgcagtgagtgctagttgtggggcccagggctggaagtgtt

SEQ ID NO: 80 - DNA, 120 bp, Artificial Sequence
  SLC28A1
tcgcaggaatctgcgtgttcgtcgctctcctctttgcctgctcaaagcatcattgcgcagtgagtgctagttgtggggcccagggctggaagtgtttgcctctctcttctgcccctaggc

SEQ ID NO: 81 - DNA, 120 bp, Artificial Sequence
  SLC28A1
tgggcgctccctgatttgtctttcagctggaaggtctgggacatggagaacgacccctcgagacgaagagagtccatctctctcacacctgtggccaagggtctggagaacatgggggct

SEQ ID NO: 82 - DNA, 120 bp, Artificial Sequence
  SLC28A1
agacgaagagagtccatctctctcacacctgtggccaagggtctggagaacatgggggctgatttcttggaaagcctggtctgtacccttccccatcagtcatcctgacccctcagcctc

SEQ ID NO: 83 - DNA, 120 bp, Artificial Sequence
  SLC28A1
ggtgggtaaggggcaggccgacctgacggctccctgcgggctgtaggaggaaggccagctccctaggagtgacttgagccccgcagagatcaggagcagctggagcgaggcggcgccgaa

SEQ ID NO: 84 - DNA, 120 bp, Artificial Sequence
  SLC28A1
ccctaggagtgacttgagccccgcagagatcaggagcagctggagcgaggcggcgccgaagcccttctccagatggtaggtgatctctggagagacaagggcgggcctggggtggaggct

SEQ ID NO: 85 - DNA, 120 bp, Artificial Sequence
  SLC28A1
gggtctgctcatgcactcatggaccctgctggtcttgttcccaggaggaacctgcagccagccctgagagccagaagcttctgcagggagcacatgcagctgtttcgatggatcggcaca

SEQ ID NO: 86 - DNA, 120 bp, Artificial Sequence
  SLC28A1
gccctgagagccagaagcttctgcagggagcacatgcagctgtttcgatggatcggcacaggcctgctctgcactggtgagcctggggcccagcactacccaggacacaatgactcctgc

SEQ ID NO: 87 - DNA, 120 bp, Artificial Sequence
  SLC28A1
ttgacccctcctctgtctcatcccccagggctctctgccttcctgctggtggcctgcctcctggatttccagagggccctggctctgtttgtcctcacctgtgtggtcctcaccttcctg

SEQ ID NO: 88 - DNA, 120 bp, Artificial Sequence
  SLC28A1
ctggatttccagagggccctggctctgtttgtcctcacctgtgtggtcctcaccttcctgggccaccgcctgctgaaacggcttctggggccaaagctgaggaggtttctcaagcctcag

SEQ ID NO: 89 - DNA, 120 bp, Artificial Sequence
  SLC28A1
ggccaccgcctgctgaaacggcttctggggccaaagctgaggaggtttctcaagcctcagggccatccccgcctgctgctctggtttaagaggtgagtgagctcacagccccgaggcagg

SEQ ID NO: 90 - DNA, 120 bp, Artificial Sequence
  SLC28A1
cagtgggtggcttcaaacaaagcagcatctttgtggtgtttcaccagttcttagtcccagttacagcaggtgactgtggtggacgaaaactggactcaacagtttcctccattcagggat

SEQ ID NO: 91 - DNA, 120 bp, Artificial Sequence
  SLC28A1
ttacagcaggtgactgtggtggacgaaaactggactcaacagtttcctccattcagggatcccaggccatggagcaaggagggcccgaatcagtacctccctcagatcacctggacagtg

SEQ ID NO: 92 - DNA, 120 bp, Artificial Sequence
  SLC28A1
ggtgggggtgcaatgctgagggtaatggctttctgtctcttgcctgcaggggtctagctcttgctgctttcctgggcctggtcctgtggctgtctctggacacctcccagcggcctgagc

SEQ ID NO: 93 - DNA, 120 bp, Artificial Sequence; identical to SEQ ID NO: 78
  SLC28A1

SEQ ID NO: 94 - DNA, 120 bp, Artificial Sequence
  SLC28A1
aactggtgtccttcgcaggaatctgcgtgttcgtcgctctcctctttgcctgctcaaagcatcattgcgcagtgagtgctagttgtggggcccagggctggaagtgtttgcctctctctt

SEQ ID NO: 95 - DNA, 120 bp, Artificial Sequence
  SLC28A1
cacccggctccctgcccatccctcaaggaactgaactcagctttctgttgggtggggtggtaggtgtcctggagggccgtgtcttggggacttggactgcagtttgtacttggactcctc

SEQ ID NO: 96 - DNA, 120 bp, Artificial Sequence
  SLC28A1
taggtgtcctggagggccgtgtcttggggacttggactgcagtttgtacttggactcctcgtcatcagaacagaaccaggattcattgcgttcgagtggctgggcgagcagatccgggta

SEQ ID NO: 97 - DNA, 120 bp, Artificial Sequence
  SLC28A1
gtcatcagaacagaaccaggattcattgcgttcgagtggctgggcgagcagatccgggtaggtatgtggggtctggctgcccagagcatcttagattactgggagtaggggagaagccac

SEQ ID NO: 98 - DNA, 120 bp, Artificial Sequence
  SLC28A1
cccttcccagcctcactgcctgtttttgtttgttttgcttttttctttcagatcttcctgagctacacgaaggctggctccagcttcgtgtttggggaggcgctggtcaaggatgtcttt

SEQ ID NO: 99 - DNA, 120 bp, Artificial Sequence
  SLC28A1
agctacacgaaggctggctccagcttcgtgtttggggaggcgctggtcaaggatgtctttgcctttcaggtcagcttgactcagggtcccagaggcctttagcagccaccgcccagcgac

SEQ ID NO: 100 - DNA, 120 bp, Artificial Sequence
  SLC28A1
tgcatcctgcctgcctctaacctgcggtcctatgatctccttcccggcaggttctgcccatcattgtctttttcagctgtgtcatatccgttctctaccacgtgggcctcatgcagtggg

SEQ ID NO: 101 - DNA, 120 bp, Artificial Sequence
  SLC28A1
tcattgtctttttcagctgtgtcatatccgttctctaccacgtgggcctcatgcagtgggtgatcctgaaggtaagttcccagtgcccatggccagggctctcccagagtcaccagctca

SEQ ID NO: 102 - DNA, 120 bp, Artificial Sequence
  SLC28A1
tctggggtttgctgatgtcagcccacaaagaacattctgcttccttctagattgcctggctgatgcaagtcaccatgggcaccacagccactgagaccctgagtgtggctggaaacatct

SEQ ID NO: 103 - DNA, 120 bp, Artificial Sequence
  SLC28A1
tgatgcaagtcaccatgggcaccacagccactgagaccctgagtgtggctggaaacatctttgtgagccaggtgggtatggaagcctcctaccctcatgctcatcagcagcttccccaaa

SEQ ID NO: 104 - DNA, 120 bp, Artificial Sequence
  SLC28A1
gagaggatgtgcccaatcacccccaccctgcttgtctgacatctttcctgtttgcagaccgaggctccattactgatccggccctacttggcagacatgacactctctgaagtccacgtt

SEQ ID NO: 105 - DNA, 120 bp, Artificial Sequence
  SLC28A1
gaggctccattactgatccggccctacttggcagacatgacactctctgaagtccacgttgtcatgaccggaggttacgccaccattgctggcagcctgctgggtgcctacatctccttt

SEQ ID NO: 106 - DNA, 120 bp, Artificial Sequence
  SLC28A1
gtcatgaccggaggttacgccaccattgctggcagcctgctgggtgcctacatctcctttggggtaggtagagccctccttctgcttggctatgttgaggacctgaagcccatctttgtg

SEQ ID NO: 107 - DNA, 120 bp, Artificial Sequence
  SLC28A1
gtcgccagcatttcttctgactgtccacctagaacctgcactctcactcttgcagatcgatgccacctcgttgattgcagcctctgtgatggctgccccttgtgccttggccctctccaa

SEQ ID NO: 108 - DNA, 120 bp, Artificial Sequence
  SLC28A1
tgccacctcgttgattgcagcctctgtgatggctgccccttgtgccttggccctctccaagctggtctacccggaggtggaggagtccaagtttaggagggaggaaggagtgaaactgac

SEQ ID NO: 109 - DNA, 120 bp, Artificial Sequence
  SLC28A1
gctggtctacccggaggtggaggagtccaagtttaggagggaggaaggagtgaaactgacctatgggtgagcacagcaggaggtcctgcagacagggtagtggtacaaggtggggggagc

SEQ ID NO: 110 - DNA, 120 bp, Artificial Sequence
  SLC28A1
caggccagtaatgatcattcttgatcccaacaacagagatgctcagaacctcatagaagcagccagcactggggccgccatctccgtgaaggtggtcgccaacatcgctgccaacctgat

SEQ ID NO: 111 - DNA, 120 bp, Artificial Sequence
  SLC28A1
agccagcactggggccgccatctccgtgaaggtggtcgccaacatcgctgccaacctgattgcgttcctggctgtgctggactttatcaatgctgccctctcctggctgggagacatggt

SEQ ID NO: 112 - DNA, 120 bp, Artificial Sequence
  SLC28A1
tgcgttcctggctgtgctggactttatcaatgctgccctctcctggctgggagacatggtggacatccaagggctcagcttccaggtgcgtttctggccaccacactcagtctgtagaga

SEQ ID NO: 113 - DNA, 120 bp, Artificial Sequence
  SLC28A1
gccataccgttgtgccctcagctcatctgctcctacatcctgcggcctgtagccttcttgatgggtgtggcgtgggaggactgcccagtggtagctgagctgctggggatcaagctgttt

SEQ ID NO: 114 - DNA, 120 bp, Artificial Sequence
  SLC28A1
atgggtgtggcgtgggaggactgcccagtggtagctgagctgctggggatcaagctgtttctgaacgagtttgtggcctatcaagacctctccaagtacaagcaacgccgcctggcaggg

SEQ ID NO: 115 - DNA, 120 bp, Artificial Sequence
  SLC28A1
ctgaacgagtttgtggcctatcaagacctctccaagtacaagcaacgccgcctggcaggggccgaggagtgggtcggcgacaggaagcagtggatctccgtgagtgtcccagtcccttcc

SEQ ID NO: 116 - DNA, 120 bp, Artificial Sequence
  SLC28A1
caggcccatctgaggggagcccctcctcatgcatcttctgtattttcaggtcagagctgaagtcctcacgacgtttgccctctgtggatttgccaatttcagctccattgggatcatgct

SEQ ID NO: 117 - DNA, 120 bp, Artificial Sequence
  SLC28A1
agtcctcacgacgtttgccctctgtggatttgccaatttcagctccattgggatcatgctgggaggcttgagtgagtctaatcagggcctcaccagtgtctaggagagtctgggacttga

SEQ ID NO: 118 - DNA, 120 bp, Artificial Sequence
  SLC28A1
acacagcttcccaggccctgagcacttctgtccccttgcagcctccatggtcccccaacggaagagcgacttctcccagatagtgctccgggcgctcttcacgggagcctgtgtgtccct

SEQ ID NO: 119 - DNA, 120 bp, Artificial Sequence
  SLC28A1
gaagagcgacttctcccagatagtgctccgggcgctcttcacgggagcctgtgtgtccctggtgaacgcctgtatggcaggtgagtgcaggcctggcaggctcagaaggtggaaccctga

SEQ ID NO: 120 - DNA, 120 bp, Artificial Sequence
  SLC28A1
ggtggaaccctgactttctggctagcccgggggccctgccccacccaccactttccctctacagggatcctctacatgcccaggggggctgaagttgactgcatgtccctcttgaacacg

SEQ ID NO: 121 - DNA, 120 bp, Artificial Sequence
  SLC28A1
acagggatcctctacatgcccaggggggctgaagttgactgcatgtccctcttgaacacgaccctcagcagcagtagctttgagatttaccagtgctgccgtgaggccttccagaggtga

SEQ ID NO: 122 - DNA, 120 bp, Artificial Sequence
  SLC28A1
accctcagcagcagtagctttgagatttaccagtgctgccgtgaggccttccagaggtgagggcctgggctgtgggacctgcagggcacccacagtgatagacagaatgcctgagcgctg

SEQ ID NO: 123 - DNA, 120 bp, Artificial Sequence
  SLC28A1
gcccgcagaaccaggcctggagctcccactgcgatctttgctttctttttagcgtcaatccagagttcagcccagaggccctggacaactgctgtcggttttacaaccacacgatctgtg

SEQ ID NO: 124 - DNA, 120 bp, Artificial Sequence
  SLC28A1
cagagttcagcccagaggccctggacaactgctgtcggttttacaaccacacgatctgtgcacagtgaggacagaacatgcttgtgcttctgcgcttctgagggctgttctcccccggga

SEQ ID NO: 125 - DNA, 120 bp, Artificial Sequence
  SLC28A1
cgatggttgttgcccctcattttatttctagttccattagttatgttccagtaacgtgtttcttgctcttaggatattcaaaagtacacctgccgagtcccagccctgaggagtgttttc

SEQ ID NO: 126 - DNA, 120 bp, Artificial Sequence
  SLC28A1
tcttgctcttaggatattcaaaagtacacctgccgagtcccagccctgaggagtgttttcgtgcttcattgttaagtatcttggaggctctcagctggaaataaatgctcttcatttatt

SEQ ID NO: 127 - DNA, 120 bp, Artificial Sequence
  KDR-E11
tgtaccatccttccattaaagagagagagattttcaaattttaaaacttcaaactcactttgttttttccttcaattagagcaaattgatttttattaacttcaattttatttcctccct

SEQ ID NO: 128 - DNA, 120 bp, Artificial Sequence
  KDR-E11
gagagattttcaaattttaaaacttcaaactcactttgttttttccttcaattagagcaaattgatttttattaacttcaattttatttcctccctggaagtcctccacacttctccatt

SEQ ID NO: 129 - DNA, 120 bp, Artificial Sequence
  KDR-E11
tcaaactcactttgttttttccttcaattagagcaaattgatttttattaacttcaattttatttcctccctggaagtcctccacacttctccattcttcacaagggtatgggtttgtca

SEQ ID NO: 130 - DNA, 120 bp, Artificial Sequence
  KDR-E11
caattagagcaaattgatttttattaacttcaattttatttcctccctggaagtcctccacacttctccattcttcacaagggtatgggtttgtcactgagacagcttggctataagaaa

SEQ ID NO: 131 - DNA, 120 bp, Artificial Sequence
  KDR-E11
ggaagtcctccacacttctccattcttcacaagggtatgggtttgtcactgagacagcttggctataagaaagagataacagcgcatattatgatttaatttttctttaattagagtcaa

SEQ ID NO: 132 - DNA, 120 bp, Artificial Sequence
  TP53-E4
agacttggctgtcccagaatgcaagaagcccagacggaaaccgtagctgccctggtaggttttctgggaagggacagaagatgacaggggccaggagggggctggtgcaggggccgccgg

SEQ ID NO: 133 - DNA, 120 bp, Artificial Sequence
  TP53-E4
gaagcccagacggaaaccgtagctgccctggtaggttttctgggaagggacagaagatgacaggggccaggagggggctggtgcaggggccgccggtgtaggagctgctggtgcaggggc

SEQ ID NO: 134 - DNA, 120 bp, Artificial Sequence
  TP53-E4
gccctggtaggttttctgggaagggacagaagatgacaggggccaggagggggctggtgcaggggccgccggtgtaggagctgctggtgcaggggccacggggggagcagcctctggcat

SEQ ID NO: 135 - DNA, 120 bp, Artificial Sequence
  TP53-E4
gacagaagatgacaggggccaggagggggctggtgcaggggccgccggtgtaggagctgctggtgcaggggccacggggggagcagcctctggcattctgggagcttcatctggacctgg

SEQ ID NO: 136 - DNA, 120 bp, Artificial Sequence
  TP53-E4
tgtaggagctgctggtgcaggggccacggggggagcagcctctggcattctgggagcttcatctggacctgggtcttcagtgaaccattgttcaatatcgtccggggacagcatcaaatc

SEQ ID NO: 137 - DNA, 120 bp, Artificial Sequence
  TP53-E4
cacggggggagcagcctctggcattctgggagcttcatctggacctgggtcttcagtgaaccattgttcaatatcgtccggggacagcatcaaatcatccattgcttgggacggcaaggg

SEQ ID NO: 138 - DNA, 120 bp, Artificial Sequence
  TP53-E4
tctgggagcttcatctggacctgggtcttcagtgaaccattgttcaatatcgtccggggacagcatcaaatcatccattgcttgggacggcaagggggactgtagatgggtgaaaagagc

SEQ ID NO: 139 - DNA, 120 bp, Artificial Sequence
  ALK
tgcgaccgagctcagggcccaggctggttcatgctattcttgcttttcagaatggtatcctcgtaatgaccagctccaggggcagtagcggcttctaagggcaagccctgttgctggtag

SEQ ID NO: 140 - DNA, 120 bp, Artificial Sequence
  ALK
tcgtaatgaccagctccaggggcagtagcggcttctaagggcaagccctgttgctggtagccgtaattgacattcccacaagggaagtgacgtagcctgaacagaggtacctccttcata

SEQ ID NO: 141 - DNA, 120 bp, Artificial Sequence
  ALK
ccgtaattgacattcccacaagggaagtgacgtagcctgaacagaggtacctccttcatattggcagtcagcgaagagggctctaggagcagtgaggcccccggaagtctcccagttgca

SEQ ID NO: 142 - DNA, 120 bp, Artificial Sequence
  ALK
ttggcagtcagcgaagagggctctaggagcagtgaggcccccggaagtctcccagttgcaacgttaggtgggacagtacagcttccctccagccccaggttacccctgtcgtgtggctcc

SEQ ID NO: 143 - DNA, 120 bp, Artificial Sequence
  ALK
acgttaggtgggacagtacagcttccctccagccccaggttacccctgtcgtgtggctccttctttgctataggattattctttttggtgggtttctctgtaaaccaggagccgtacgtt

SEQ ID NO: 144 - DNA, 120 bp, Artificial Sequence
  ALK
ttctttgctataggattattctttttggtgggtttctctgtaaaccaggagccgtacgttgggttccacaagctggtgggcttgtttctggatccgtggaccttgtgcaactccgaagga

SEQ ID NO: 145 - DNA, 120 bp, Artificial Sequence
  ALK
gggttccacaagctggtgggcttgtttctggatccgtggaccttgtgcaactccgaaggagggttggactgagagaatgccatattcacgtgtcccccttccacggccggccctctaggg

SEQ ID NO: 146 - DNA, 120 bp, Artificial Sequence
  ALK
gggttggactgagagaatgccatattcacgtgtcccccttccacggccggccctctagggactcgaacagagatctctgcagctgtgggtttctttgcagccttgccagaggaggtggta

SEQ ID NO: 147 - DNA, 120 bp, Artificial Sequence
  ALK
actcgaacagagatctctgcagctgtgggtttctttgcagccttgccagaggaggtggtaggcagaggtggtggggcagctgggctgcgctcctcctcccgttttgcctgttgagagacc

SEQ ID NO: 148 - DNA, 120 bp, Artificial Sequence
  ALK
ggcagaggtggtggggcagctgggctgcgctcctcctcccgttttgcctgttgagagaccaggagaggaggaaccccctcagggtccttgggcctcacaggcactttctcttcctcttcc

SEQ ID NO: 149 - DNA, 120 bp, Artificial Sequence
  ALK
aggagaggaggaaccccctcagggtccttgggcctcacaggcactttctcttcctcttccacaagtggaccatattctatcggcaaagcggtgttgattacatccgggtcctgccgtagg

SEQ ID NO: 150 - DNA, 120 bp, Artificial Sequence
  ALK
gtttcatatagagtaaatgttgaccaaagggagaaaatgttttacctgggtgcagtattcaatcctctccaaaatgatggcaaagttgggcctgtcttcaggctgatgttgccagcactg

SEQ ID NO: 151 - DNA, 120 bp, Artificial Sequence
  ALK
aatcctctccaaaatgatggcaaagttgggcctgtcttcaggctgatgttgccagcactgagtcattatccggtatctaaaagaagaagcacattaattaaaataaggagaagcacaatg

SEQ ID NO: 152 - DNA, 120 bp, Artificial Sequence
  ALK
tgaaaagaaaaactgcttagtaactagcagaagtgttcctaaaagagtcatacacaggcccagggcagttcttgggtgggtccatccggcctccactggtgacaaactccagaacttcct

SEQ ID NO: 153 - DNA, 120 bp, Artificial Sequence
  ALK
cagggcagttcttgggtgggtccatccggcctccactggtgacaaactccagaacttcctggttgcttttgctggggtatggcatatatccaagagaaaagatttcccatagcagcactc

SEQ ID NO: 154 - DNA, 120 bp, Artificial Sequence
  ALK
ggttgcttttgctggggtatggcatatatccaagagaaaagatttcccatagcagcactccaaaggacctgggcatgggacagaggacatggagatggatatagacacacccacccacat

SEQ ID NO: 155 - DNA, 120 bp, Artificial Sequence
  ALK
tagagtcctttggcccaggagcaccaccttatggctgcagggatacctggaggatgatggctgacttaccatgtgtctgttttagaagtgaatattccttccatgaaggcctctgggggc

SEQ ID NO: 156 - DNA, 120 bp, Artificial Sequence
  ALK
ctgacttaccatgtgtctgttttagaagtgaatattccttccatgaaggcctctgggggcatccacttaactggcagcatggcacagcctccctttctatagtagctcgccctgtgggga

SEQ ID NO: 157 - DNA, 120 bp, Artificial Sequence
  ALK
atccacttaactggcagcatggcacagcctccctttctatagtagctcgccctgtggggaaggagaggaaaaccaaactaggatctggagatggcattaagcatctgccctgctgggaaa

SEQ ID NO: 158 - DNA, 120 bp, Artificial Sequence
  ALK
ggtggaagagacaggcccggaggggtgaggcagtctttactcacctgtagatgtctcgggccatcccgaagtctccaatcttggccactcttccagggcctggacaggtcaagaggcagt

SEQ ID NO: 159 - DNA, 120 bp, Artificial Sequence
  ALK
ccatcccgaagtctccaatcttggccactcttccagggcctggacaggtcaagaggcagtttctggcagcaatgtctctgggaagaaaggaaatgcatttcctaattttatccctaggaa

SEQ ID NO: 160 - DNA, 120 bp, Artificial Sequence
  ALK
agcgacaggatgacaggaagagcacagtcactttgactcaccggtggatgaagtggttttcctccaaatactgacagccacaggcaatgtcccgagccacgtgcagaaggtccagcatgg

SEQ ID NO: 161 - DNA, 120 bp, Artificial Sequence
  ALK
cctccaaatactgacagccacaggcaatgtcccgagccacgtgcagaaggtccagcatggccagggaggagggctggctctgtggggagacagaagcgggccactgacgaggagcttgtc

SEQ ID NO: 162 - DNA, 120 bp, Artificial Sequence
  ALK
atccttgctcctgtccttggcacaacaactgcagcaaagactggttctcactcaccgggcgagggcgggtctctcggaggaaggacttgaggtctccccccgccatgagctccagcagga

SEQ ID NO: 163 - DNA, 120 bp, Artificial Sequence
  ALK
gagggcgggtctctcggaggaaggacttgaggtctccccccgccatgagctccagcaggatgaaccggggcagggattgcaggctcaccccaatgcagcgaacaatgttctggtggttga

SEQ ID NO: 164 - DNA, 120 bp, Artificial Sequence
  ALK
tgaaccggggcagggattgcaggctcaccccaatgcagcgaacaatgttctggtggttgaatttgctgcagagcagagagggatgtaaccaaaattaactgagctgagtctgggcaaatc

SEQ ID NO: 165 - DNA, 120 bp, Artificial Sequence
  ALK
gggcagcaggggtcccgggctgagcctaaacccagaatcttgctggtgagcaggtgggaagaaccacagcaggctccacaggagttccatttgcaggagagtggctggagctgtgaggat

SEQ ID NO: 166 - DNA, 120 bp, Artificial Sequence
  ALK
gaaccacagcaggctccacaggagttccatttgcaggagagtggctggagctgtgaggatgttgctcaggcacttgggtgaggaagtgtctcagggggcaggagagtgtctttctcagat

SEQ ID NO: 167 - DNA, 120 bp, Artificial Sequence
  ALK
gttgctcaggcacttgggtgaggaagtgtctcagggggcaggagagtgtctttctcagatactggtgcgtggactgggtgctagaattcatggtcgatttctcccaggaaggcctcaggc

SEQ ID NO: 168 - DNA, 120 bp, Artificial Sequence
  ALK
actggtgcgtggactgggtgctagaattcatggtcgatttctcccaggaaggcctcaggcagaaggtgaagcaaaacaactgcttccaagagagactgggtgagacttgccaagtgacag

SEQ ID NO: 169 - DNA, 120 bp, Artificial Sequence
  ALK
tccaggttctttgggggcagaggggagttggggtgagggtgtctctctgtggctttacctgatgatcagggcttccatgaggaaatccagttcgtcctgttcagagcacacttcaggcag

SEQ ID NO: 170 - DNA, 120 bp, Artificial Sequence
  ALK
gatgatcagggcttccatgaggaaatccagttcgtcctgttcagagcacacttcaggcagcgtctgggcagagaaggggagggtggggaggaggaggaggctgtgagctgagaactgcag

SEQ ID NO: 171 - DNA, 120 bp, Artificial Sequence
  ALK
gagtccgcaagccaagggcaggctcaagagtgagccacttcttaccttcacagccacttgcagggggcttgggtcgttgggcattccggacacctggccttcatacacctccccaaaggc

SEQ ID NO: 172 - DNA, 120 bp, Artificial Sequence
  ALK
cagggggcttgggtcgttgggcattccggacacctggccttcatacacctccccaaaggcgccatggcccagacccctgtgcaaaggagaagacaagaggagacagagtcaaacaggcca

SEQ ID NO: 173 - DNA, 120 bp, Artificial Sequence
  ALK
ctcccaggacggcagcagggcgctcaccgaatgagggtgatgtttttccgcggcacctccttcaggtcactgatggaggaggtcttgccagcaaagcagtagttggggttgtagtcggtc

SEQ ID NO: 174 - DNA, 120 bp, Artificial Sequence
  ALK
ttcaggtcactgatggaggaggtcttgccagcaaagcagtagttggggttgtagtcggtcatgatggtcgaggtgcggagcttgctcagcttgtactcagggctctgcagctccatctgc

SEQ ID NO: 175 - DNA, 120 bp, Artificial Sequence
  ALK
atgatggtcgaggtgcggagcttgctcagcttgtactcagggctctgcagctccatctgcatggcttgcagctcctggtgcttccggcggtacactgcaggtgggtggtcagctgcaaca

SEQ ID NO: 176 - DNA, 120 bp, Artificial Sequence
  ALK
cagcctgagacactattcagtcctgccttcctgcccccttgggagtccctggggctctgtgcactcaccaatcatgatgccggagaaagccaggaccagggcggccacgagggcagaggt

SEQ ID NO: 177 - DNA, 120 bp, Artificial Sequence
  ALK
gcactcaccaatcatgatgccggagaaagccaggaccagggcggccacgagggcagaggtcaccacagagaggatcagcgagagtggcaggtgtggctccggggtgggtgacactggaag

SEQ ID NO: 178 - DNA, 120 bp, Artificial Sequence
  ALK
caccacagagaggatcagcgagagtggcaggtgtggctccggggtgggtgacactggaagacaggtcccactggggtattgacaaccacaccaggtctcctttgagttggtcccaagtca

SEQ ID NO: 179 - DNA, 120 bp, Artificial Sequence
  ALK
tcaggctatgggcccctctgcctcccctggccctgcccccttaccaatgcaggagacgccatcctcagccagcaccgtcccgtggtcacagaagcagatgaccttgtggctttcagggtc

SEQ ID NO: 180 - DNA, 120 bp, Artificial Sequence
  ALK
atcctcagccagcaccgtcccgtggtcacagaagcagatgaccttgtggctttcagggtccatgtgacattcgtctacctcacagtgactgcagtttagataatgcttaatattcacttc

SEQ ID NO: 181 - DNA, 120 bp, Artificial Sequence
  ALK
catgtgacattcgtctacctcacagtgactgcagtttagataatgcttaatattcacttccccgtggccttccatcactagtgacaaggagggagggtcagtcttgggccgagcctgcct

SEQ ID NO: 182 - DNA, 120 bp, Artificial Sequence
  ALK
gacctaagcaagtttgttctgctgcctggcagagaagctaccttttaaagctggggtgtacaggatgcccagtggactgatgaaggaaaccccatcttccccatccatttcggggtcatt

SEQ ID NO: 183 - DNA, 120 bp, Artificial Sequence
  ALK
caggatgcccagtggactgatgaaggaaaccccatcttccccatccatttcggggtcattgtttgaggctgcattgccgcctgagtagcaaaccagagcagagtttaacatggggggtgg

SEQ ID NO: 184 - DNA, 120 bp, Artificial Sequence
  ALK
gtgacaccttgaacacgaatcatctttacctatatatcctccgcctcctccacctgaggagcacccccctccaccccctccgaaaccccctcttgtctcccacccccacttcttcatggc

SEQ ID NO: 185 - DNA, 120 bp, Artificial Sequence
  ALK
gcacccccctccaccccctccgaaaccccctcttgtctcccacccccacttcttcatggcctgggggcaggaatgtcctccggtggcaccctcctgcaaagattttccggcccagagcaa

SEQ ID NO: 186 - DNA, 120 bp, Artificial Sequence
  ALK
ctgggggcaggaatgtcctccggtggcaccctcctgcaaagattttccggcccagagcaaggaagtgttatcattccagccacctccaccacctgcgggaagagatagggaacctgcgtg

SEQ ID NO: 187 - DNA, 120 bp, Artificial Sequence
  ALK
gaaggcctgggagaggttctgggagagggcacgcttgcagcgctttacctgcggctccggaattgccgtttagccctagaaccgaggagttattctccagtctctctgggtggaacgtgt

SEQ ID NO: 188 - DNA, 120 bp, Artificial Sequence
  ALK
aattgccgtttagccctagaaccgaggagttattctccagtctctctgggtggaacgtgtctgtcttggccccgtaggccctgccaccacctccggctgcaatgatcaggggcaccggca

SEQ ID NO: 189 - DNA, 120 bp, Artificial Sequence
  ALK
ctgtcttggccccgtaggccctgccaccacctccggctgcaatgatcaggggcaccggcactccatccttcatctgaccaggggagacattcagacattgagaaaccgagctgtgcttcc

SEQ ID NO: 190 - DNA, 120 bp, Artificial Sequence
  ALK
ctgacattgcagatgcacaggaacctggtggaaatctggcagcacacaccataccttaaatacgtaggtggctccaccccctcctcctccgcctcctgcccactcatgcacgcttctgtt

SEQ ID NO: 191 - DNA, 120 bp, Artificial Sequence
  ALK
tacgtaggtggctccaccccctcctcctccgcctcctgcccactcatgcacgcttctgttcacacggatttcttcttctatcacattgttctctccaatgcagactttctggattaactg

SEQ ID NO: 192 - DNA, 120 bp, Artificial Sequence
  ALK
cacacggatttcttcttctatcacattgttctctccaatgcagactttctggattaactggtttgtctgtagaaacaaaaagcacgttaggtttgtggccaaaccagagttctccacttt

SEQ ID NO: 193 - DNA, 120 bp, Artificial Sequence
  ALK
ggcctgacagagtgcagacgagaaacccctgctctgggcacttacactggggcaggcgtcctctccctgctgcccaaccaggatgtacagcatgtcatccttctccaggttgaagatgcc

SEQ ID NO: 194 - DNA, 120 bp, Artificial Sequence
  ALK
ctctccctgctgcccaaccaggatgtacagcatgtcatccttctccaggttgaagatgcccagcacagacacgccgtgggaccgcatcatggtgttcttcccgcctttcccgccagcagc

SEQ ID NO: 195 - DNA, 120 bp, Artificial Sequence
  ALK
cagcacagacacgccgtgggaccgcatcatggtgttcttcccgcctttcccgccagcagctccgtagcccgagatgctgcaatgggacaaagaacgttggctcccgctgtggtatgaaga

SEQ ID NO: 196 - DNA, 120 bp, Artificial Sequence
  ALK
gggtggtctgcccctcccctccccctcttccatacgcacctgtaggtgtcggtggctggcaccttccagatctggatgcctttcagggggccctcgctccccacctccacgctcaggttg

SEQ ID NO: 197 - DNA, 120 bp, Artificial Sequence
  ALK
accttccagatctggatgcctttcagggggccctcgctccccacctccacgctcaggttggagttctggtaggcgttgttgcactgtgcctgggtggggccatggggcccgctggcccca

SEQ ID NO: 198 - DNA, 120 bp, Artificial Sequence
  ALK
gagttctggtaggcgttgttgcactgtgcctgggtggggccatggggcccgctggccccacatgtggtgaacagccaatgaactgtggcacaagaggagaggcagtcactcatgtggcca

SEQ ID NO: 199 - DNA, 120 bp, Artificial Sequence
  ALK
ttctgccttttgcaacaagaagttactgtgctcacatttgtgagctgaacccttacctgtagggtcaaagatgggggtctgtcttggtgaattttccccgggtttcagctccttgtttgg

SEQ ID NO: 200 - DNA, 120 bp, Artificial Sequence
  ALK
agggtcaaagatgggggtctgtcttggtgaattttccccgggtttcagctccttgtttgggtttctctcaaacaggtttcttgatttgggtgctgtattctgcaggatcttgtcctctcc

SEQ ID NO: 201 - DNA, 120 bp, Artificial Sequence
  ALK
gtttctctcaaacaggtttcttgatttgggtgctgtattctgcaggatcttgtcctctccgctaactgcaatagagaagaccccacgggctgagttaggtgagggttgatttcagggtga

SEQ ID NO: 202 - DNA, 120 bp, Artificial Sequence
  ALK
atgggggttgggggacagagtgctggggtcagagtgaactcactggtgaggtagcagtccaggctgatggagatattgtcaaaagccacgatggctctggatccttgtccccaccatgcg

SEQ ID NO: 203 - DNA, 120 bp, Artificial Sequence
  ALK
aggctgatggagatattgtcaaaagccacgatggctctggatccttgtccccaccatgcgaccatctgcagccagaacctgtacacatcaagaggaatgtgtgtgaggagcaaactgggg

SEQ ID NO: 204 - DNA, 120 bp, Artificial Sequence
  ALK
ggagaagggtattgggggagatgcatagagcctacctgtcagacacatcgaggagaggcaacaccatccactgccacaggctcaagccttcataggcggcgacatgccagaccatcctgc

SEQ ID NO: 205 - DNA, 120 bp, Artificial Sequence
  ALK
acaccatccactgccacaggctcaagccttcataggcggcgacatgccagaccatcctgccttgctccttcccggttttgttctccactagcaccaaggacacgtttcccctcaagactc

SEQ ID NO: 206 - DNA, 120 bp, Artificial Sequence
  ALK
cttgctccttcccggttttgttctccactagcaccaaggacacgtttcccctcaagactccacgaatgagccaggacattcggagctgtgagggcgagaagagtcagaggacaaggtatg

SEQ ID NO: 207 - DNA, 120 bp, Artificial Sequence
  ALK
taatctgggttccggaagtgacaagaggtgggaggagaaattagagaactagagaaacaaggagacttgcctcacatggagagctcttgatcggtgcaggaaacgtagcactggtcactg

SEQ ID NO: 208 - DNA, 120 bp, Artificial Sequence
  ALK
ggagacttgcctcacatggagagctcttgatcggtgcaggaaacgtagcactggtcactgtagcactttcagaagcggggacatcagtggtactgagcaatagagcatggtctaggagag

SEQ ID NO: 209 - DNA, 120 bp, Artificial Sequence
  ALK
tagcactttcagaagcggggacatcagtggtactgagcaatagagcatggtctaggagagaggaaaagaatcacaagcacgccattatcaggaactgggggaccaggggtgcagggttaa

SEQ ID NO: 210 - DNA, 120 bp, Artificial Sequence
  ALK
gtctatgtgggcatgaagatgggcaccagagagaaggcaggagagcagtagtaccttggtggtcctggaaccgggcatcctttagggtcctgacctgccattgaggagtgtggggtgaca

SEQ ID NO: 211 - DNA, 120 bp, Artificial Sequence
  ALK
ggtcctggaaccgggcatcctttagggtcctgacctgccattgaggagtgtggggtgacagtgtgccttgggtccagccacagaagccatcttcaaagttgcagtaaaaacccacaggca

SEQ ID NO: 212 - DNA, 120 bp, Artificial Sequence
  ALK
gtgtgccttgggtccagccacagaagccatcttcaaagttgcagtaaaaacccacaggcagtttccctatggagagagcagagaggcaccatcattttcaggaccactaaaggcaaaata

SEQ ID NO: 213 - DNA, 120 bp, Artificial Sequence
  ALK
gggttatgagcatgggctgggctcaggcagggtggggcagccccatctactcacggcacatctggctctcatcttctccctgggcacagtcctggtggaagtcacaggcctgcccaagct

SEQ ID NO: 214 - DNA, 120 bp, Artificial Sequence
  ALK
tctggctctcatcttctccctgggcacagtcctggtggaagtcacaggcctgcccaagctggaggactgtcccattccaacaagtgaaggagctctgcagggccatcttggagcctgggg

SEQ ID NO: 215 - DNA, 120 bp, Artificial Sequence
  ALK
ggaggactgtcccattccaacaagtgaaggagctctgcagggccatcttggagcctggggatgttcctggagagcacacagacacacaaccatggtaagtttgcatggccccaggcagca

SEQ ID NO: 216 - DNA, 120 bp, Artificial Sequence
  ALK
tgacacatctaacacaataggctaccaaggagcgtgggaaagccagattcagataccttcactgcagttcttcagggcaaagaagtccactgcagacaagctgcggtttccactggagat

SEQ ID NO: 217 - DNA, 120 bp, Artificial Sequence
  ALK
actgcagttcttcagggcaaagaagtccactgcagacaagctgcggtttccactggagatgtattccagggccactcgaaatgggttgtctggacgcccgattcttccctggagcactgt

SEQ ID NO: 218 - DNA, 120 bp, Artificial Sequence
  ALK
gtattccagggccactcgaaatgggttgtctggacgcccgattcttccctggagcactgtccaactggttgcattggaaaacagaggagaaaagcatagagaaacagatatgagaattag

SEQ ID NO: 219 - DNA, 120 bp, Artificial Sequence
  ALK
gacatggagaagtacttacccatgcttccctggagtgggcatcaggaggatctctcttgcagcctcgttgtggggcagcagctgggcaatgtaccttccagagggctgcaggtgcctgtg

SEQ ID NO: 220 - DNA, 120 bp, Artificial Sequence
  ALK
agcctcgttgtggggcagcagctgggcaatgtaccttccagagggctgcaggtgcctgtgcaccgagacggccagtgtgcagtgctcactgctgctcctcatccacggactcaggatggt

SEQ ID NO: 221 - DNA, 120 bp, Artificial Sequence
  ALK
caccgagacggccagtgtgcagtgctcactgctgctcctcatccacggactcaggatggtgtgcttggagtcagctgaggtgttgagaaggagaaaggagcctggaaagagacagggaaa

SEQ ID NO: 222 - DNA, 120 bp, Artificial Sequence
  ALK
tgacccacccaggacatcaccagcagcctctcccttacctctgggcatctccttagaacgctctgccccaggcccatccagcaagtccatctgggaggcctcctcggaggggatgcggcg

SEQ ID NO: 223 - DNA, 120 bp, Artificial Sequence
  ALK
ctctgccccaggcccatccagcaagtccatctgggaggcctcctcggaggggatgcggcgccaggaccagctctggttcctgaggtcatgcagtggaggggaatactccagctcacaggg

SEQ ID NO: 224 - DNA, 120 bp, Artificial Sequence
  ALK
ccaggaccagctctggttcctgaggtcatgcagtggaggggaatactccagctcacaggggaagtcaaagctgcactccagacctgcaataatagccaagggtcaatggaaaaaaccatt

SEQ ID NO: 225 - DNA, 120 bp, Artificial Sequence
  ALK
acagagtccttattatgagatagtgacagtgtatctcaagtaaatattaaacatatacttaccatatcggctgcgatgagacaggaaagggaaggagtctttcattatccaggtgagatt

SEQ ID NO: 226 - DNA, 120 bp, Artificial Sequence
  ALK
accatatcggctgcgatgagacaggaaagggaaggagtctttcattatccaggtgagattccatgtaaaataatcaggagaaggagaaggcatgtttgttggtgattccaaggagctatg

SEQ ID NO: 227 - DNA, 120 bp, Artificial Sequence
  ALK
ccatgtaaaataatcaggagaaggagaaggcatgtttgttggtgattccaaggagctatgacctggacataaaaataaagaaaacactgatccatgtgcttggggtgtgtcttttagctg

SEQ ID NO: 228 - DNA, 120 bp, Artificial Sequence
  ALK
cggcacactcaggcgggagctgctcaccagtcccgaagatctggaagagaaggcggggctgggaggcgcgaattgccgcggacagccttccctctctgcccacttccgacgccttcttct

SEQ ID NO: 229 - DNA, 120 bp, Artificial Sequence
  ALK
gggaggcgcgaattgccgcggacagccttccctctctgcccacttccgacgccttcttctcgggcatcaggcggatcctcagtcgcccttcgccttggcgaatccaccaactgaacagct

SEQ ID NO: 230 - DNA, 120 bp, Artificial Sequence
  ALK
cgggcatcaggcggatcctcagtcgcccttcgccttggcgaatccaccaactgaacagctcgctgagattgaactggagcagccccacagccgcctccccggggggcccgacgcaaccct

SEQ ID NO: 231 - DNA, 120 bp, Artificial Sequence
  ALK
cgctgagattgaactggagcagccccacagccgcctccccggggggcccgacgcaaccctccaagatcgcctcctcgcccagctccagcaccaactgcttggcacgccggagcttgcgca

SEQ ID NO: 232 - DNA, 120 bp, Artificial Sequence
  ALK
ccaagatcgcctcctcgcccagctccagcaccaactgcttggcacgccggagcttgcgcacggagccgcccttcagcaccctggacagcgtccgggcctctgccggggctggtgaaccgg

SEQ ID NO: 233 - DNA, 120 bp, Artificial Sequence
  ALK
cggagccgcccttcagcaccctggacagcgtccgggcctctgccggggctggtgaaccggcggtccaggagacccccggcgccggccccagcaacctgagcagcggggcgcagtccagag

SEQ ID NO: 234 - DNA, 120 bp, Artificial Sequence
  ALK
cggtccaggagacccccggcgccggccccagcaacctgagcagcggggcgcagtccagagctagcgagccgcgggcctcgggcctgccagccttcagctccgaggaggatggtggcagca

SEQ ID NO: 235 - DNA, 120 bp, Artificial Sequence
  ALK
ctagcgagccgcgggcctcgggcctgccagccttcagctccgaggaggatggtggcagcagtaggtcccgggcgtagacacggaagagcgagggcaccacgaagtcaactgccagactct

SEQ ID NO: 236 - DNA, 120 bp, Artificial Sequence
  ALK
gtaggtcccgggcgtagacacggaagagcgagggcaccacgaagtcaactgccagactcttcctctgcaggcgcgagtagctgagtggctcccggggctgcagcggcggccccgcagctg

SEQ ID NO: 237 - DNA, 120 bp, Artificial Sequence
  ALK
tcctctgcaggcgcgagtagctgagtggctcccggggctgcagcggcggccccgcagctggggagcccgcgcgctggccggtccccatcccggagcccacagctgccgtggaaagcagca

SEQ ID NO: 238 - DNA, 120 bp, Artificial Sequence
  ALK
gggagcccgcgcgctggccggtccccatcccggagcccacagctgccgtggaaagcagcagcggcaggagccacaggagcccgatggctcccatcccgccggaggaggccgtttacactg

SEQ ID NO: 239 - DNA, 120 bp, Artificial Sequence; identical to SEQ ID NO: 162
  ALK-E23

SEQ ID NO: 240 - DNA, 120 bp, Artificial Sequence
  ALK-E23
ctcggaggaaggacttgaggtctccccccgccatgagctccagcaggatgaaccggggcagggattgcaggctcaccccaatgcagcgaacaatgttctggtggttgaatttgctgcaga

SEQ ID NO: 241 - DNA, 120 bp, Artificial Sequence
  ALK-E23
cccccgccatgagctccagcaggatgaaccggggcagggattgcaggctcaccccaatgcagcgaacaatgttctggtggttgaatttgctgcagagcagagagggatgtaaccaaaatt

SEQ ID NO: 242 - DNA, 120 bp, Artificial Sequence; identical to SEQ ID NO: 164
  ALK-E23

SEQ ID NO: 243 - DNA, 120 bp, Artificial Sequence
  ALK-E24
gacctagtattctgctctgaagggggaaatgtgagcccttgagatctgcggggaagcacacagatcagcgacaggatgacaggaagagcacagtcactttgactcaccggtggatgaagt

SEQ ID NO: 244 - DNA, 120 bp, Artificial Sequence
  ALK-E24
ggaaatgtgagcccttgagatctgcggggaagcacacagatcagcgacaggatgacaggaagagcacagtcactttgactcaccggtggatgaagtggttttcctccaaatactgacagc

SEQ ID NO: 245 - DNA, 120 bp, Artificial Sequence
  ALK-E24
cggggaagcacacagatcagcgacaggatgacaggaagagcacagtcactttgactcaccggtggatgaagtggttttcctccaaatactgacagccacaggcaatgtcccgagccacgt

SEQ ID NO: 246 - DNA, 120 bp, Artificial Sequence
  ALK-E24
aggatgacaggaagagcacagtcactttgactcaccggtggatgaagtggttttcctccaaatactgacagccacaggcaatgtcccgagccacgtgcagaaggtccagcatggccaggg

SEQ ID NO: 247 - DNA, 120 bp, Artificial Sequence
  ALK-E24
ggttttcctccaaatactgacagccacaggcaatgtcccgagccacgtgcagaaggtccagcatggccagggaggagggctggctctgtggggagacagaagcgggccactgacgaggag

SEQ ID NO: 248 - DNA, 120 bp, Artificial Sequence
  ALK-E24
cacaggcaatgtcccgagccacgtgcagaaggtccagcatggccagggaggagggctggctctgtggggagacagaagcgggccactgacgaggagcttgtcagtgagaggagggaaatc

SEQ ID NO: 249 - DNA, 120 bp, Artificial Sequence
  ALK-E24
gcagaaggtccagcatggccagggaggagggctggctctgtggggagacagaagcgggccactgacgaggagcttgtcagtgagaggagggaaatctgaaatgctggcttccagtgctca

SEQ ID NO: 250 - DNA, 120 bp, Artificial Sequence
  ALK-E24
aggagggctggctctgtggggagacagaagcgggccactgacgaggagcttgtcagtgagaggagggaaatctgaaatgctggcttccagtgctcacaaggaggcagaccgtgaacatgc

SEQ ID NO: 251 - DNA, 120 bp, Artificial Sequence
  ALK-E25
ctcgggccatcccgaagtctccaatcttggccactcttccagggcctggacaggtcaagaggcagtttctggcagcaatgtctctgggaagaaaggaaatgcatttcctaattttatccc

SEQ ID NO: 252 - DNA, 120 bp, Artificial Sequence
  ALK-E25
tcttggccactcttccagggcctggacaggtcaagaggcagtttctggcagcaatgtctctgggaagaaaggaaatgcatttcctaattttatccctaggaagatgagtgtacaacggcc

SEQ ID NO: 253 - DNA, 120 bp, Artificial Sequence
  ALK-E25
gacaggtcaagaggcagtttctggcagcaatgtctctgggaagaaaggaaatgcatttcctaattttatccctaggaagatgagtgtacaacggccatcactaggattttatctccaagc

SEQ ID NO: 254 - DNA, 120 bp, Artificial Sequence
  ALK-E25
cagcaatgtctctgggaagaaaggaaatgcatttcctaattttatccctaggaagatgagtgtacaacggccatcactaggattttatctccaagctgaagtttaaatagttccttccct

SEQ ID NO: 255 - DNA, 120 bp, Artificial Sequence
  ALK-E25
atgtaagggacaagcagccacaccccattcttgaggggctgaggtggaagagacaggcccggaggggtgaggcagtctttactcacctgtagatgtctcgggccatcccgaagtctccaa

SEQ ID NO: 256 - DNA, 120 bp, Artificial Sequence
  ALK-E25
ccattcttgaggggctgaggtggaagagacaggcccggaggggtgaggcagtctttactcacctgtagatgtctcgggccatcccgaagtctccaatcttggccactcttccagggcctg

SEQ ID NO: 257 - DNA, 120 bp, Artificial Sequence
  ALK-E25
agagacaggcccggaggggtgaggcagtctttactcacctgtagatgtctcgggccatcccgaagtctccaatcttggccactcttccagggcctggacaggtcaagaggcagtttctgg

SEQ ID NO: 258 - DNA, 120 bp, Artificial Sequence
  ALK-E25
aagttgacagggtaccaggagatgatgtaagggacaagcagccacaccccattcttgaggggctgaggtggaagagacaggcccggaggggtgaggcagtctttactcacctgtagatgt

SEQ ID NO: 259 - DNA, 120 bp, Artificial Sequence
  BRAF
acagaactgtgttttgatgttaacaaattgtacgaacacaagacttaagaaataagagcagatgctgccatgatggtggctacttgaaggctgcaaattctcctgtagagggaggacaag

SEQ ID NO: 260 - DNA, 120 bp, Artificial Sequence
  BRAF
gatgctgccatgatggtggctacttgaaggctgcaaattctcctgtagagggaggacaagagctaattttaaaaaagtcatctcaaataacctagagacacagaaaagcctcatttgagc

SEQ ID NO: 261 - DNA, 120 bp, Artificial Sequence
  BRAF
ttccttttgttgctactctcctgaactctctcactcatttgtttcagtggacaggaaacgcaccatatccccctgcctggatgggtgtttttggagaagcacaagcatatagactaaaat

SEQ ID NO: 262 - DNA, 120 bp, Artificial Sequence
  BRAF
caccatatccccctgcctggatgggtgtttttggagaagcacaagcatatagactaaaatcctctgtttggaaaccagcccgattcaaggagggttctgatgcactgcggtgaatttttg

SEQ ID NO: 263 - DNA, 120 bp, Artificial Sequence
  BRAF
cctctgtttggaaaccagcccgattcaaggagggttctgatgcactgcggtgaatttttggcaatgagcgggccagcagctcaatagaggcgagaatctacaaaaaaaaaaagaaaaaaa

SEQ ID NO: 264 - DNA, 120 bp, Artificial Sequence
  BRAF
tctgtctatgaatgttagtctgttcttttggatagcatgaagcttttacttacttggggaaagagtggtctctcatctcttttctttttgaggcactctgccattaatctcttcatggct

SEQ ID NO: 265 - DNA, 120 bp, Artificial Sequence
  BRAF
aagagtggtctctcatctcttttctttttgaggcactctgccattaatctcttcatggcttttggacagttactccgtaccttactgagatctggagacaggtatcctcgtcccaccata

SEQ ID NO: 266 - DNA, 120 bp, Artificial Sequence
  BRAF
tttggacagttactccgtaccttactgagatctggagacaggtatcctcgtcccaccataaaaattatctggagagagaaaaaaaagggaaataattcaaccttgtagataagttgaaaa

SEQ ID NO: 267 - DNA, 120 bp, Artificial Sequence
  BRAF
aagaattaactagtaaaggccttacccttctgttggtcacacattcctctcatggagagtaagcccttgccacatcatttattatactcccatggaggacaaagcacctaaaatgccaag

SEQ ID NO: 268 - DNA, 120 bp, Artificial Sequence
  BRAF
aagcccttgccacatcatttattatactcccatggaggacaaagcacctaaaatgccaagaagtggatgagagaagaactctgggatgcttttatctgtattttggagataatacttgtt

SEQ ID NO: 269 - DNA, 120 bp, Artificial Sequence
  BRAF
tggagccttgtatatagacggtaaaataaacaccaagacgtggtaaatatttacctggtccctgttgttgatgtttgaataaggtaactgtccagtcatcaattcatacagaacaattcc

SEQ ID NO: 270 - DNA, 120 bp, Artificial Sequence
  BRAF
cctgttgttgatgtttgaataaggtaactgtccagtcatcaattcatacagaacaattccaaatgcatatacatctgactgaaagctgtatggatttttatcttgcattctgatgacttc

SEQ ID NO: 271 - DNA, 120 bp, Artificial Sequence
  BRAF
aaatgcatatacatctgactgaaagctgtatggatttttatcttgcattctgatgacttctggtgcctgttagaacatacaaagaaaaatattcttcacttcaattgaataaagactgaa

SEQ ID NO: 272 - DNA, 120 bp, Artificial Sequence
  BRAF
taactcagcagcatctcagggccaaaaatttaatcagtggaaaaatagcctcaattcttaccatccacaaaatggatccagacaactgttcaaactgatgggacccactccatcgagatt

SEQ ID NO: 273 - DNA, 120 bp, Artificial Sequence
  BRAF
ccatccacaaaatggatccagacaactgttcaaactgatgggacccactccatcgagatttcactgtagctagaccaaaatcacctatttttactgtgaggtcttcatgaagaaatatat

SEQ ID NO: 274 - DNA, 120 bp, Artificial Sequence
  BRAF
tcactgtagctagaccaaaatcacctatttttactgtgaggtcttcatgaagaaatatatctgaggtgtagtaagtaaaggaaaacagtagatctcattttcctatcagagcaagcatta

SEQ ID NO: 275 - DNA, 120 bp, Artificial Sequence
  BRAF
aagacaaaatgcagaagaaaaagtcaggatgttttcaaacttcgcagacaaatttcaggaaggatactattactcttgaggtctctgtggatgattgacttggcgtgtaagtaactgaaa

SEQ ID NO: 276 - DNA, 120 bp, Artificial Sequence
  BRAF
aggatactattactcttgaggtctctgtggatgattgacttggcgtgtaagtaactgaaaaacaaaacatcattttaacctgagtagggctaaaggactctggcctcgaaatctacagaa

SEQ ID NO: 277 - DNA, 120 bp, Artificial Sequence
  BRAF
aatttacaagacatttaacgaatggaacttactccatgccctgtgcagtctgtcgtgcaatatctataagtttgatcatctcaaatttggtctcaatgatatggagatggtgatacaagc

SEQ ID NO: 278 - DNA, 120 bp, Artificial Sequence
  BRAF
tatctataagtttgatcatctcaaatttggtctcaatgatatggagatggtgatacaagctggagccctcacaccactgggtaacaatagccagttgtggctttgtggaatagcccatga

SEQ ID NO: 279 - DNA, 120 bp, Artificial Sequence
  BRAF
tggagccctcacaccactgggtaacaatagccagttgtggctttgtggaatagcccatgaagagtaggatattcacatgtcgtgttttcctgtacaaagaaatgtgacagtaaacattaa

SEQ ID NO: 280 - DNA, 120 bp, Artificial Sequence
  BRAF
ataaaaataacttctttctctggaaaagagtaattcacacaagctcacctgagtactcctacttcatttttgaaggcttgtaactgctgaggtgtaggtgctgtcacattcaacattttc

SEQ ID NO: 281 - DNA, 120 bp, Artificial Sequence
  BRAF
acttcatttttgaaggcttgtaactgctgaggtgtaggtgctgtcacattcaacattttcactgccacatcacctaaaaggcaattgttactccaagtgtcatttcaatttttaaaattt

SEQ ID NO: 282 - DNA, 120 bp, Artificial Sequence
  BRAF
taaaagttgttaaacatatcctattatgacttgtcacaatgtcaccacattacatacttaccatgccactttcccttgtagactgttccaaatgatccagatccaattctttgtcccact

SEQ ID NO: 283 - DNA, 120 bp, Artificial Sequence
  BRAF
ccatgccactttcccttgtagactgttccaaatgatccagatccaattctttgtcccactgtaatctgcccatcaggaatctcccaatcatcactcgagtcccgtctaccaagtgttttc

SEQ ID NO: 284 - DNA, 120 bp, Artificial Sequence
  BRAF
gtaatctgcccatcaggaatctcccaatcatcactcgagtcccgtctaccaagtgttttcttgataaaaacagtaaaaaagtcaagtcaagccaaacagaaaaagaaaaccttatgtttc

SEQ ID NO: 285 - DNA, 120 bp, Artificial Sequence
  BRAF
tgacttctaagaagaaagaattcagagaaaaaaagatatcatatactcttaccattcgattcctgtcttctgaggatgaagatgacttcctttctcgctgaggtcctggagatttctgta

SEQ ID NO: 286 - DNA, 120 bp, Artificial Sequence
  BRAF
tcctgtcttctgaggatgaagatgacttcctttctcgctgaggtcctggagatttctgtaaggctttcacgttagttagtgagccaggtaatgaggcagggggggtagcagacaaacctg

SEQ ID NO: 287 - DNA, 120 bp, Artificial Sequence
  BRAF
aggctttcacgttagttagtgagccaggtaatgaggcagggggggtagcagacaaacctgtggttgatcctaaattagtgaaaagaaaaatgtatacattaaggaggagcaagtatgtta

SEQ ID NO: 288 - DNA, 120 bp, Artificial Sequence
  BRAF
tataaaggaaataagcagcaaagcaattgcagtttccttgagtttttaaaaaaacctgaaatcactacttacctccatcaccacgaaatccttggtctctaatcaagtcctacaaataaa

SEQ ID NO: 289 - DNA, 120 bp, Artificial Sequence
  BRAF
atcactacttacctccatcaccacgaaatccttggtctctaatcaagtcctacaaataaatagtaatgtatatttattccaagcaagcatataatcagagagtagcgataacactgaatt

SEQ ID NO: 290 - DNA, 120 bp, Artificial Sequence
  BRAF
acttggtttttttttagttctagcaatgctggatacttacatcaatattgacaggttctattgtgtttatatgcacattgggagctgatgaggatcggtctcgttgcccaaattgatttc

SEQ ID NO: 291 - DNA, 120 bp, Artificial Sequence
  BRAF
ttgtgtttatatgcacattgggagctgatgaggatcggtctcgttgcccaaattgatttcgatgatcttcatctgctggtcggaagggctgtggaattggaatggattttgaaggagacg

SEQ ID NO: 292 - DNA, 120 bp, Artificial Sequence
  BRAF
gatgatcttcatctgctggtcggaagggctgtggaattggaatggattttgaaggagacggactggtgagaatttggggcctggaaaaatgaagtcattggaagataagattcagagtaa

SEQ ID NO: 293 - DNA, 120 bp, Artificial Sequence
  BRAF
gagatccaaaagaaagcggttcaagtagcatgtcgcccaagagcagaagtcaaaccatacccaatagagtccgaggcgggtgcggaaggggatgatccagatgttagggcagtctctgct

SEQ ID NO: 294 - DNA, 120 bp, Artificial Sequence
  BRAF
ccaatagagtccgaggcgggtgcggaaggggatgatccagatgttagggcagtctctgctaaggacgcctcttcctgtggtattgggtggtgttcaaagaacttggagacaaacagcaaa

SEQ ID NO: 295 - DNA, 120 bp, Artificial Sequence
  BRAF
aaggacgcctcttcctgtggtattgggtggtgttcaaagaacttggagacaaacagcaaactgtgaggcaaaacaaaacaaacctaacttgtgcaaaacccagaagcttcatataccaaa

SEQ ID NO: 296 - DNA, 120 bp, Artificial Sequence
  BRAF
aagtgtaaaatggtaggtagaaaagagatatttttggattacttactcaagttggtcataattaacacacatcagtggaacttctgtactacaacgctggtgaaatttataaccacatgt

SEQ ID NO: 297 - DNA, 120 bp, Artificial Sequence
  BRAF
attaacacacatcagtggaacttctgtactacaacgctggtgaaatttataaccacatgtttgacagcggaaaccctggaaaagcagctttcgacaaaagtcacaaaatgctaaggtgaa

SEQ ID NO: 298 - DNA, 120 bp, Artificial Sequence
  BRAF
ttgacagcggaaaccctggaaaagcagctttcgacaaaagtcacaaaatgctaaggtgaaaaacgtttttcgtacctgcaaagtaaaaaatcacagagatttcaaaaactcacaagaaaa

SEQ ID NO: 299 - DNA, 120 bp, Artificial Sequence
  BRAF
taaataaaaattcattcattaaaatctaaacatttttgacatttcaaaaaaaaatgtaaagatacatacaaagttgtgtgttgtaagtggaacattctccaacacttccacatgcaattc

SEQ ID NO: 300 - DNA, 120 bp, Artificial Sequence
  BRAF
gatacatacaaagttgtgtgttgtaagtggaacattctccaacacttccacatgcaattcttctccagtaagccaggaaatatcagtgtcccaaccaattggtttcttctctctgaaaaa

SEQ ID NO: 301 - DNA, 120 bp, Artificial Sequence
  BRAF
ttctccagtaagccaggaaatatcagtgtcccaaccaattggtttcttctctctgaaaaatgtagacacaagcctttcttggttattacacctaaaaatattcatatacctcatgctgaa

SEQ ID NO: 302 - DNA, 120 bp, Artificial Sequence
  BRAF
tccatcgttagaaatttaaatggcaataaattaattttaagtttaccccaaataaatgtatcactcttggacaaacagcagggtaaagagatgtactcttttcttcaagtcagctccaga

SEQ ID NO: 303 - DNA, 120 bp, Artificial Sequence
  BRAF
tcactcttggacaaacagcagggtaaagagatgtactcttttcttcaagtcagctccagaaaagacctacaacagcagaaaatggattgttcctggggtccaaaaaaaaaaaaaaaaaaa

SEQ ID NO: 304 - DNA, 120 bp, Artificial Sequence
  BRAF
agaaaacttcaaagtttaatgtgtgattttctttttaaacaaaatttcacgtcacatacaaaccatacccatcctgaattctgtaaacagcacagcactctgggattagacctctcatca

SEQ ID NO: 305 - DNA, 120 bp, Artificial Sequence
  BRAF
aaccatacccatcctgaattctgtaaacagcacagcactctgggattagacctctcatcatcagtgctttctttagactgtctcggactgtaactccacaccttgcaggtacctatggta

SEQ ID NO: 306 - DNA, 120 bp, Artificial Sequence
  BRAF
tcagtgctttctttagactgtctcggactgtaactccacaccttgcaggtacctatggtatcataaatatattgataagaggtaaagggagcaaattacattttttcatatcattaaaaa

SEQ ID NO: 307 - DNA, 120 bp, Artificial Sequence
  BRAF
atattaaaactgactcaccactgtcctctgtttgttgggcaggaagactctaacgataggtttttgtggtgacttggggttgctccgtgccacatctgtgggattttgaaaaactgaaag

SEQ ID NO: 308 - DNA, 120 bp, Artificial Sequence
  BRAF
tttttgtggtgacttggggttgctccgtgccacatctgtgggattttgaaaaactgaaagagatgaaggtagcactgaaaggctagaagaggaagaagatgtaacggtatccattgatgc

SEQ ID NO: 309 - DNA, 120 bp, Artificial Sequence
  BRAF
agatgaaggtagcactgaaaggctagaagaggaagaagatgtaacggtatccattgatgcagagctagaaacagaaaaatcagttccgttccccagagattccaataactgttgttctct

SEQ ID NO: 310 - DNA, 120 bp, Artificial Sequence
  BRAF
agagctagaaacagaaaaatcagttccgttccccagagattccaataactgttgttctctttgttggagtgcatctagcttgctggtgtattcttcataggcctataaaataaagcagac

SEQ ID NO: 311 - DNA, 120 bp, Artificial Sequence
  BRAF
gtacaaatgtttttataagttcattttttttcttttcaaaattactagatatgatactcaaaagcttacctccagatatattgatggtggattatgctccccaccaaatttgtccaatag

SEQ ID NO: 312 - DNA, 120 bp, Artificial Sequence
  BRAF
aaagcttacctccagatatattgatggtggattatgctccccaccaaatttgtccaatagggcctctatatgttcctgtgtcaacttaatcatttgtttgatattccacacctaaaaaat

SEQ ID NO: 313 - DNA, 120 bp, Artificial Sequence
  BRAF
ggcctctatatgttcctgtgtcaacttaatcatttgtttgatattccacacctaaaaaatatttcaaaagaatttaaataaaaatcacttagtatatgaattagaaatattttaacatag

SEQ ID NO: 314 - DNA, 120 bp, Artificial Sequence
  BRAF
gcccgcggagctggcccgagaaggtggctgagggcatcaagcccccaccgccgcctctttccaaaataaacaccagccagccgccgagcccggagtcgggagggcggcagggtggcgcca

SEQ ID NO: 315 - DNA, 120 bp, Artificial Sequence
  BRAF
ccaaaataaacaccagccagccgccgagcccggagtcgggagggcggcagggtggcgccagcactcacctcctccggaatggcagggtccgcagccgaagaggccgcggcgccggcgccg

SEQ ID NO: 316 - DNA, 120 bp, Artificial Sequence; identical to SEQ ID NO: 282
  BRAF-E11

SEQ ID NO: 317 - DNA, 120 bp, Artificial Sequence
  BRAF-E11
tatgacttgtcacaatgtcaccacattacatacttaccatgccactttcccttgtagactgttccaaatgatccagatccaattctttgtcccactgtaatctgcccatcaggaatctcc

SEQ ID NO: 318 - DNA, 120 bp, Artificial Sequence
  BRAF-E11
attacatacttaccatgccactttcccttgtagactgttccaaatgatccagatccaattctttgtcccactgtaatctgcccatcaggaatctcccaatcatcactcgagtcccgtcta

SEQ ID NO: 319 - DNA, 120 bp, Artificial Sequence
  BRAF-E11
cccttgtagactgttccaaatgatccagatccaattctttgtcccactgtaatctgcccatcaggaatctcccaatcatcactcgagtcccgtctaccaagtgttttcttgataaaaaca

SEQ ID NO: 320 - DNA, 120 bp, Artificial Sequence
  BRAF-E11
ccagatccaattctttgtcccactgtaatctgcccatcaggaatctcccaatcatcactcgagtcccgtctaccaagtgttttcttgataaaaacagtaaaaaagtcaagtcaagccaaa

SEQ ID NO: 321 - DNA, 120 bp, Artificial Sequence; identical to SEQ ID NO: 284
  BRAF-E11

SEQ ID NO: 322 - DNA, 120 bp, Artificial Sequence; identical to SEQ ID NO: 272
  BRAF-E15

SEQ ID NO: 323 - DNA, 120 bp, Artificial Sequence
  BRAF-E15
aaaatttaatcagtggaaaaatagcctcaattcttaccatccacaaaatggatccagacaactgttcaaactgatgggacccactccatcgagatttcactgtagctagaccaaaatcac

SEQ ID NO: 324 - DNA, 120 bp, Artificial Sequence
  BRAF-E15
cctcaattcttaccatccacaaaatggatccagacaactgttcaaactgatgggacccactccatcgagatttcactgtagctagaccaaaatcacctatttttactgtgaggtcttcat

SEQ ID NO: 325 - DNA, 120 bp, Artificial Sequence
  BRAF-E15
gatgggacccactccatcgagatttcactgtagctagaccaaaatcacctatttttactgtgaggtcttcatgaagaaatatatctgaggtgtagtaagtaaaggaaaacagtagatctc

SEQ ID NO: 326 - DNA, 120 bp, Artificial Sequence; identical to SEQ ID NO: 274
  BRAF-E15

SEQ ID NO: 327 - DNA, 120 bp, Artificial Sequence
  EGFR
cccctgactccgtccagtattgatcgggagagccggagcgagctcttcggggagcagcgatgcgaccctccgggacggccggggcagcgctcctggcgctgctggctgcgctctgcccgg

SEQ ID NO: 328 - DNA, 120 bp, Artificial Sequence
  EGFR
tgcgaccctccgggacggccggggcagcgctcctggcgctgctggctgcgctctgcccggcgagtcgggctctggaggaaaagaaaggtaagggcgtgtctcgccggctcccgcgccgcc

SEQ ID NO: 329 - DNA, 120 bp, Artificial Sequence
  EGFR
tgcatttctcagtatttcatgtgatatctgtctttttcttccagtttgccaaggcacgagtaacaagctcacgcagttgggcacttttgaagatcattttctcagcctccagaggatgtt

SEQ ID NO: 330 - DNA, 120 bp, Artificial Sequence
  EGFR
taacaagctcacgcagttgggcacttttgaagatcattttctcagcctccagaggatgttcaataactgtgaggtggtccttgggaatttggaaattacctatgtgcagaggaattatga

SEQ ID NO: 331 - DNA, 120 bp, Artificial Sequence
  EGFR
caataactgtgaggtggtccttgggaatttggaaattacctatgtgcagaggaattatgatctttccttcttaaaggttggtgactttgattttcctacacaaataaaattggagaaaat

SEQ ID NO: 332 - DNA, 120 bp, Artificial Sequence
  EGFR
atcacgcatttatgttttctcttcttagaccatccaggaggtggctggttatgtcctcattgccctcaacacagtggagcgaattcctttggaaaacctgcagatcatcagaggaaatat

SEQ ID NO: 333 - DNA, 120 bp, Artificial Sequence
  EGFR
tgccctcaacacagtggagcgaattcctttggaaaacctgcagatcatcagaggaaatatgtactacgaaaattcctatgccttagcagtcttatctaactatgatgcaaataaaaccgg

SEQ ID NO: 334 - DNA, 120 bp, Artificial Sequence
  EGFR
gtactacgaaaattcctatgccttagcagtcttatctaactatgatgcaaataaaaccggactgaaggagctgcccatgagaaatttacagggtgagaggctgggatgccaaggctgggg

SEQ ID NO: 335 - DNA, 120 bp, Artificial Sequence
  EGFR
gggaatttaaaggagctggaaagagtgctcaccgcagttccattctcccgcagaaatcctgcatggcgccgtgcggttcagcaacaaccctgccctgtgcaacgtggagagcatccagtg

SEQ ID NO: 336 - DNA, 120 bp, Artificial Sequence
  EGFR
gcatggcgccgtgcggttcagcaacaaccctgccctgtgcaacgtggagagcatccagtggcgggacatagtcagcagtgactttctcagcaacatgtcgatggacttccagaaccacct

SEQ ID NO: 337 - DNA, 120 bp, Artificial Sequence
  EGFR
gcgggacatagtcagcagtgactttctcagcaacatgtcgatggacttccagaaccacctgggcagctgtaagtgtcgcatacacactatctctgcctccagctcctatgggggacagct

SEQ ID NO: 338 - DNA, 120 bp, Artificial Sequence
  EGFR
gtcatcagtttctcatcatttcactgagatatgcatctattacttttacatttcaggccaaaagtgtgatccaagctgtcccaatgggagctgctggggtgcaggagaggagaactgcca

SEQ ID NO: 339 - DNA, 120 bp, Artificial Sequence
  EGFR
aaagtgtgatccaagctgtcccaatgggagctgctggggtgcaggagaggagaactgccagaaacgtaagtcagtgaacagcctcagacccatgtgtgaccgcccctctcttccttcact

SEQ ID NO: 340 - DNA, 120 bp, Artificial Sequence
  EGFR
tccctgggaaatgatcctaccctcactcttcagctcacagggaacctttgctctttttcagtgaccaaaatcatctgtgcccagcagtgctccgggcgctgccgtggcaagtcccccagt

SEQ ID NO: 341 - DNA, 120 bp, Artificial Sequence
  EGFR
gtgaccaaaatcatctgtgcccagcagtgctccgggcgctgccgtggcaagtcccccagtgactgctgccacaaccagtgtgctgcaggctgcacaggcccccgggagagcgactgcctg

SEQ ID NO: 342 - DNA, 120 bp, Artificial Sequence
  EGFR
gactgctgccacaaccagtgtgctgcaggctgcacaggcccccgggagagcgactgcctggtaagatgcccctccagcagcctccctggagcaggctggggctgcacccgccccacccac

SEQ ID NO: 343 - DNA, 120 bp, Artificial Sequence
  EGFR
gctgagtgtacttacctcacttgcccagcgtgtcctctctcctccataggtctgccgcaaattccgagacgaagccacgtgcaaggacacctgccccccactcatgctctacaaccccac

SEQ ID NO: 344 - DNA, 120 bp, Artificial Sequence
  EGFR
attccgagacgaagccacgtgcaaggacacctgccccccactcatgctctacaaccccaccacgtaccagatggatgtgaaccccgagggcaaatacagctttggtgccacctgcgtgaa

SEQ ID NO: 345 - DNA, 120 bp, Artificial Sequence
  EGFR
cacgtaccagatggatgtgaaccccgagggcaaatacagctttggtgccacctgcgtgaagaagtgtccccgtgagtcctcctctgtgggccctctaactggtcaggcatccttgtcccg

SEQ ID NO: 346 - DNA, 120 bp, Artificial Sequence
  EGFR
tgtgtgaggcccgagcacctggtgccaccgtcatcaccttcctttcatgctctcttccccaggtaattatgtggtgacagatcacggctcgtgcgtccgagcctgtggggccgacagcta

SEQ ID NO: 347 - DNA, 120 bp, Artificial Sequence
  EGFR
aggtaattatgtggtgacagatcacggctcgtgcgtccgagcctgtggggccgacagctatgagatggaggaagacggcgtccgcaagtgtaagaagtgcgaagggccttgccgcaaagg

SEQ ID NO: 348 - DNA, 120 bp, Artificial Sequence
  EGFR
tgagatggaggaagacggcgtccgcaagtgtaagaagtgcgaagggccttgccgcaaaggtaggaagcccgccggtgtgcggacgaggcttgttctcggctgctgaggctgggctctcat

SEQ ID NO: 349 - DNA, 120 bp, Artificial Sequence
  EGFR
tagctattcttaatccaacaaatgtgaacggaatacacgtctctcttatctctgcagtgtgtaacggaataggtattggtgaatttaaagactcactctccataaatgctacgaatatta

SEQ ID NO: 350 - DNA, 120 bp, Artificial Sequence
  EGFR
gtaacggaataggtattggtgaatttaaagactcactctccataaatgctacgaatattaaacacttcaaaaactgcacctccatcagtggcgatctccacatcctgccggtggcattta

SEQ ID NO: 351 - DNA, 120 bp, Artificial Sequence
  EGFR
aacacttcaaaaactgcacctccatcagtggcgatctccacatcctgccggtggcatttagggggtgagtcacaggttcagttgcttgtataaagaaaaacaaaatctgcctttttaact

SEQ ID NO: 352 - DNA, 120 bp, Artificial Sequence
  EGFR
taactggtagagattggtgatcaataatcaccctgttgtttgtttcagtgactccttcacacatactcctcctctggatccacaggaactggatattctgaaaaccgtaaaggaaatcac

SEQ ID NO: 353 - DNA, 120 bp, Artificial Sequence
  EGFR
acatactcctcctctggatccacaggaactggatattctgaaaaccgtaaaggaaatcacaggtttgagctgaattatcacatgaatataaatgggaaatcagtgttttagagagagaac

SEQ ID NO: 354 - DNA, 120 bp, Artificial Sequence
  EGFR
aactcctacgtggtgtgtgtctgaagtctttcatctgccttacagggtttttgctgattcaggcttggcctgaaaacaggacggacctccatgcctttgagaacctagaaatcatacgcg

SEQ ID NO: 355 - DNA, 120 bp, Artificial Sequence
  EGFR
aggcttggcctgaaaacaggacggacctccatgcctttgagaacctagaaatcatacgcggcaggaccaagcaacagtaagttgaccacagccaaagcctggtagattacatttgccttt

SEQ ID NO: 356 - DNA, 120 bp, Artificial Sequence
  EGFR
ttttcttctctccaatgtagtggtcagttttctcttgcagtcgtcagcctgaacataacatccttgggattacgctccctcaaggagataagtgatggagatgtgataatttcaggaaac

SEQ ID NO: 357 - DNA, 120 bp, Artificial Sequence
  EGFR
tccttgggattacgctccctcaaggagataagtgatggagatgtgataatttcaggaaacaaaaatttgtgctatgcaaatacaataaactggaaaaaactgtttgggacctccggtcag

SEQ ID NO: 358 - DNA, 120 bp, Artificial Sequence
  EGFR
aaaaatttgtgctatgcaaatacaataaactggaaaaaactgtttgggacctccggtcagaaaaccaaaattataagcaacagaggtgaaaacagctgcagtaagtcaccgctttctgtt

SEQ ID NO: 359 - DNA, 120 bp, Artificial Sequence
  EGFR
cccctcgggtccctgctctgtcactgactgctgtgacccactctgtctccgcagaggccacaggccaggtctgccatgccttgtgctcccccgagggctgctggggcccggagcccaggg

SEQ ID NO: 360 - DNA, 120 bp, Artificial Sequence
  EGFR
caggccaggtctgccatgccttgtgctcccccgagggctgctggggcccggagcccagggactgcgtctcttgccggaatgtcagccgaggcagggaatgcgtggacaagtgcaaccttc

SEQ ID NO: 361 - DNA, 120 bp, Artificial Sequence
  EGFR
actgcgtctcttgccggaatgtcagccgaggcagggaatgcgtggacaagtgcaaccttctggaggggtaggaggttatttctttaatccccttgcgttgatcaaaaataaggctccagg

SEQ ID NO: 362 - DNA, 120 bp, Artificial Sequence
  EGFR
aatgtctcaggggtgggctgacgggtttcctcttcctcctctcagtgagccaagggagtttgtggagaactctgagtgcatacagtgccacccagagtgcctgcctcaggccatgaacat

SEQ ID NO: 363 - DNA, 120 bp, Artificial Sequence
  EGFR
tgtggagaactctgagtgcatacagtgccacccagagtgcctgcctcaggccatgaacatcacctgcacaggacgggtaagagccccttgctgctatccacgtccatttcatgggaaggg

SEQ ID NO: 364 - DNA, 120 bp, Artificial Sequence
  EGFR
gaaagagacatgcatgaacatttttctccaccttggtgcagggaccagacaactgtatccagtgtgcccactacattgacggcccccactgcgtcaagacctgcccggcaggagtcatgg

SEQ ID NO: 365 - DNA, 120 bp, Artificial Sequence
  EGFR
agtgtgcccactacattgacggcccccactgcgtcaagacctgcccggcaggagtcatgggagaaaacaacaccctggtctggaagtacgcagacgccggccatgtgtgccacctgtgcc

SEQ ID NO: 366 - DNA, 120 bp, Artificial Sequence
  EGFR
gagaaaacaacaccctggtctggaagtacgcagacgccggccatgtgtgccacctgtgccatccaaactgcacctacgggtgagtggaaagtgaaggagaacagaacatttcctctcttg

SEQ ID NO: 367 - DNA, 120 bp, Artificial Sequence
  EGFR
gccaaatatagaaagaggggatttagtcaagatttaaattaaaaatgttagtggtcatttttctaatgtctttctattttttcccaggtcctaataaatcttcactgtctgactttagtc

SEQ ID NO: 368 - DNA, 120 bp, Artificial Sequence
  EGFR
ttctaatgtctttctattttttcccaggtcctaataaatcttcactgtctgactttagtctcccactaaaactgcatttcctttctacaatttcaatttctccctttgcttcaaataaag

SEQ ID NO: 369 - DNA, 120 bp, Artificial Sequence
  EGFR
tattgaaatgtacttgtccatctttctccaggccaggaaatgagagtctcaaagccatgttattctgcctttttaaactatcatcctgtaatcaaagtaatgatggcagcgtgtcccacc

SEQ ID NO: 370 - DNA, 120 bp, Artificial Sequence
  EGFR
tattctgcctttttaaactatcatcctgtaatcaaagtaatgatggcagcgtgtcccaccagagcgggagcccagctgctcaggagtcatgcttaggatggatcccttctcttctgccgt

SEQ ID NO: 371 - DNA, 120 bp, Artificial Sequence
  EGFR
agagcgggagcccagctgctcaggagtcatgcttaggatggatcccttctcttctgccgtcagagtttcagctgggttggggtggatgcagccacctccatgcctggccttctgcatctg

SEQ ID NO: 372 - DNA, 120 bp, Artificial Sequence
  EGFR
cagagtttcagctgggttggggtggatgcagccacctccatgcctggccttctgcatctgtgatcatcacggcctcctcctgccactgagcctcatgccttcacgtgtctgttccccccg

SEQ ID NO: 373 - DNA, 120 bp, Artificial Sequence
  EGFR
taaaaatctccaaaatatatgccaaagaagtagaatgagaaaaatgtatatttctctttcacttcctacagatgcactgggccaggtcttgaaggctgtccaacgaatgggtaagtgttc

SEQ ID NO: 374 - DNA, 120 bp, Artificial Sequence
  EGFR
acttcctacagatgcactgggccaggtcttgaaggctgtccaacgaatgggtaagtgttcacagctctgtgtcacatggacctcgtcaagaatgaccacactgctgtgggtgaagatgct

SEQ ID NO: 375 - DNA, 120 bp, Artificial Sequence
  EGFR
gactggggagagcttgagaaagttggaaacgttgccttagaagcctgttttttctccttttagaagctacatagtgtctcactttccaagatcattctacaagatgtcagtgcactgaaa

SEQ ID NO: 376 - DNA, 120 bp, Artificial Sequence
  EGFR
tagaagctacatagtgtctcactttccaagatcattctacaagatgtcagtgcactgaaacatgcaggggcgtgttgagtgccaaggccatggaatctgtcagcaacctcacccttcctt

SEQ ID NO: 377 - DNA, 120 bp, Artificial Sequence
  EGFR
ggaatctgtcagcaacctcacccttccttgttcctccacctcattccaggcctaagatcccgtccatcgccactgggatggtgggggccctcctcttgctgctggtggtggccctgggga

SEQ ID NO: 378 - DNA, 120 bp, Artificial Sequence
  EGFR
cgtccatcgccactgggatggtgggggccctcctcttgctgctggtggtggccctggggatcggcctcttcatgcgaaggcgccacatcgttcggaagcgcacgctgcggaggctgctgc

SEQ ID NO: 379 - DNA, 120 bp, Artificial Sequence
  EGFR
tcggcctcttcatgcgaaggcgccacatcgttcggaagcgcacgctgcggaggctgctgcaggagagggaggtgagtgccagtcctgggtgggctcaggagccctcgcaccccgacagga

SEQ ID NO: 380 - DNA, 120 bp, Artificial Sequence
  EGFR
gctttccagcatggtgagggctgaggtgacccttgtctctgtgttcttgtcccccccagcttgtggagcctcttacacccagtggagaagctcccaaccaagctctcttgaggatcttga

SEQ ID NO: 381 - DNA, 120 bp, Artificial Sequence
  EGFR
ttgtggagcctcttacacccagtggagaagctcccaaccaagctctcttgaggatcttgaaggaaactgaattcaaaaagatcaaagtgctgggctccggtgcgttcggcacggtgtata

SEQ ID NO: 382 - DNA, 120 bp, Artificial Sequence
  EGFR
aggaaactgaattcaaaaagatcaaagtgctgggctccggtgcgttcggcacggtgtataaggtaaggtccctggcacaggcctctgggctgggccgcagggcctctcatggtctggtgg

SEQ ID NO: 383 - DNA, 120 bp, Artificial Sequence
  EGFR
cacaattgccagttaacgtcttccttctctctctgtcatagggactctggatcccagaaggtgagaaagttaaaattcccgtcgctatcaaggaattaagagaagcaacatctccgaaag

SEQ ID NO: 384 - DNA, 120 bp, Artificial Sequence
  EGFR
gtgagaaagttaaaattcccgtcgctatcaaggaattaagagaagcaacatctccgaaagccaacaaggaaatcctcgatgtgagtttctgctttgctgtgtgggggtccatggctctga

SEQ ID NO: 385 - DNA, 120 bp, Artificial Sequence
  EGFR
cactgacgtgcctctccctccctccaggaagcctacgtgatggccagcgtggacaacccccacgtgtgccgcctgctgggcatctgcctcacctccaccgtgcagctcatcacgcagctc

SEQ ID NO: 386 - DNA, 120 bp, Artificial Sequence
  EGFR
cacgtgtgccgcctgctgggcatctgcctcacctccaccgtgcagctcatcacgcagctcatgcccttcggctgcctcctggactatgtccgggaacacaaagacaatattggctcccag

SEQ ID NO: 387 - DNA, 120 bp, Artificial Sequence
  EGFR
atgcccttcggctgcctcctggactatgtccgggaacacaaagacaatattggctcccagtacctgctcaactggtgtgtgcagatcgcaaaggtaatcagggaagggagatacggggag

SEQ ID NO: 388 - DNA, 120 bp, Artificial Sequence
  EGFR
catgatgatctgtccctcacagcagggtcttctctgtttcagggcatgaactacttggaggaccgtcgcttggtgcaccgcgacctggcagccaggaacgtactggtgaaaacaccgcag

SEQ ID NO: 389 - DNA, 120 bp, Artificial Sequence
  EGFR
gaccgtcgcttggtgcaccgcgacctggcagccaggaacgtactggtgaaaacaccgcagcatgtcaagatcacagattttgggctggccaaactgctgggtgcggaagagaaagaatac

SEQ ID NO: 390 - DNA, 120 bp, Artificial Sequence
  EGFR
catgtcaagatcacagattttgggctggccaaactgctgggtgcggaagagaaagaataccatgcagaaggaggcaaagtaaggaggtggctttaggtcagccagcattttcctgacacc

SEQ ID NO: 391 - DNA, 120 bp, Artificial Sequence
  EGFR
aacagagggaaactaatagttgtctcactgcctcatctctcaccatcccaaggtgcctatcaagtggatggcattggaatcaattttacacagaatctatacccaccagagtgatgtctg

SEQ ID NO: 392 - DNA, 120 bp, Artificial Sequence
  EGFR
caagtggatggcattggaatcaattttacacagaatctatacccaccagagtgatgtctggagctacggtgagtcataatcctgatgctaatgagtttgtactgaggccaagctggcttt

SEQ ID NO: 393 - DNA, 120 bp, Artificial Sequence
  EGFR
gttcattcatgatcccactgccttcttttcttgcttcatcctctcaggggtgactgtttgggagttgatgacctttggatccaagccatatgacggaatccctgccagcgagatctcctc

SEQ ID NO: 394 - DNA, 120 bp, Artificial Sequence
  EGFR
ggagttgatgacctttggatccaagccatatgacggaatccctgccagcgagatctcctccatcctggagaaaggagaacgcctccctcagccacccatatgtaccatcgatgtctacat

SEQ ID NO: 395 - DNA, 120 bp, Artificial Sequence
  EGFR
catcctggagaaaggagaacgcctccctcagccacccatatgtaccatcgatgtctacatgatcatggtcaagtgtgagtgactggtgggtctgtccacactgcctagctgagccttggt

SEQ ID NO: 396 - DNA, 120 bp, Artificial Sequence
  EGFR
cagtgttctaattgcactgttttttctcattccttccccaggctggatgatagacgcagatagtcgcccaaagttccgtgagttgatcatcgaattctccaaaatggcccgagaccccca

SEQ ID NO: 397 - DNA, 120 bp, Artificial Sequence
  EGFR
tagtcgcccaaagttccgtgagttgatcatcgaattctccaaaatggcccgagacccccagcgctaccttgtcattcaggtacaaattgcagtctgtgcttccattgggaagagtccctc

SEQ ID NO: 398 - DNA, 120 bp, Artificial Sequence
  EGFR
cgggccattctaatagcctcaaaatctctgcaccagggggatgaaagaatgcatttgccaagtcctacagactccaacttctaccgtgccctgatggatgaagaagacatggacgacgtg

SEQ ID NO: 399 - DNA, 120 bp, Artificial Sequence
  EGFR
agtcctacagactccaacttctaccgtgccctgatggatgaagaagacatggacgacgtggtggatgccgacgagtacctcatcccacagcagggcttcttcagcagcccctccacgtca

SEQ ID NO: 400 - DNA, 120 bp, Artificial Sequence
  EGFR
gtggatgccgacgagtacctcatcccacagcagggcttcttcagcagcccctccacgtcacggactcccctcctgagctctctggtatgaaatctctgtctctctctctctctcaagctg

SEQ ID NO: 401 - DNA, 120 bp, Artificial Sequence
  EGFR
attcaggaaaagtggatgagatgtggtacaagcattccatgggcaacttctctgtttctttttcagagtgcaaccagcaacaattccaccgtggcttgcattgatagaaatggggtatgt

SEQ ID NO: 402 - DNA, 120 bp, Artificial Sequence
  EGFR
tttcagagtgcaaccagcaacaattccaccgtggcttgcattgatagaaatggggtatgtatgaacaccttataagccagaatttacagctctccactatggctctattttacatggaaa

SEQ ID NO: 403 - DNA, 120 bp, Artificial Sequence
  EGFR
taaccttccctcatttcctcctgcagctgcaaagctgtcccatcaaggaagacagcttcttgcagcgatacagctcagaccccacaggcgccttgactgaggacagcatagacgacacct

SEQ ID NO: 404 - DNA, 120 bp, Artificial Sequence
  EGFR
tgcagcgatacagctcagaccccacaggcgccttgactgaggacagcatagacgacaccttcctcccagtgcctggtgagtggcttgtctggaaacagtcctgctcctcaacctcctcga

SEQ ID NO: 405 - DNA, 120 bp, Artificial Sequence
  EGFR
tcctcccagtgcctggtgagtggcttgtctggaaacagtcctgctcctcaacctcctcgacccactcagcagcagccagtctccagtgtccaagccaggtgctccctccagcatctccag

SEQ ID NO: 406 - DNA, 120 bp, Artificial Sequence
  EGFR
cccactcagcagcagccagtctccagtgtccaagccaggtgctccctccagcatctccagagggggaaacagtggcagatttgcagacacagtgaagggcgtaaggagcagataaacaca

SEQ ID NO: 407 - DNA, 120 bp, Artificial Sequence
  EGFR
atttctttccactttcagaatacataaaccagtccgttcccaaaaggcccgctggctctgtgcagaatcctgtctatcacaatcagcctctgaaccccgcgcccagcagagacccacact

SEQ ID NO: 408 - DNA, 120 bp, Artificial Sequence
  EGFR
tgcagaatcctgtctatcacaatcagcctctgaaccccgcgcccagcagagacccacactaccaggacccccacagcactgcagtgggcaaccccgagtatctcaacactgtccagccca

SEQ ID NO: 409 - DNA, 120 bp, Artificial Sequence
  EGFR
accaggacccccacagcactgcagtgggcaaccccgagtatctcaacactgtccagcccacctgtgtcaacagcacattcgacagccctgcccactgggcccagaaaggcagccaccaaa

SEQ ID NO: 410 - DNA, 120 bp, Artificial Sequence
  EGFR
cctgtgtcaacagcacattcgacagccctgcccactgggcccagaaaggcagccaccaaattagcctggacaaccctgactaccagcaggacttctttcccaaggaagccaagccaaatg

SEQ ID NO: 411 - DNA, 120 bp, Artificial Sequence
  EGFR
ttagcctggacaaccctgactaccagcaggacttctttcccaaggaagccaagccaaatggcatctttaagggctccacagctgaaaatgcagaatacctaagggtcgcgccacaaagca

SEQ ID NO: 412 - DNA, 120 bp, Artificial Sequence
  EGFR
gcatctttaagggctccacagctgaaaatgcagaatacctaagggtcgcgccacaaagcagtgaatttattggagcatgaccacggaggatagtatgagccctaaaaatccagactcttt

SEQ ID NO: 413 - DNA, 120 bp, Artificial Sequence; identical to SEQ ID NO: 380
  EGFR-E18

SEQ ID NO: 414 - DNA, 120 bp, Artificial Sequence
  EGFR-E18
ggtgacccttgtctctgtgttcttgtcccccccagcttgtggagcctcttacacccagtggagaagctcccaaccaagctctcttgaggatcttgaaggaaactgaattcaaaaagatca

SEQ ID NO: 415 - DNA, 120 bp, Artificial Sequence
  EGFR-E18
accaagctctcttgaggatcttgaaggaaactgaattcaaaaagatcaaagtgctgggctccggtgcgttcggcacggtgtataaggtaaggtccctggcacaggcctctgggctgggcc

SEQ ID NO: 416 - DNA, 120 bp, Artificial Sequence; identical to SEQ ID NO: 382
  EGFR-E18

SEQ ID NO: 417 - DNA, 120 bp, Artificial Sequence
  EGFR-E19
cctcaccttcggggtgcatcgctggtaacatccacccagatcactgggcagcatgtggcaccatctcacaattgccagttaacgtcttccttctctctctgtcatagggactctggatcc

SEQ ID NO: 418 - DNA, 120 bp, Artificial Sequence
  EGFR-E19
gtaacatccacccagatcactgggcagcatgtggcaccatctcacaattgccagttaacgtcttccttctctctctgtcatagggactctggatcccagaaggtgagaaagttaaaattc

SEQ ID NO: 419 - DNA, 120 bp, Artificial Sequence
  EGFR-E19
cagcatgtggcaccatctcacaattgccagttaacgtcttccttctctctctgtcatagggactctggatcccagaaggtgagaaagttaaaattcccgtcgctatcaaggaattaagag

SEQ ID NO: 420 - DNA, 120 bp, Artificial Sequence
  EGFR-E19
tgccagttaacgtcttccttctctctctgtcatagggactctggatcccagaaggtgagaaagttaaaattcccgtcgctatcaaggaattaagagaagcaacatctccgaaagccaaca

SEQ ID NO: 421 - DNA, 120 bp, Artificial Sequence
  EGFR-E19
cagaaggtgagaaagttaaaattcccgtcgctatcaaggaattaagagaagcaacatctccgaaagccaacaaggaaatcctcgatgtgagtttctgctttgctgtgtgggggtccatgg

SEQ ID NO: 422 - DNA, 120 bp, Artificial Sequence
  EGFR-E19
ccgtcgctatcaaggaattaagagaagcaacatctccgaaagccaacaaggaaatcctcgatgtgagtttctgctttgctgtgtgggggtccatggctctgaacctcaggcccacctttt

SEQ ID NO: 423 - DNA, 120 bp, Artificial Sequence
  EGFR-E19
aagcaacatctccgaaagccaacaaggaaatcctcgatgtgagtttctgctttgctgtgtgggggtccatggctctgaacctcaggcccaccttttctcatgtctggcagctgctctgct

SEQ ID NO: 424 - DNA, 120 bp, Artificial Sequence
  EGFR-E19
aggaaatcctcgatgtgagtttctgctttgctgtgtgggggtccatggctctgaacctcaggcccaccttttctcatgtctggcagctgctctgctctagaccctgctcatctccacatc

SEQ ID NO: 425 - DNA, 120 bp, Artificial Sequence
  EGFR-E20
ccttctggccaccatgcgaagccacactgacgtgcctctccctccctccaggaagcctacgtgatggccagcgtggacaacccccacgtgtgccgcctgctgggcatctgcctcacctcc

SEQ ID NO: 426 - DNA, 120 bp, Artificial Sequence; identical to SEQ ID NO: 425
  EGFR-E20

SEQ ID NO: 427 - DNA, 120 bp, Artificial Sequence
  EGFR-E20
gtggacaacccccacgtgtgccgcctgctgggcatctgcctcacctccaccgtgcagctcatcacgcagctcatgcccttcggctgcctcctggactatgtccgggaacacaaagacaat

SEQ ID NO: 428 - DNA, 120 bp, Artificial Sequence
  EGFR-E20
ctgctgggcatctgcctcacctccaccgtgcagctcatcacgcagctcatgcccttcggctgcctcctggactatgtccgggaacacaaagacaatattggctcccagtacctgctcaac

SEQ ID NO: 429 - DNA, 120 bp, Artificial Sequence; identical to SEQ ID NO: 387
  EGFR-E20

SEQ ID NO: 430 - DNA, 120 bp, Artificial Sequence
  EGFR-E20
tatgtccgggaacacaaagacaatattggctcccagtacctgctcaactggtgtgtgcagatcgcaaaggtaatcagggaagggagatacggggaggggagataaggagccaggatcctc

SEQ ID NO: 431 - DNA, 120 bp, Artificial Sequence
  EGFR-E21
agagcttcttcccatgatgatctgtccctcacagcagggtcttctctgtttcagggcatgaactacttggaggaccgtcgcttggtgcaccgcgacctggcagccaggaacgtactggtg

SEQ ID NO: 432 - DNA, 120 bp, Artificial Sequence
  EGFR-E21
tccctcacagcagggtcttctctgtttcagggcatgaactacttggaggaccgtcgcttggtgcaccgcgacctggcagccaggaacgtactggtgaaaacaccgcagcatgtcaagatc

SEQ ID NO: 433 - DNA, 120 bp, Artificial Sequence; identical to SEQ ID NO: 389
  EGFR-E21

SEQ ID NO: 434 - DNA, 120 bp, Artificial Sequence
  EGFR-E21
aaaacaccgcagcatgtcaagatcacagattttgggctggccaaactgctgggtgcggaagagaaagaataccatgcagaaggaggcaaagtaaggaggtggctttaggtcagccagcat

SEQ ID NO: 435 - DNA, 120 bp, Artificial Sequence
  EGFR-E21
acagattttgggctggccaaactgctgggtgcggaagagaaagaataccatgcagaaggaggcaaagtaaggaggtggctttaggtcagccagcattttcctgacaccagggaccaggct

SEQ ID NO: 436 - DNA, 120 bp, Artificial Sequence
  ERBB2
gccctcccagccgggtccagccggagccatggggccggagccgcagtgagcaccatggagctggcggccttgtgccgctgggggctcctcctcgccctcttgccccccggagccgcgagc

SEQ ID NO: 437 - DNA, 120 bp, Artificial Sequence
  ERBB2
ctggcggccttgtgccgctgggggctcctcctcgccctcttgccccccggagccgcgagcacccaaggtgggtctggtgtggggaggggacggagcagcggcgggaccctgccctgtgga

SEQ ID NO: 438 - DNA, 120 bp, Artificial Sequence
  ERBB2
catctgctctctcctgccagtgtgcaccggcacagacatgaagctgcggctccctgccagtcccgagacccacctggacatgctccgccacctctaccagggctgccaggtggtgcaggg

SEQ ID NO: 439 - DNA, 120 bp, Artificial Sequence
  ERBB2
tcccgagacccacctggacatgctccgccacctctaccagggctgccaggtggtgcagggaaacctggaactcacctacctgcccaccaatgccagcctgtccttcctgcaggtgaggcc

SEQ ID NO: 440 - DNA, 120 bp, Artificial Sequence
  ERBB2
aaacctggaactcacctacctgcccaccaatgccagcctgtccttcctgcaggtgaggcccgtgggcaacccagccaggccctgcctccagctgggctgagccctctgtttacaggtggg

SEQ ID NO: 441 - DNA, 120 bp, Artificial Sequence
  ERBB2
ttccccctcccaggatatccaggaggtgcagggctacgtgctcatcgctcacaaccaagtgaggcaggtcccactgcagaggctgcggattgtgcgaggcacccagctctttgaggacaa

SEQ ID NO: 442 - DNA, 120 bp, Artificial Sequence
  ERBB2
gaggcaggtcccactgcagaggctgcggattgtgcgaggcacccagctctttgaggacaactatgccctggccgtgctagacaatggagacccgctgaacaataccacccctgtcacagg

SEQ ID NO: 443 - DNA, 120 bp, Artificial Sequence
  ERBB2
ctatgccctggccgtgctagacaatggagacccgctgaacaataccacccctgtcacaggggcctccccaggaggcctgcgggagctgcagcttcgaagcctcacaggtggccttcaccg

SEQ ID NO: 444 - DNA, 120 bp, Artificial Sequence
  ERBB2
agcagaaggtgacagaaggggaaagggtcctctgatcattgctcaccccacagagatcttgaaaggaggggtcttgatccagcggaacccccagctctgctaccaggacacgattttgtg

SEQ ID NO: 445 - DNA, 120 bp, Artificial Sequence
  ERBB2
gaaaggaggggtcttgatccagcggaacccccagctctgctaccaggacacgattttgtggaaggacatcttccacaagaacaaccagctggctctcacactgatagacaccaaccgctc

SEQ ID NO: 446 - DNA, 120 bp, Artificial Sequence
  ERBB2
gaaggacatcttccacaagaacaaccagctggctctcacactgatagacaccaaccgctctcgggcctgtaagccatgcccctccctgctgcctcttctctcagacagcctgaccccagc

SEQ ID NO: 447 - DNA, 120 bp, Artificial Sequence
  ERBB2
ccgtcctctcgctgttagacatctctctcactgcctgtctctggttctgtcctcaggccacccctgttctccgatgtgtaagggctcccgctgctggggagagagttctgaggattgtca

SEQ ID NO: 448 - DNA, 120 bp, Artificial Sequence
  ERBB2
cccctgttctccgatgtgtaagggctcccgctgctggggagagagttctgaggattgtcagagccgtgagtctcagggaggcctggagtcagggaaggggagggctggggccgggtggaa

SEQ ID NO: 449 - DNA, 120 bp, Artificial Sequence
  ERBB2
tgctgatgagggtctggtgcccagggcgccactcagccctcatcctgccctttgcccaacagtgacgcgcactgtctgtgccggtggctgtgcccgctgcaaggggccactgcccactga

SEQ ID NO: 450 - DNA, 120 bp, Artificial Sequence
  ERBB2
agtgacgcgcactgtctgtgccggtggctgtgcccgctgcaaggggccactgcccactgactgctgccatgagcagtgtgctgccggctgcacgggccccaagcactctgactgcctggt

SEQ ID NO: 451 - DNA, 120 bp, Artificial Sequence
  ERBB2
ctgctgccatgagcagtgtgctgccggctgcacgggccccaagcactctgactgcctggtatgtgcctctgctttgtgcccaatgtgctctaccccccaggatgcaaggggtgggcaccc

SEQ ID NO: 452 - DNA, 120 bp, Artificial Sequence
  ERBB2
cacaccagggcaaaacagcacagtgaaagccagccacctgtccccccaggcctgcctccacttcaaccacagtggcatctgtgagctgcactgcccagccctggtcacctacaacacaga

SEQ ID NO: 453 - DNA, 120 bp, Artificial Sequence
  ERBB2
cttcaaccacagtggcatctgtgagctgcactgcccagccctggtcacctacaacacagacacgtttgagtccatgcccaatcccgagggccggtatacattcggcgccagctgtgtgac

SEQ ID NO: 454 - DNA, 120 bp, Artificial Sequence
  ERBB2
cacgtttgagtccatgcccaatcccgagggccggtatacattcggcgccagctgtgtgactgcctgtccctgtgagtgccagggagaaacacagttttctcattttggtggggaggtttg

SEQ ID NO: 455 - DNA, 120 bp, Artificial Sequence
  ERBB2
ctgctcatggtggtgcacgaagggccagggtatgtggctacatgttcctgatctccttagacaactacctttctacggacgtgggatcctgcaccctcgtctgccccctgcacaaccaag

SEQ ID NO: 456 - DNA, 120 bp, Artificial Sequence
  ERBB2
acaactacctttctacggacgtgggatcctgcaccctcgtctgccccctgcacaaccaagaggtgacagcagaggatggaacacagcggtgtgagaagtgcagcaagccctgtgcccgag

SEQ ID NO: 457 - DNA, 120 bp, Artificial Sequence
  ERBB2
aggtgacagcagaggatggaacacagcggtgtgagaagtgcagcaagccctgtgcccgaggtacccactcactgcccccgaggccagctgcagttcctgtccctctgcgcatgcagcctg

SEQ ID NO: 458 - DNA, 120 bp, Artificial Sequence
  ERBB2
cctgtcccggtatgaaggctgagacggccccttccccacccacccccacctcctcagtgtgctatggtctgggcatggagcacttgcgagaggtgagggcagttaccagtgccaatatcc

SEQ ID NO: 459 - DNA, 120 bp, Artificial Sequence
  ERBB2
gctatggtctgggcatggagcacttgcgagaggtgagggcagttaccagtgccaatatccaggagtttgctggctgcaagaagatctttgggagcctggcatttctgccggagagctttg

SEQ ID NO: 460 - DNA, 120 bp, Artificial Sequence
  ERBB2
aggagtttgctggctgcaagaagatctttgggagcctggcatttctgccggagagctttgatgggtaagagtgggcacgatgacctgagacagtgtcagggcagacagagtcctgaggat

SEQ ID NO: 461 - DNA, 120 bp, Artificial Sequence
  ERBB2
agtgatgtccaccctgttcctggccctgctgactcctctcctgacccctccagggacccagcctccaacactgccccgctccagccagagcagctccaagtgtttgagactctggaagag

SEQ ID NO: 462 - DNA, 120 bp, Artificial Sequence
  ERBB2
gcctccaacactgccccgctccagccagagcagctccaagtgtttgagactctggaagagatcacaggtgggctctgtctctgcatcctgttctgcaggggctgggagtccttgtcctgt

SEQ ID NO: 463 - DNA, 120 bp, Artificial Sequence
  ERBB2
tccttgtcctgtccccactcctttaatctcaccctctgcctgcaggttacctatacatctcagcatggccggacagcctgcctgacctcagcgtcttccagaacctgcaagtaatccggg

SEQ ID NO: 464 - DNA, 120 bp, Artificial Sequence
  ERBB2
cagcatggccggacagcctgcctgacctcagcgtcttccagaacctgcaagtaatccggggacgaattctgcacaagtgagcactgagaaagagggggcctgatggggaggagtcccagg

SEQ ID NO: 465 - DNA, 120 bp, Artificial Sequence
  ERBB2
tgcccacctttctcccatagtggcgcctactcgctgaccctgcaagggctgggcatcagctggctggggctgcgctcactgagggaactgggcagtggactggccctcatccaccataac

SEQ ID NO: 466 - DNA, 120 bp, Artificial Sequence
  ERBB2
tggctggggctgcgctcactgagggaactgggcagtggactggccctcatccaccataacacccacctctgcttcgtgcacacggtgccctgggaccagctctttcggaacccgcaccaa

SEQ ID NO: 467 - DNA, 120 bp, Artificial Sequence
  ERBB2
acccacctctgcttcgtgcacacggtgccctgggaccagctctttcggaacccgcaccaagctctgctccacactgccaaccggccagaggacgagtgtggtaagacagggagcccagtg

SEQ ID NO: 468 - DNA, 120 bp, Artificial Sequence
  ERBB2
tggacctggggcctcccctaaaagtcccctgcggtcccttcctcctcactgcagtgggcgagggcctggcctgccaccagctgtgcgcccgagggcactgctggggtccagggcccaccc

SEQ ID NO: 469 - DNA, 120 bp, Artificial Sequence
  ERBB2
agggcctggcctgccaccagctgtgcgcccgagggcactgctggggtccagggcccacccagtgtgtcaactgcagccagttccttcggggccaggagtgcgtggaggaatgccgagtac

SEQ ID NO: 470 - DNA, 120 bp, Artificial Sequence
  ERBB2
agtgtgtcaactgcagccagttccttcggggccaggagtgcgtggaggaatgccgagtactgcaggggtatgaggggcggaggagagggtggctggaggggtgcatggggctcctctcag

SEQ ID NO: 471 - DNA, 120 bp, Artificial Sequence
  ERBB2
catggggctcctctcagaccccctcaccactgtcccttctctcaggctccccagggagtatgtgaatgccaggcactgtttgccgtgccaccctgagtgtcagccccagaatggctcagt

SEQ ID NO: 472 - DNA, 120 bp, Artificial Sequence
  ERBB2
tgtgaatgccaggcactgtttgccgtgccaccctgagtgtcagccccagaatggctcagtgacctgttttggaccggtgagctgctggcgggctcagagctgggtggaggggggcagcga

SEQ ID NO: 473 - DNA, 120 bp, Artificial Sequence
  ERBB2
agtgccagccccccacaaatcttttctgccccccccaggaggctgaccagtgtgtggcctgtgcccactataaggaccctcccttctgcgtggcccgctgccccagcggtgtgaaacctg

SEQ ID NO: 474 - DNA, 120 bp, Artificial Sequence
  ERBB2
gtgcccactataaggaccctcccttctgcgtggcccgctgccccagcggtgtgaaacctgacctctcctacatgcccatctggaagtttccagatgaggagggcgcatgccagccttgcc

SEQ ID NO: 475 - DNA, 120 bp, Artificial Sequence
  ERBB2
acctctcctacatgcccatctggaagtttccagatgaggagggcgcatgccagccttgccccatcaactgcacccactcgtgagtccaacggtcttttctgcagaaaggaggactttcct

SEQ ID NO: 476 - DNA, 120 bp, Artificial Sequence
  ERBB2
aggctggaaaggtggttcccaagagggtggttcccagaattgttgatgagactgtttctcctgcagctgtgtggacctggatgacaagggctgccccgccgagcagagagccaggttggc

SEQ ID NO: 477 - DNA, 120 bp, Artificial Sequence
  ERBB2
ctgcagctgtgtggacctggatgacaagggctgccccgccgagcagagagccaggttggcctggaccccaggatgtacccttcattgcccttcactcccccactggatgctgggtggtca

SEQ ID NO: 478 - DNA, 120 bp, Artificial Sequence
  ERBB2
cctcccaccccaaactagccctcaatccctgaccctggcttccgcccccagccctctgacgtccatcatctctgcggtggttggcattctgctggtcgtggtcttgggggtggtctttgg

SEQ ID NO: 479 - DNA, 120 bp, Artificial Sequence
  ERBB2
gtccatcatctctgcggtggttggcattctgctggtcgtggtcttgggggtggtctttgggatcctcatcaagcgacggcagcagaagatccggaagtacacgatgcggagactgctgca

SEQ ID NO: 480 - DNA, 120 bp, Artificial Sequence
  ERBB2
gatcctcatcaagcgacggcagcagaagatccggaagtacacgatgcggagactgctgcaggaaacggaggtgaggcggggtgaagtcctcccagcccgcgtggggtctgcaccggcccc

SEQ ID NO: 481 - DNA, 120 bp, Artificial Sequence
  ERBB2
ccagcccgcgtggggtctgcaccggcccccggcactgacccaccaccccctcaccccagctggtggagccgctgacacctagcggagcgatgcccaaccaggcgcagatgcggatcctga

SEQ ID NO: 482 - DNA, 120 bp, Artificial Sequence
  ERBB2
tggtggagccgctgacacctagcggagcgatgcccaaccaggcgcagatgcggatcctgaaagagacggagctgaggaaggtgaaggtgcttggatctggcgcttttggcacagtctaca

SEQ ID NO: 483 - DNA, 120 bp, Artificial Sequence
  ERBB2
aagagacggagctgaggaaggtgaaggtgcttggatctggcgcttttggcacagtctacaaggtcagggccaggtcctggggtgggcggccccagaggatgggggcggtgcctggagggg

SEQ ID NO: 484 - DNA, 120 bp, Artificial Sequence
  ERBB2
gcccacgctcttctcactcatatcctcctctttctgcccagggcatctggatccctgatggggagaatgtgaaaattccagtggccatcaaagtgttgagggaaaacacatcccccaaag

SEQ ID NO: 485 - DNA, 120 bp, Artificial Sequence
  ERBB2
gggagaatgtgaaaattccagtggccatcaaagtgttgagggaaaacacatcccccaaagccaacaaagaaatcttagacgtaagcccctccaccctctcctgctaggaggacaggaagg

SEQ ID NO: 486 - DNA, 120 bp, Artificial Sequence
  ERBB2
accctctcagcgtacccttgtccccaggaagcatacgtgatggctggtgtgggctccccatatgtctcccgccttctgggcatctgcctgacatccacggtgcagctggtgacacagctt

SEQ ID NO: 487 - DNA, 120 bp, Artificial Sequence
  ERBB2
tatgtctcccgccttctgggcatctgcctgacatccacggtgcagctggtgacacagcttatgccctatggctgcctcttagaccatgtccgggaaaaccgcggacgcctgggctcccag

SEQ ID NO: 488 - DNA, 120 bp, Artificial Sequence
  ERBB2
atgccctatggctgcctcttagaccatgtccgggaaaaccgcggacgcctgggctcccaggacctgctgaactggtgtatgcagattgccaaggtatgcacctgggctctttgcaggtct

SEQ ID NO: 489 - DNA, 120 bp, Artificial Sequence
  ERBB2
caggccctcccagaaggtctacatgggtgcttcccattccaggggatgagctacctggaggatgtgcggctcgtacacagggacttggccgctcggaacgtgctggtcaagagtcccaac

SEQ ID NO: 490 - DNA, 120 bp, Artificial Sequence
  ERBB2
gatgtgcggctcgtacacagggacttggccgctcggaacgtgctggtcaagagtcccaaccatgtcaaaattacagacttcgggctggctcggctgctggacattgacgagacagagtac

SEQ ID NO: 491 - DNA, 120 bp, Artificial Sequence
  ERBB2
catgtcaaaattacagacttcgggctggctcggctgctggacattgacgagacagagtaccatgcagatgggggcaaggttaggtgaaggaccaaggagcagaggaggctgggtggagtg

SEQ ID NO: 492 - DNA, 120 bp, Artificial Sequence
  ERBB2
ggccacctccccacaacacacagttggaggacttcctcttctgccctcccaggtgcccatcaagtggatggcgctggagtccattctccgccggcggttcacccaccagagtgatgtgtg

SEQ ID NO: 493 - DNA, 120 bp, Artificial Sequence
  ERBB2
caagtggatggcgctggagtccattctccgccggcggttcacccaccagagtgatgtgtggagttatggtgtgtgatggggggtgttgggaggggtgggtgaggagccatggctggaggg

SEQ ID NO: 494 - DNA, 120 bp, Artificial Sequence
  ERBB2
taaagctccctctggccctcccactcctgaccctgtctctgccttaggtgtgactgtgtgggagctgatgacttttggggccaaaccttacgatgggatcccagcccgggagatccctga

SEQ ID NO: 495 - DNA, 120 bp, Artificial Sequence
  ERBB2
ggagctgatgacttttggggccaaaccttacgatgggatcccagcccgggagatccctgacctgctggaaaagggggagcggctgccccagccccccatctgcaccattgatgtctacat

SEQ ID NO: 496 - DNA, 120 bp, Artificial Sequence
  ERBB2
cctgctggaaaagggggagcggctgccccagccccccatctgcaccattgatgtctacatgatcatggtcaaatgtgcgtggctgagctgtgctggctgcctggaggagggtgggaggtc

SEQ ID NO: 497 - DNA, 120 bp, Artificial Sequence
  ERBB2
cagggcctgggactagcatgctgacctccctcctgccccaggttggatgattgactctgaatgtcggccaagattccgggagttggtgtctgaattctcccgcatggccagggaccccca

SEQ ID NO: 498 - DNA, 120 bp, Artificial Sequence
  ERBB2
atgtcggccaagattccgggagttggtgtctgaattctcccgcatggccagggacccccagcgctttgtggtcatccaggtactgggcctctgtgccccatccctgcctgtggctaagag

SEQ ID NO: 499 - DNA, 120 bp, Artificial Sequence
  ERBB2
ccatcctgcctctccttcctccacagaatgaggacttgggcccagccagtcccttggacagcaccttctaccgctcactgctggaggacgatgacatgggggacctggtggatgctgagg

SEQ ID NO: 500 - DNA, 120 bp, Artificial Sequence
  ERBB2
gcaccttctaccgctcactgctggaggacgatgacatgggggacctggtggatgctgaggagtatctggtaccccagcagggcttcttctgtccagaccctgccccgggcgctgggggca

SEQ ID NO: 501 - DNA, 120 bp, Artificial Sequence
  ERBB2
agtatctggtaccccagcagggcttcttctgtccagaccctgccccgggcgctgggggcatggtccaccacaggcaccgcagctcatctaccagggtcagtgccctcggtcacactgtgt

SEQ ID NO: 502 - DNA, 120 bp, Artificial Sequence
  ERBB2
catgactttctttcttgtccccagagtggcggtggggacctgacactagggctggagccctctgaagaggaggcccccaggtctccactggcaccctccgaaggggctggctccgatgta

SEQ ID NO: 503 - DNA, 120 bp, Artificial Sequence
  ERBB2
tctgaagaggaggcccccaggtctccactggcaccctccgaaggggctggctccgatgtatttgatggtgacctgggaatgggggcagccaaggggctgcaaagcctccccacacatgac

SEQ ID NO: 504 - DNA, 120 bp, Artificial Sequence
  ERBB2
tttgatggtgacctgggaatgggggcagccaaggggctgcaaagcctccccacacatgaccccagccctctacagcggtacagtgaggaccccacagtacccctgccctctgagactgat

SEQ ID NO: 505 - DNA, 120 bp, Artificial Sequence
  ERBB2
cccagccctctacagcggtacagtgaggaccccacagtacccctgccctctgagactgatggctacgttgcccccctgacctgcagcccccagcctggtatggagtccagtctaagcaga

SEQ ID NO: 506 - DNA, 120 bp, Artificial Sequence
  ERBB2
ccctaatgggtcaccttctcttgacctttcagaatatgtgaaccagccagatgttcggccccagcccccttcgccccgagagggccctctgcctgctgcccgacctgctggtgccactct

SEQ ID NO: 507 - DNA, 120 bp, Artificial Sequence
  ERBB2
ccagcccccttcgccccgagagggccctctgcctgctgcccgacctgctggtgccactctggaaaggcccaagactctctccccagggaagaatggggtcgtcaaagacgtttttgcctt

SEQ ID NO: 508 - DNA, 120 bp, Artificial Sequence
  ERBB2
ggaaaggcccaagactctctccccagggaagaatggggtcgtcaaagacgtttttgcctttgggggtgccgtggagaaccccgagtacttgacaccccagggaggagctgcccctcagcc

SEQ ID NO: 509 - DNA, 120 bp, Artificial Sequence
  ERBB2
tgggggtgccgtggagaaccccgagtacttgacaccccagggaggagctgcccctcagccccaccctcctcctgccttcagcccagccttcgacaacctctattactgggaccaggaccc

SEQ ID NO: 510 - DNA, 120 bp, Artificial Sequence
  ERBB2
ccaccctcctcctgccttcagcccagccttcgacaacctctattactgggaccaggacccaccagagcggggggctccacccagcaccttcaaagggacacctacggcagagaacccaga

SEQ ID NO: 511 - DNA, 120 bp, Artificial Sequence
  ERBB2
accagagcggggggctccacccagcaccttcaaagggacacctacggcagagaacccagagtacctgggtctggacgtgccagtgtgaaccagaaggccaagtccgcagaagccctgatg

SEQ ID NO: 512 - DNA, 120 bp, Artificial Sequence
  ERBB4
aaaaaccacaactgagcttacaccacagtattccggtgtctgtaaggtggaggcggcagcacagtgcctggcttcagggagaactcagagaggtattcaggattctctgccacaataggc

SEQ ID NO: 513 - DNA, 120 bp, Artificial Sequence
  ERBB4
acagtgcctggcttcagggagaactcagagaggtattcaggattctctgccacaataggccggatccgcccattctgtttataaaaatattttgtgctgtactcctgcaggtagtctggg

SEQ ID NO: 514 - DNA, 120 bp, Artificial Sequence
  ERBB4
cggatccgcccattctgtttataaaaatattttgtgctgtactcctgcaggtagtctgggtgctgaagggtgctccgaggtggcaggctgtggttccagtagtcagggttgtcaaacgct

SEQ ID NO: 515 - DNA, 120 bp, Artificial Sequence
  ERBB4
tgctgaagggtgctccgaggtggcaggctgtggttccagtagtcagggttgtcaaacgctttcttggccttctctggcattgacagtatgttgttcttcaggtactcagcttttcccaag

SEQ ID NO: 516 - DNA, 120 bp, Artificial Sequence
  ERBB4
ttcttggccttctctggcattgacagtatgttgttcttcaggtactcagcttttcccaaggtgttggcaaaggtgttgaggtacagtggctcattcacatactcatcctcggccttgggt

SEQ ID NO: 517 - DNA, 120 bp, Artificial Sequence
  ERBB4
gtgttggcaaaggtgttgaggtacagtggctcattcacatactcatcctcggccttgggtggaccattggatgcattgtgatattcgggattatccaatgcttgaaggtctccatttttt

SEQ ID NO: 518 - DNA, 120 bp, Artificial Sequence
  ERBB4
ggaccattggatgcattgtgatattcgggattatccaatgcttgaaggtctccattttttctccgagaaacaaaagggttctcctccactggattcaggtattctaaaggaataaaaaaa

SEQ ID NO: 519 - DNA, 120 bp, Artificial Sequence
  ERBB4
tggcgatcgtttctgaataatcagttcataccttgtttgggtttgtctcgcataggagtcatgtaaccttcctcatccagctctcctcgtgggctccgttctggggcaaacacggtgggg

SEQ ID NO: 520 - DNA, 120 bp, Artificial Sequence
  ERBB4
atgtaaccttcctcatccagctctcctcgtgggctccgttctggggcaaacacggtggggtcagcactgtacctctgggtgctactgtcctcttggacatggggtgccactggcttgcgt

SEQ ID NO: 521 - DNA, 120 bp, Artificial Sequence
  ERBB4
tcagcactgtacctctgggtgctactgtcctcttggacatggggtgccactggcttgcgtagggtgccattacagcaggagtcatcaaaaatctcagcagtagcaccctgtgccacagga

SEQ ID NO: 522 - DNA, 120 bp, Artificial Sequence
  ERBB4
agggtgccattacagcaggagtcatcaaaaatctcagcagtagcaccctgtgccacaggagcttctggaattgtgctagttggggctctgtagggcacagacactccttgttcagcagca

SEQ ID NO: 523 - DNA, 120 bp, Artificial Sequence
  ERBB4
gcttctggaattgtgctagttggggctctgtagggcacagacactccttgttcagcagcaaaacctccatctcggtatacaaactggttctgttaataagagaaacatatgtggagagaa

SEQ ID NO: 524 - DNA, 120 bp, Artificial Sequence
  ERBB4
gagaggaaacatggtaagcaaagaccgaaaatcctaaaagatgaaggttgattgtgaaatacttactcctgacatgggggtgtaggcaggaggagggctgtgtccaatttcactctaata

SEQ ID NO: 525 - DNA, 120 bp, Artificial Sequence
  ERBB4
acttactcctgacatgggggtgtaggcaggaggagggctgtgtccaatttcactctaataggaaagaaaaatggaatgatggatataataagaggcaatatgaatgaaaaaattaaaaaa

SEQ ID NO: 526 - DNA, 120 bp, Artificial Sequence
  ERBB4
aaagaatatgatatgtgtatataattatttcttaccctattcgagtcaattcttgctctggaagtatagatgggaggtgggatgttgaaagcctgagggaccaagtactcctcagcatcc

SEQ ID NO: 527 - DNA, 120 bp, Artificial Sequence
  ERBB4
gaagtatagatgggaggtgggatgttgaaagcctgagggaccaagtactcctcagcatccatcatatcttccaaatcctcttcatccaagagattctgaaagaacttgctgtcatttgga

SEQ ID NO: 528 - DNA, 120 bp, Artificial Sequence
  ERBB4
atcatatcttccaaatcctcttcatccaagagattctgaaagaacttgctgtcatttggactgggaagcttcatacgatcatcaccctaaaagaaagattgcccatcagacacaaatatg

SEQ ID NO: 529 - DNA, 120 bp, Artificial Sequence
  ERBB4
ccattggcctagtcttaaaggcataagtcaaatgtactcacctgaataactaggtatctttgagggtctcgagccatccttgaaaactcagcagccagttccttaaatttaggtctactg

SEQ ID NO: 530 - DNA, 120 bp, Artificial Sequence
  ERBB4
tgagggtctcgagccatccttgaaaactcagcagccagttccttaaatttaggtctactgtcagcatcaatcatccaacctggaaatttacacagtgaaaatgtcactatattcgtaact

SEQ ID NO: 531 - DNA, 120 bp, Artificial Sequence
  ERBB4
actttactaagaatgatgatggtgataacattattttgcagtcttacatttgaccatgaccatgtaaacgtcaatagtgcagatgggaggctgaggcaaacgttctcctttctctaataa

SEQ ID NO: 532 - DNA, 120 bp, Artificial Sequence
  ERBB4
catgtaaacgtcaatagtgcagatgggaggctgaggcaaacgttctcctttctctaataaatcagggatttctcgcgttggaattccatcatagggttttcctccaaaggtcatcagttc

SEQ ID NO: 533 - DNA, 120 bp, Artificial Sequence
  ERBB4
atcagggatttctcgcgttggaattccatcatagggttttcctccaaaggtcatcagttcccatatagtaactcctatattggagaaaaaattcttacttaagcatattaacaacatatg

SEQ ID NO: 534 - DNA, 120 bp, Artificial Sequence
  ERBB4
acatatgtatttttgctttacaagctttaattcgcaaagaagatttatttaccatagctccaaacgtcactctgatgggtgaatttcctgtaatgtatacactccagagccatccattta

SEQ ID NO: 535 - DNA, 120 bp, Artificial Sequence
  ERBB4
caaacgtcactctgatgggtgaatttcctgtaatgtatacactccagagccatccatttaattggcatctatagagaagtaagaagtaaaagttttaaaattacattaaaaattcatttc

SEQ ID NO: 536 - DNA, 120 bp, Artificial Sequence
  ERBB4
tactatattttcaagcaagattgctctcaaaaagatacccacctttcctccatcagcattgtactctttttcatctccttccaagagtctggctagcccaaaatctgtgattttcacatg

SEQ ID NO: 537 - DNA, 120 bp, Artificial Sequence
  ERBB4
gtactctttttcatctccttccaagagtctggctagcccaaaatctgtgattttcacatggtttggagatttcactaagacattacgggctgccaaatcccgatgaacgagtcgtctttc

SEQ ID NO: 538 - DNA, 120 bp, Artificial Sequence
  ERBB4
gtttggagatttcactaagacattacgggctgccaaatcccgatgaacgagtcgtctttcttccaggtacatcattccctgaaaaatatcaagttccttaatgatattcagttaatgccc

SEQ ID NO: 539 - DNA, 120 bp, Artificial Sequence
  ERBB4
tttccatagaaattgacaggcacttaccttagctatctggacacaccagttaagcagcagttgtgatccaatgttatccttgtgctcgtggacatactccaacaggcagccatggggcat

SEQ ID NO: 540 - DNA, 120 bp, Artificial Sequence
  ERBB4
ttgtgatccaatgttatccttgtgctcgtggacatactccaacaggcagccatggggcataagttgagtaaccagctggatggttgggctcagacacacacccagcaaccggactaggtg

SEQ ID NO: 541 - DNA, 120 bp, Artificial Sequence
  ERBB4
aagttgagtaaccagctggatggttgggctcagacacacacccagcaaccggactaggtgtggatgatccatacttgccatgatcagagcttcctgtaagaaaaaaatgcaataccatga

SEQ ID NO: 542 - DNA, 120 bp, Artificial Sequence
  ERBB4
ataatggagaaaaatgtgattgcctgggtgtctgtacttacatccatgaactccacatttgccttgggaccagttgtctcattaagaatcttaatagccacaggaatcttcacagtttct

SEQ ID NO: 543 - DNA, 120 bp, Artificial Sequence
  ERBB4
gccttgggaccagttgtctcattaagaatcttaatagccacaggaatcttcacagtttctccttcaggtacccaaataccctttggggaaaaaaatttacattaaatatgacatctcaac

SEQ ID NO: 544 - DNA, 120 bp, Artificial Sequence
  ERBB4
ttattttctaaacatctaaaacaaaacttaactaacgatatgcgttgttttttacttactttataaaccgttccaaaagcacctgagccaaggacttttaccctcttcagctcagtttct

SEQ ID NO: 545 - DNA, 120 bp, Artificial Sequence
  ERBB4
ttataaaccgttccaaaagcacctgagccaaggacttttaccctcttcagctcagtttctttcaaaatacgaagttgagcttgattgggtgctgtgccactgggagttaatggttccacc

SEQ ID NO: 546 - DNA, 120 bp, Artificial Sequence
  ERBB4
ttcaaaatacgaagttgagcttgattgggtgctgtgccactgggagttaatggttccaccaactgcaaagcggaaagaagaaggttatactttcagtccgatagtcagtcctctctctct

SEQ ID NO: 547 - DNA, 120 bp, Artificial Sequence
  ERBB4
tctaaacctgatgaaaatccccaaacacatgaagaggagaaagaaatacctcacctctgtttccaagaatcttctcaaggctcttttctttttgatgctcttccttctaacataaacagc

SEQ ID NO: 548 - DNA, 120 bp, Artificial Sequence
  ERBB4
ttccaagaatcttctcaaggctcttttctttttgatgctcttccttctaacataaacagcaaatgtcagacccacaatgaccagaatgaagagcccaccaattactccagctgcaatcag

SEQ ID NO: 549 - DNA, 120 bp, Artificial Sequence
  ERBB4
aaatgtcagacccacaatgaccagaatgaagagcccaccaattactccagctgcaatcaggggagttctgacaaccagaatgagaaaaaaaaaaataaaaagtatgaagagagagaagac

SEQ ID NO: 550 - DNA, 120 bp, Artificial Sequence
  ERBB4
atgataactaggaaaggatttgagcgacaaaatggaaacatggtagatgttacctagcatgttgtggtaaagtggaatggcccgtccatgggtagtaaatgcagtcatgactagtgggac

SEQ ID NO: 551 - DNA, 120 bp, Artificial Sequence
  ERBB4
gttgtggtaaagtggaatggcccgtccatgggtagtaaatgcagtcatgactagtgggaccgttacacctgcaggcaattacagaacagaaaacatcattctccatccacagtgacatgc

SEQ ID NO: 552 - DNA, 120 bp, Artificial Sequence
  ERBB4
cacacatgcaccagtgctcacacatggagccttggaggaagaacatgggaagcaagcacaccaagtacctatccatcaggccgatgcagtcttcaatacttgagcctatgcacctgcaga

SEQ ID NO: 553 - DNA, 120 bp, Artificial Sequence
  ERBB4
ccaagtacctatccatcaggccgatgcagtcttcaatacttgagcctatgcacctgcagaaaatgcaaatttaaaaaaatacaaggggaaaaaattagtcatttaaaaaatcagtaaaat

SEQ ID NO: 554 - DNA, 120 bp, Artificial Sequence
  ERBB4
ataacacataccaggtgagcccttggccagcaagaatgcttacccttgggtgcagtttggatggcatgggtggcactcccgatctggatcagcatacttgaaaatgaaactgtttgcccc

SEQ ID NO: 555 - DNA, 120 bp, Artificial Sequence
  ERBB4
atggcatgggtggcactcccgatctggatcagcatacttgaaaatgaaactgtttgccccctgtaagccatctggacatttttccacacagtttgggccatctttaaaatgagagcactt

SEQ ID NO: 556 - DNA, 120 bp, Artificial Sequence
  ERBB4
ctgtaagccatctggacatttttccacacagtttgggccatctttaaaatgagagcactttgtacagttgtcaggaccctgaaatgtgaaaacgaaaaaaaaagaaaaaagaaaagtggt

SEQ ID NO: 557 - DNA, 120 bp, Artificial Sequence
  ERBB4
gatactaaataagccaacacaccacagatgtcttcaggcttaccggtccatggcatgtgaggaggccatcttccatcttctcacactgggggtcacactccacacagatggagccattct

SEQ ID NO: 558 - DNA, 120 bp, Artificial Sequence
  ERBB4
ggaggccatcttccatcttctcacactgggggtcacactccacacagatggagccattctcaaactcccgaaattcactgtgaaaacatcagccacatgaggaggtgtaagcaaacaagc

SEQ ID NO: 559 - DNA, 120 bp, Artificial Sequence
  ERBB4
ctaatcagtccttcaaagctcatgaggtgaaggcaaccctagaagaagccttacccatcatagaggttacaagactctatgcagatccttcctctactgaagcggcgacacgacagacat

SEQ ID NO: 560 - DNA, 120 bp, Artificial Sequence
  ERBB4
tagaggttacaagactctatgcagatccttcctctactgaagcggcgacacgacagacattggtctggcccaggtccccaacagccatcactggaacacagatggttgcacaccattcct

SEQ ID NO: 561 - DNA, 120 bp, Artificial Sequence
  ERBB4
tggtctggcccaggtccccaacagccatcactggaacacagatggttgcacaccattccttcagcagctgtgaaacaccaaaatcaaggggaaataaaacagaggattgtgtcaaaactt

SEQ ID NO: 562 - DNA, 120 bp, Artificial Sequence
  ERBB4
tgtctgagtaatgtacttactacaattttcagcttttctgttgtcccggattactattctctggttgattgtgctgaagagtgttgtccagttaatggtatgataataacacaggttgct

SEQ ID NO: 563 - DNA, 120 bp, Artificial Sequence
  ERBB4
ctggttgattgtgctgaagagtgttgtccagttaatggtatgataataacacaggttgctgttgtcagtaatatagatgtttcctgcgctgatttccttcagggactggaactgtagaga

SEQ ID NO: 564 - DNA, 120 bp, Artificial Sequence
  ERBB4
gttgtcagtaatatagatgtttcctgcgctgatttccttcagggactggaactgtagagaggtgatgccctgttgcttgaggataagcaaggacaggccactaaggagggggaagtgaga

SEQ ID NO: 565 - DNA, 120 bp, Artificial Sequence
  ERBB4
ctcttgaaatctgtgagccctgcagctttaaacatatccacttacctatagagtactcttccaccaatggtcaccaggttagaaaaaacactgaagtcagtcatgtttggtggccatgac

SEQ ID NO: 566 - DNA, 120 bp, Artificial Sequence
  ERBB4
ccaccaatggtcaccaggttagaaaaaacactgaagtcagtcatgtttggtggccatgactgtatgttcaggaaacctacaagtgaagagtagaaaaaataaatcagaatatcattgtct

SEQ ID NO: 567 - DNA, 120 bp, Artificial Sequence
  ERBB4
ttttaaaaaaattatattgttcatagcgcaacagttgcagtttaaaaaattacctgttatctctctgactgtccgaaagacgttcagtttctctgggtctatggcttcaattgcattgta

SEQ ID NO: 568 - DNA, 120 bp, Artificial Sequence
  ERBB4
ctctctgactgtccgaaagacgttcagtttctctgggtctatggcttcaattgcattgtaagggtccctagaaaatcaagaagagatgtagccaaatttaaattttactaaaggattgaa

SEQ ID NO: 569 - DNA, 120 bp, Artificial Sequence
  ERBB4
tctcttcagttttgtctacactttgtaaaataacttgcacaaaaatttaatactgacccatgaataccagtgactagaaagatcaaattcccattgatcttggtacagtttatgaatttg

SEQ ID NO: 570 - DNA, 120 bp, Artificial Sequence
  ERBB4
tgaataccagtgactagaaagatcaaattcccattgatcttggtacagtttatgaatttgtcaatgttactggaatccacagtctgagctgacatcaatgatcctgtgccaatgccatca

SEQ ID NO: 571 - DNA, 120 bp, Artificial Sequence
  ERBB4
tcaatgttactggaatccacagtctgagctgacatcaatgatcctgtgccaatgccatcacaagctgtagaaacaagactcagagttaggggattgagaaacttatttttggccaataaa

SEQ ID NO: 572 - DNA, 120 bp, Artificial Sequence
  ERBB4
agtgaattaaaaaccttgttatataggcccagttctaactaaataatctgagctaccactcaccttttgggcaaatgtcagtgcaaggtttacacattttaatcccattttcttctactt

SEQ ID NO: 573 - DNA, 120 bp, Artificial Sequence
  ERBB4
caccttttgggcaaatgtcagtgcaaggtttacacattttaatcccattttcttctacttccatcttggaactagggcaggcacgcacacaagaactggaatctaccacaaagttatctg

SEQ ID NO: 574 - DNA, 120 bp, Artificial Sequence
  ERBB4
ccatcttggaactagggcaggcacgcacacaagaactggaatctaccacaaagttatctgattaaaaaaaaaaaaaaggtaaaataagcattaatgttaacattcagcaaacaagctcaa

SEQ ID NO: 575 - DNA, 120 bp, Artificial Sequence
  ERBB4
tttcaaataatgacctaattaatttggttattcttattctgttacttacgtggacatttcttgacacagaatgctccatatgtgtactttgcattgaaattgtgctccagttgaaaggtg

SEQ ID NO: 576 - DNA, 120 bp, Artificial Sequence
  ERBB4
ttgacacagaatgctccatatgtgtactttgcattgaaattgtgctccagttgaaaggtggttggattgtagacaaaggtttggggacactgagtaacacatgctccactgtcattgaaa

SEQ ID NO: 577 - DNA, 120 bp, Artificial Sequence
  ERBB4
gttggattgtagacaaaggtttggggacactgagtaacacatgctccactgtcattgaaattcatgcaggcctgcaacacagcaaatattactttcatttacaaataaactcataatact

SEQ ID NO: 578 - DNA, 120 bp, Artificial Sequence
  ERBB4
ctgaatcaaatagggaaggaaaggagagcaggataataaaagagagaaatcacagacatacaaagcagtctgtgtccttaggtcctgagcagcctccagcacattctcgatggcagcagt

SEQ ID NO: 579 - DNA, 120 bp, Artificial Sequence
  ERBB4
caaagcagtctgtgtccttaggtcctgagcagcctccagcacattctcgatggcagcagtcactgacgtaaggtccgtagcatctgccgtcacattgttctgcacacaccgtccttgtca

SEQ ID NO: 580 - DNA, 120 bp, Artificial Sequence
  ERBB4
cactgacgtaaggtccgtagcatctgccgtcacattgttctgcacacaccgtccttgtcactgcagaagacagagataggaccatgatcaaagtctgccaccaggagaaactcataagct

SEQ ID NO: 581 - DNA, 120 bp, Artificial Sequence
  ERBB4
atcattaaaattccttgaccacatcaaacctgtgtgctctcactgatgaacacttacaagtctggcaatgattttctgtgggtccccagcaacggccagtacaggacttatggcaacgtc

SEQ ID NO: 582 - DNA, 120 bp, Artificial Sequence
  ERBB4
tctggcaatgattttctgtgggtccccagcaacggccagtacaggacttatggcaacgtccacctgcagaacacgaaaagggaaaaaggacatgcacgttataatctttcactccttgac

SEQ ID NO: 583 - DNA, 120 bp, Artificial Sequence
  ERBB4
tcgccacatagggtagaacattttgagaaattaaaaagaataattctacttacatcctgaactaccatttgttgacacaagagtcaagttggaaggccatgggttccgaacaatatcttg

SEQ ID NO: 584 - DNA, 120 bp, Artificial Sequence
  ERBB4
actaccatttgttgacacaagagtcaagttggaaggccatgggttccgaacaatatcttgccaatgaatggtgtctgcataacaaaggaatttgttctggtctacatagactccaccatt

SEQ ID NO: 585 - DNA, 120 bp, Artificial Sequence
  ERBB4
ccaatgaatggtgtctgcataacaaaggaatttgttctggtctacatagactccaccatttaggatttctgtattaaaaaacaaataaacaaattttttgtcaaactgcttgttgatgaa

SEQ ID NO: 586 - DNA, 120 bp, Artificial Sequence
  ERBB4
atttgccattttggatatattccttacctgtcaagttctttaatccaagttcttgaagtccaaagtttccatcttttctgtagtttaaaaatattgccaaggcatatcgatcctcataaa

SEQ ID NO: 587 - DNA, 120 bp, Artificial Sequence
  ERBB4
caaagtttccatcttttctgtagtttaaaaatattgccaaggcatatcgatcctcataaagttttgtcccacgaataatgcgtaaattctccagaggcaggtaacgaaactgattaagag

SEQ ID NO: 588 - DNA, 120 bp, Artificial Sequence
  ERBB4
gttttgtcccacgaataatgcgtaaattctccagaggcaggtaacgaaactgattaagagccactaacacgtagcctgtgacttctcgaacagactgaaaagacacaaacagttgcctgt

SEQ ID NO: 589 - DNA, 120 bp, Artificial Sequence
  ERBB4
ccactgtccattcacaaagaagagaaagaaagccacagctttacccgcaggaaggagaggtcccggttgtgctcaatgctggttatctccaggttgcccatgacaacctcacagttttca

SEQ ID NO: 590 - DNA, 120 bp, Artificial Sequence
  ERBB4
tcccggttgtgctcaatgctggttatctccaggttgcccatgacaacctcacagttttcatagtacttgcgcaaggctcggtactgctgttccaggtcagagagagagctcagtttattc

SEQ ID NO: 591 - DNA, 120 bp, Artificial Sequence
  ERBB4
tagtacttgcgcaaggctcggtactgctgttccaggtcagagagagagctcagtttattctccgttcctgcacacactgcaaagacaagaagatacacgtgaaattacataacctttata

SEQ ID NO: 592 - DNA, 120 bp, Artificial Sequence
  ERBB4
cccgccggcggctgcaggttcggcgaccggagtgccagaaggaacccacctgactgagaatcgctgggctggacggtccccgccgccacgagaaggctcacccagacccaaagtcctgtc

SEQ ID NO: 593 - DNA, 120 bp, Artificial Sequence
  ERBB4
tcgctgggctggacggtccccgccgccacgagaaggctcacccagacccaaagtcctgtcgccggcttcattttttggaagtctcagatcccgtgctgacaattacatgtccaaatggca

SEQ ID NO: 594 - DNA, 120 bp, Artificial Sequence
  HER2-E20
gtttgggggtgtgtggtctcccataccctctcagcgtacccttgtccccaggaagcatacgtgatggctggtgtgggctccccatatgtctcccgccttctgggcatctgcctgacatcc

SEQ ID NO: 595 - DNA, 120 bp, Artificial Sequence; identical to SEQ ID NO: 486
  HER2-E20

SEQ ID NO: 596 - DNA, 120 bp, Artificial Sequence
  HER2-E20
gtgggctccccatatgtctcccgccttctgggcatctgcctgacatccacggtgcagctggtgacacagcttatgccctatggctgcctcttagaccatgtccgggaaaaccgcggacgc

SEQ ID NO: 597 - DNA, 120 bp, Artificial Sequence
  HER2-E20
cttctgggcatctgcctgacatccacggtgcagctggtgacacagcttatgccctatggctgcctcttagaccatgtccgggaaaaccgcggacgcctgggctcccaggacctgctgaac

SEQ ID NO: 598 - DNA, 120 bp, Artificial Sequence; identical to SEQ ID NO: 488
  HER2-E20

SEQ ID NO: 599 - DNA, 120 bp, Artificial Sequence
  HER2-E20
catgtccgggaaaaccgcggacgcctgggctcccaggacctgctgaactggtgtatgcagattgccaaggtatgcacctgggctctttgcaggtctctccggagcaaacccctatgtcca

SEQ ID NO: 600 - DNA, 120 bp, Artificial Sequence
  HER4-E10
atattgttcatagcgcaacagttgcagtttaaaaaattacctgttatctctctgactgtccgaaagacgttcagtttctctgggtctatggcttcaattgcattgtaagggtccctagaa

SEQ ID NO: 601 - DNA, 120 bp, Artificial Sequence
  HER4-E10
tctctgactgtccgaaagacgttcagtttctctgggtctatggcttcaattgcattgtaagggtccctagaaaatcaagaagagatgtagccaaatttaaattttactaaaggattgaaa

SEQ ID NO: 602 - DNA, 120 bp, Artificial Sequence
  HER4-E10
agtttctctgggtctatggcttcaattgcattgtaagggtccctagaaaatcaagaagagatgtagccaaatttaaattttactaaaggattgaaaatatgagaaatgtgacaatatttt

SEQ ID NO: 603 - DNA, 120 bp, Artificial Sequence; identical to SEQ ID NO: 600
  HER4-E10

SEQ ID NO: 604 - DNA, 120 bp, Artificial Sequence; identical to SEQ ID NO: 45
  HER4-E10

SEQ ID NO: 605 - DNA, 120 bp, Artificial Sequence; identical to SEQ ID NO: 601
  HER4-E10

SEQ ID NO: 606 - DNA, 120 bp, Artificial Sequence; identical to SEQ ID NO: 602
  HER4-E10

SEQ ID NO: 607 - DNA, 120 bp, Artificial Sequence
  HER4-E12
aagaatgggaaaaaatttaagtttctatgttttaaatgtctgagtaatgtacttactacaattttcagcttttctgttgtcccggattactattctctggttgattgtgctgaagagtgt

SEQ ID NO: 608 - DNA, 120 bp, Artificial Sequence
  HER4-E12
ctatgttttaaatgtctgagtaatgtacttactacaattttcagcttttctgttgtcccggattactattctctggttgattgtgctgaagagtgttgtccagttaatggtatgataata

SEQ ID NO: 609 - DNA, 120 bp, Artificial Sequence
  HER4-E12
tctgttgtcccggattactattctctggttgattgtgctgaagagtgttgtccagttaatggtatgataataacacaggttgctgttgtcagtaatatagatgtttcctgcgctgatttc

SEQ ID NO: 610 - DNA, 120 bp, Artificial Sequence; identical to SEQ ID NO: 563
  HER4-E12

SEQ ID NO: 611 - DNA, 120 bp, Artificial Sequence
  HER4-E12
tgtccagttaatggtatgataataacacaggttgctgttgtcagtaatatagatgtttcctgcgctgatttccttcagggactggaactgtagagaggtgatgccctgttgcttgaggat

SEQ ID NO: 612 - DNA, 120 bp, Artificial Sequence
  HER4-E12
atagatgtttcctgcgctgatttccttcagggactggaactgtagagaggtgatgccctgttgcttgaggataagcaaggacaggccactaaggagggggaagtgagaaaacggaaccat

SEQ ID NO: 613 - DNA, 120 bp, Artificial Sequence
  HER4-E12
cttcagggactggaactgtagagaggtgatgccctgttgcttgaggataagcaaggacaggccactaaggagggggaagtgagaaaacggaaccatgaaacgcattccggagtaaaataa

SEQ ID NO: 614 - DNA, 120 bp, Artificial Sequence; identical to SEQ ID NO: 607
  HER4-E12

SEQ ID NO: 615 - DNA, 120 bp, Artificial Sequence; identical to SEQ ID NO: 608
  HER4-E12

SEQ ID NO: 616 - DNA, 120 bp, Artificial Sequence; identical to SEQ ID NO: 46
  HER4-E12

SEQ ID NO: 617 - DNA, 120 bp, Artificial Sequence; identical to SEQ ID NO: 609
  HER4-E12

SEQ ID NO: 618 - DNA, 120 bp, Artificial Sequence; identical to SEQ ID NO: 563
  HER4-E12

SEQ ID NO: 619 - DNA, 120 bp, Artificial Sequence; identical to SEQ ID NO: 611
  HER4-E12

SEQ ID NO: 620 - DNA, 120 bp, Artificial Sequence; identical to SEQ ID NO: 47
  HER4-E12

SEQ ID NO: 621 - DNA, 120 bp, Artificial Sequence; identical to SEQ ID NO: 612
  HER4-E12

SEQ ID NO: 622 - DNA, 120 bp, Artificial Sequence; identical to SEQ ID NO: 613
  HER4-E12

SEQ ID NO: 623 - DNA, 120 bp, Artificial Sequence
  KDR
catgtgatgtccaggagttgggggtgtggatgcttccttttaaacaggaggagagctcagtgtggtccccgagtcaggctggagaatctgggctgtgctaccggtttgcactccaatctc

SEQ ID NO: 624 - DNA, 120 bp, Artificial Sequence
  KDR
tgtggtccccgagtcaggctggagaatctgggctgtgctaccggtttgcactccaatctctatcagctttaaaagttctgcttcctcactggagtacacggtggtgtctgtgtcatcgga

SEQ ID NO: 625 - DNA, 120 bp, Artificial Sequence
  KDR
tatcagctttaaaagttctgcttcctcactggagtacacggtggtgtctgtgtcatcggagtgatatccggactggtagccgcttgtctggtttgagccttcagatgccacagactccct

SEQ ID NO: 626 - DNA, 120 bp, Artificial Sequence
  KDR
gtgatatccggactggtagccgcttgtctggtttgagccttcagatgccacagactccctgcttttgctgggcaccattccactgcagaagaaatggcaaacaaaggagttggcagagag

SEQ ID NO: 627 - DNA, 120 bp, Artificial Sequence
  KDR
caaaaattcctattgaaatttgtctttttaatatggctgagtcttacccaaaagatggagataatttggttctgtcttccaaagttttcagctcttctgaggcaagaaccataccactgt

SEQ ID NO: 628 - DNA, 120 bp, Artificial Sequence
  KDR
ataatttggttctgtcttccaaagttttcagctcttctgaggcaagaaccataccactgtccgtctggttgtcctttttaagagacaatgagatggcacagttaattgagcatataaaat

SEQ ID NO: 629 - DNA, 120 bp, Artificial Sequence
  KDR
ttgtattatttctaagactatttttaaaagacgtacttacatctgggattacttttacttctggttcttctaacgggatatcttcaaatgtttttacactcacaggccggctctttcgct

SEQ ID NO: 630 - DNA, 120 bp, Artificial Sequence
  KDR
ctggttcttctaacgggatatcttcaaatgtttttacactcacaggccggctctttcgcttactgttctgcagatactgactgcaaaagaacaaatatttatattttagtggtggtatat

SEQ ID NO: 631 - DNA, 120 bp, Artificial Sequence
  KDR
ttgaagtcaccctcccccgggggatgttaggccatatacagtacctgattcctgctgtgttgtcataatggaatttggggtcacatacttcctcctcctccatacaggaaacaggtgagg

SEQ ID NO: 632 - DNA, 120 bp, Artificial Sequence
  KDR
tgtcataatggaatttggggtcacatacttcctcctcctccatacaggaaacaggtgaggtaggcagagagagtccagaatcctcttccatgctcaaagtctctgatatcggaagaacaa

SEQ ID NO: 633 - DNA, 120 bp, Artificial Sequence
  KDR
taggcagagagagtccagaatcctcttccatgctcaaagtctctgatatcggaagaacaatgtagtctttgccatcctgaaacaataaacacagaagactgttgttatggcttcagttct

SEQ ID NO: 634 - DNA, 120 bp, Artificial Sequence
  KDR
aggcagtaggaaagtccttgacatctaagtactctttgtaggtgcttcttggatggaggtgacaaacctgctgagcattagcttgcaagagatttcccaaatgttccaccaactctgaaa

SEQ ID NO: 635 - DNA, 120 bp, Artificial Sequence
  KDR
gacaaacctgctgagcattagcttgcaagagatttcccaaatgttccaccaactctgaaaacgtgggtctctgactgggctccccgtgccagcagtccagcatggtctggtacctagaga

SEQ ID NO: 636 - DNA, 120 bp, Artificial Sequence
  KDR
acgtgggtctctgactgggctccccgtgccagcagtccagcatggtctggtacctagagaagcaaaacactgatttcattaaatgcctctttcttcctgaatgctgaaaataagcactta

SEQ ID NO: 637 - DNA, 120 bp, Artificial Sequence
  KDR
gcaaagaaagagaacacaggaatacttcttaaagtcttacatttctggtgtagtataatcaggggccctcattctagttccttctttcaatcgcctacaaaattcttcatcaatctttac

SEQ ID NO: 638 - DNA, 120 bp, Artificial Sequence
  KDR
aggggccctcattctagttccttctttcaatcgcctacaaaattcttcatcaatctttaccccaggatatggagaagcacctagaataaaacagggaggagacattctttgatttgattt

SEQ ID NO: 639 - DNA, 120 bp, Artificial Sequence
  KDR
ggaaaagacaacttttgtcttcctctttggagtctggatggaaggacaaaaagaaatgacttacctaaggaaaatatttcccacagcaaaacaccaaaagaccagacgtcactctggatt

SEQ ID NO: 640 - DNA, 120 bp, Artificial Sequence
  KDR
ttacctaaggaaaatatttcccacagcaaaacaccaaaagaccagacgtcactctggattgtgtacactctgtcaaaaattgtttctggggccatccatttcaaagggaggcgagcctac

SEQ ID NO: 641 - DNA, 120 bp, Artificial Sequence
  KDR
gtgtacactctgtcaaaaattgtttctggggccatccatttcaaagggaggcgagcctacaggggtagaagacaaggattcagaacccaaattagcaaatatctgaagaaaaaaacttcc

SEQ ID NO: 642 - DNA, 120 bp, Artificial Sequence
  KDR
ctacgaggagttttaattctgttacttaaccaagcactgggttcatatttgaaacttacatctccttttctgacataatctggatctttataaatatcccgggccaagccaaagtcacag

SEQ ID NO: 643 - DNA, 120 bp, Artificial Sequence
  KDR
tctccttttctgacataatctggatctttataaatatcccgggccaagccaaagtcacagattttaaccacgttcttctccgataagaggatatttcgtgccgccaggtccctgtggata

SEQ ID NO: 644 - DNA, 120 bp, Artificial Sequence
  KDR
attttaaccacgttcttctccgataagaggatatttcgtgccgccaggtccctgtggatacactgcaaagagaatcatgtgtgcattaggtctcggcacagctgatctctttcacatctg

SEQ ID NO: 645 - DNA, 120 bp, Artificial Sequence
  KDR
tgatctgaaaagatagctgatttcccctcaacctttcttacctttcgcgatgccaagaactccatgcccttagccacttggaagctgtaacagatgagatgctccaaggtcaggaagtcc

SEQ ID NO: 646 - DNA, 120 bp, Artificial Sequence
  KDR
tccatgcccttagccacttggaagctgtaacagatgagatgctccaaggtcaggaagtccttatacagatcttcaggagctgtccaaagaggcaggaggatggagatcagtatttccatg

SEQ ID NO: 647 - DNA, 120 bp, Artificial Sequence
  KDR
tgacaagagcatgccatagcatgcaggaagcactagccagtaccttcctcttcttctacatcactgagggacttctcctccacaaatccagagctggctgagctctggctactggtgatg

SEQ ID NO: 648 - DNA, 120 bp, Artificial Sequence
  KDR
tcactgagggacttctcctccacaaatccagagctggctgagctctggctactggtgatgctgtccaagcgccgtttcagatccacagggattgctccaacgtagtctttcccttgacgg

SEQ ID NO: 649 - DNA, 120 bp, Artificial Sequence
  KDR
ctgtccaagcgccgtttcagatccacagggattgctccaacgtagtctttcccttgacggaatcgtgcccctttggtctataaaaaagcaaaggaacaaacaaactccttgaatacaaaa

SEQ ID NO: 650 - DNA, 120 bp, Artificial Sequence
  KDR
ccttcattttataacatggccagagcaggattaggagatgacataccttgtaggggacaaattcatttctcttgctcctcaggtaagtggacaggtttccaaatttgcagaattccacaa

SEQ ID NO: 651 - DNA, 120 bp, Artificial Sequence
  KDR
attcatttctcttgctcctcaggtaagtggacaggtttccaaatttgcagaattccacaatcaccatgagtggccctgcaggcagcatgtccaggaaggaaaatgggttttcactcatat

SEQ ID NO: 652 - DNA, 120 bp, Artificial Sequence
  KDR
cctcaaacactatcagagaggcatgttaaaattgggtgaccaaaaccacccacagttactcacctcctggcttggtacaggcacctagaaggttgaccacattgagatggtgaccaatat

SEQ ID NO: 653 - DNA, 120 bp, Artificial Sequence
  KDR
cacctcctggcttggtacaggcacctagaaggttgaccacattgagatggtgaccaatatgaatgaggatcttgagttcagacatgagagctcgatgctcactgtgtgttgctccttcta

SEQ ID NO: 654 - DNA, 120 bp, Artificial Sequence
  KDR
gaatgaggatcttgagttcagacatgagagctcgatgctcactgtgtgttgctccttctacaaatacagtacaaagagggaaatcataggtatggacatttccttcaataattggggtcc

SEQ ID NO: 655 - DNA, 120 bp, Artificial Sequence
  KDR
aagccttgcaacatatttaaagactagataaaacagaaagatagatcaccacataattttgcttttacctttcaacattttgactgctactgtcctgcaagttgctgtcttgtcaattcc

SEQ ID NO: 656 - DNA, 120 bp, Artificial Sequence
  KDR
gcttttacctttcaacattttgactgctactgtcctgcaagttgctgtcttgtcaattccaaaggcatctgcttcaatcacttggccaaaggcaccacggccaagaggcttacctagagt

SEQ ID NO: 657 - DNA, 120 bp, Artificial Sequence
  KDR
aaaggcatctgcttcaatcacttggccaaaggcaccacggccaagaggcttacctagagtcaacaacaacagcaacaagaaaacagacttggattactatacaaccaaagtgatacgcag

SEQ ID NO: 658 - DNA, 120 bp, Artificial Sequence
  KDR
aagagatggcctggtaaacacaatatcaaattaatagcaattgaaaatgcacctagcttcagccggtctctggggaattcccatttgctggcatcataaggcagtcgttcacaatgttca

SEQ ID NO: 659 - DNA, 120 bp, Artificial Sequence
  KDR
agccggtctctggggaattcccatttgctggcatcataaggcagtcgttcacaatgttcatccaatgggagttcatctggatccatgacgatggacaagtagcctgtcttcagttcccct

SEQ ID NO: 660 - DNA, 120 bp, Artificial Sequence
  KDR
tccaatgggagttcatctggatccatgacgatggacaagtagcctgtcttcagttcccctccattggcctggaaagcatcaatccttccagtcataaacacactgttgtttggctgttgt

SEQ ID NO: 661 - DNA, 120 bp, Artificial Sequence
  KDR
accccagtcagttttcattaatcatgaaaaccaatgtgcatgggcagaagggaaattatttttttacccgcttaacggtccgtaggatgatgacaagaagtagccagaagaacatggcaa

SEQ ID NO: 662 - DNA, 120 bp, Artificial Sequence
  KDR
tttttacccgcttaacggtccgtaggatgatgacaagaagtagccagaagaacatggcaatcaccgccgtgcctactagaataatgatttccaagttcgtcttttcctgggcacctggaa

SEQ ID NO: 663 - DNA, 120 bp, Artificial Sequence
  KDR
tcaccgccgtgcctactagaataatgatttccaagttcgtcttttcctgggcacctggaaagacacaattgaatgagtatcaacagttggaaacttatactttttgtttgtaagatgaca

SEQ ID NO: 664 - DNA, 120 bp, Artificial Sequence
  KDR
accacatttttttttatcccactgaccttctattatgaaaaatgcctccacttttgcacagccaagaacactgcatgcctggcaggtgtagaggccttcgtcctccttcctcactctgcg

SEQ ID NO: 665 - DNA, 120 bp, Artificial Sequence
  KDR
gccaagaacactgcatgcctggcaggtgtagaggccttcgtcctccttcctcactctgcggatagtgaggttccggttcccatccttcaatacaatgcctaacagaggaagaaaacgatc

SEQ ID NO: 666 - DNA, 120 bp, Artificial Sequence
  KDR
gatagtgaggttccggttcccatccttcaatacaatgcctaacagaggaagaaaacgatcattctcatttatgatgatgtagtctgtgaagtttttcagggaaatttagaaaatataaat

SEQ ID NO: 667 - DNA, 120 bp, Artificial Sequence
  KDR
cctgggaaagttctgcaacccaagagtgatagccaaattctatttacctgagtcttctacaagggtctcattatctttaaaccacatgatctgtggagggggattcccagatgccgtgca

SEQ ID NO: 668 - DNA, 120 bp, Artificial Sequence
  KDR
aagggtctcattatctttaaaccacatgatctgtggagggggattcccagatgccgtgcatgagacttcgatgctttccccaatacttgtcgtctgattctccaggtttcctgtgatcgt

SEQ ID NO: 669 - DNA, 120 bp, Artificial Sequence
  KDR
tgagacttcgatgctttccccaatacttgtcgtctgattctccaggtttcctgtgatcgtgggtgccacacgctctagacacacaaaaagaaaatcacagaacatggaattataactttt

SEQ ID NO: 670 - DNA, 120 bp, Artificial Sequence
  KDR
caactgcctctgcacaatgatccagaattgtctccctacctaggactgtgagctgcctgaccacgcaatgtcttttcttggtcttcctgtcttgagcaaggcagacatagtctccttggt

SEQ ID NO: 671 - DNA, 120 bp, Artificial Sequence
  KDR
ccacgcaatgtcttttcttggtcttcctgtcttgagcaaggcagacatagtctccttggtcctgcaaggatgcattcttaagctccatgatcaaaatgtcatttgtgctattagagaaca

SEQ ID NO: 672 - DNA, 120 bp, Artificial Sequence
  KDR
cctgcaaggatgcattcttaagctccatgatcaaaatgtcatttgtgctattagagaacatggtggcattcaatttccaaagagtatccaagttcttgcaaacaggtgtgggcaactctc

SEQ ID NO: 673 - DNA, 120 bp, Artificial Sequence
  KDR
tggtggcattcaatttccaaagagtatccaagttcttgcaaacaggtgtgggcaactctcccacatggattggcagaggctgtgggccaagcttgtaccatgtgaggttctcaaacgtag

SEQ ID NO: 674 - DNA, 120 bp, Artificial Sequence
  KDR
ccacatggattggcagaggctgtgggccaagcttgtaccatgtgaggttctcaaacgtagatctgtctgcagtgcaccacaaagacacgctctcctgctcagtgggctgcatgtcaggtt

SEQ ID NO: 675 - DNA, 120 bp, Artificial Sequence
  KDR
atctgtctgcagtgcaccacaaagacacgctctcctgctcagtgggctgcatgtcaggttgcaaagtaatttcaggaccccctaaaatgaagaggccatagttattgaatggtgatttaa

SEQ ID NO: 676 - DNA, 120 bp, Artificial Sequence
  KDR
gaattacatagcttagtacccactgtgtgagtgatccaacccaaacctccagagaagagtacttactggtcacgtggaaggagatcaccctctctcctctcccgactttgttgaccgctt

SEQ ID NO: 677 - DNA, 120 bp, Artificial Sequence
  KDR
acttactggtcacgtggaaggagatcaccctctctcctctcccgactttgttgaccgcttcacatttgtacaaagctgacacatttgccgcttggataacaagggtacttacagtctgtg

SEQ ID NO: 678 - DNA, 120 bp, Artificial Sequence
  KDR
cacatttgtacaaagctgacacatttgccgcttggataacaagggtacttacagtctgtgcggggaaaaaacaaatcccaggccataaacaacgcggctgtttgtgcacaagcactcagt

SEQ ID NO: 679 - DNA, 120 bp, Artificial Sequence; identical to SEQ ID NO: 127
  KDR

SEQ ID NO: 680 - DNA, 120 bp, Artificial Sequence
  KDR
tgttttttccttcaattagagcaaattgatttttattaacttcaattttatttcctccctggaagtcctccacacttctccattcttcacaagggtatgggtttgtcactgagacagctt

SEQ ID NO: 681 - DNA, 120 bp, Artificial Sequence; identical to SEQ ID NO: 131
  KDR

SEQ ID NO: 682 - DNA, 120 bp, Artificial Sequence
  KDR
tgcaagatggcaggaaagcaaagagcatgtggccttactcacctgggctcgttggcgcactcttcctccaactgccaataccagtggatgtgatgcgggggaggaatggcatagaccgta

SEQ ID NO: 683 - DNA, 120 bp, Artificial Sequence
  KDR
tcttcctccaactgccaataccagtggatgtgatgcgggggaggaatggcatagaccgtacatgtcagcgtttgagtggtgccgtactggtaggaatccacaggagagattagagatttc

SEQ ID NO: 684 - DNA, 120 bp, Artificial Sequence
  KDR
catgtcagcgtttgagtggtgccgtactggtaggaatccacaggagagattagagatttctcaccaatctggggtgggactgaagatgggaaaaacaacttttgaattgtcagtcagctt

SEQ ID NO: 685 - DNA, 120 bp, Artificial Sequence
  KDR
ataaatcttgggcagagaggaaaattgaatggactcaccatacacaaccagagagaccacatggctctgcttctcctttgaaatgggattggtaaggatgacagtgtaatttcctgtgtc

SEQ ID NO: 686 - DNA, 120 bp, Artificial Sequence
  KDR
atggctctgcttctcctttgaaatgggattggtaaggatgacagtgtaatttcctgtgtctctttcactcacttccataatcgtcagtacatgccccgctttaattgtgtgattggactc

SEQ ID NO: 687 - DNA, 120 bp, Artificial Sequence
  KDR
tctttcactcacttccataatcgtcagtacatgccccgctttaattgtgtgattggactcaaggggtattccatttttatacctatgaaaaaaaattctcaggaattagtatagtcaaag

SEQ ID NO: 688 - DNA, 120 bp, Artificial Sequence
  KDR
tagtatagtcaaaggatttgctctcacacgaaatgatgctttgcatttatttccagtagttaccattttatttctgggggtgggtaaccaaggtacttcgcagggattctgacacgctcc

SEQ ID NO: 689 - DNA, 120 bp, Artificial Sequence
  KDR
taccattttatttctgggggtgggtaaccaaggtacttcgcagggattctgacacgctcccccaccgtggcttccaccagagattccatgccacttccaaaagcaacaaaaggtttttct

SEQ ID NO: 690 - DNA, 120 bp, Artificial Sequence
  KDR
cccaccgtggcttccaccagagattccatgccacttccaaaagcaacaaaaggtttttctggaagaaaataaaaaaaaaaaaaggtcaacttactgtaaatggtcatttgatttagtttt

SEQ ID NO: 691 - DNA, 120 bp, Artificial Sequence
  KDR
gcacagaataatttccaagaccatagcttaccatggaccctgacaaatgtgctgttcttcttggtcatcagcccactggatgctgcacaggtgtacaatccttggtcactccgggttaca

SEQ ID NO: 692 - DNA, 120 bp, Artificial Sequence
  KDR
ttggtcatcagcccactggatgctgcacaggtgtacaatccttggtcactccgggttacaccatctatagttaaggtgctcaaaaatttcttcatctcactcccagactgggtttttagg

SEQ ID NO: 693 - DNA, 120 bp, Artificial Sequence
  KDR
ccatctatagttaaggtgctcaaaaatttcttcatctcactcccagactgggtttttaggtctcggtttacaagtttcttatgctgatgctgaaaaaaagagttgactgaacttccaaag

SEQ ID NO: 694 - DNA, 120 bp, Artificial Sequence
  KDR
ggcttattatctaagtatttggaggtctggctttgaatcattagcgttaccttcgaagaagggtattcccagttgaagtcaatccccacatttagttcagttcttgctgtacaatttaag

SEQ ID NO: 695 - DNA, 120 bp, Artificial Sequence
  KDR
gggtattcccagttgaagtcaatccccacatttagttcagttcttgctgtacaatttaagacaagcttttctccaacagatagttcaattccatgagacggactcagaaccacatcataa

SEQ ID NO: 696 - DNA, 120 bp, Artificial Sequence
  KDR
acaagcttttctccaacagatagttcaattccatgagacggactcagaaccacatcataaatcctataccctagagcaagtaaattgaaaaaacagaacatgagagagcaaataagccta

SEQ ID NO: 697 - DNA, 120 bp, Artificial Sequence
  KDR
tgttattaatgatatggaaaggaaatgtcctcttacctacaacgacaactatgtacataatagactggtaactttcatcattaatttttgcttcacagaagaccatgccagcatagctga

SEQ ID NO: 698 - DNA, 120 bp, Artificial Sequence
  KDR
tagactggtaactttcatcattaatttttgcttcacagaagaccatgccagcatagctgatcatgtagctgggaatagtaaagcccttcttgctgtcccaggaaattctgttaccatcag

SEQ ID NO: 699 - DNA, 120 bp, Artificial Sequence
  KDR
tcatgtagctgggaatagtaaagcccttcttgctgtcccaggaaattctgttaccatcaggaacaaatctcttttctgggtatctctgggtaataaaaagacatatcaaatatttaatcc

SEQ ID NO: 700 - DNA, 120 bp, Artificial Sequence
  KDR
atattagcttaaaattataaaaacttaagagacgattggaggagatgcaacttactgcacaaagtgacacgttgagatttgaaatggacccgagacatggaatcaccacagttttgtttt

SEQ ID NO: 701 - DNA, 120 bp, Artificial Sequence
  KDR
aaagtgacacgttgagatttgaaatggacccgagacatggaatcaccacagttttgtttttgttctcagtaatgtacacgactccatgttggtcactaacagaagcaataaatggagatc

SEQ ID NO: 702 - DNA, 120 bp, Artificial Sequence
  KDR
tgttctcagtaatgtacacgactccatgttggtcactaacagaagcaataaatggagatctgtaatctagaagaaaatttagttttattaatgagttaatagtatttactagaaaagttg

SEQ ID NO: 703 - DNA, 120 bp, Artificial Sequence
  KDR
tgaattttatttcaccacttaccttgaacatagacataaatgaccgaggccaagtcagtttcccggtagaagcacttgtaggctccagtgtcatttccgatcacttttggaattgtgagt

SEQ ID NO: 704 - DNA, 120 bp, Artificial Sequence
  KDR
tcccggtagaagcacttgtaggctccagtgtcatttccgatcacttttggaattgtgagtgtcttacagaagaggccatcgctgcactcagtcacctccaccctttgctcactgccactc

SEQ ID NO: 705 - DNA, 120 bp, Artificial Sequence
  KDR
gtcttacagaagaggccatcgctgcactcagtcacctccaccctttgctcactgccactctgattattgggccaaagccagtccaagtccctctgtcccctgaaaaattaatttcaggga

SEQ ID NO: 706 - DNA, 120 bp, Artificial Sequence
  KDR
agttacttaacacaagaaatctagatctagaatgaatccttacctgcaagtaatttgaagagttgtattagccttaattgtaagtatgtctttttgtatgctgagcctgggcagatcaag

SEQ ID NO: 707 - DNA, 120 bp, Artificial Sequence
  KDR
agttgtattagccttaattgtaagtatgtctttttgtatgctgagcctgggcagatcaagagaaacactaggcaaacctagaaacaaattaaataaatgaatgtagttgccactgagtta

SEQ ID NO: 708 - DNA, 120 bp, Artificial Sequence
  KDR
gtcctctccgccctcacccgacctgtctgccttcctcctccagagtgggctccttacccacagaggcggcccgggtctccacgcagagccacagggcgacggccagcagcaccttgctct

SEQ ID NO: 709 - DNA, 120 bp, Artificial Sequence
  KDR
cagaggcggcccgggtctccacgcagagccacagggcgacggccagcagcaccttgctctgcatcctgcacctcgagccgggcgaaatgcccagaactcgggagccggttctttctccca

SEQ ID NO: 710 - DNA, 120 bp, Artificial Sequence
  KIT
cacttgggcgagagctggaacgtggaccagagctcggatcccatcgcagctaccgcgatgagaggcgctcgcggcgcctgggattttctctgcgttctgctcctactgcttcgcgtccag

SEQ ID NO: 711 - DNA, 120 bp, Artificial Sequence
  KIT
agaggcgctcgcggcgcctgggattttctctgcgttctgctcctactgcttcgcgtccagacaggtgggacaccgcggctggcaccccgaccgtgcgactactcggcgaagcctgtgcct

SEQ ID NO: 712 - DNA, 120 bp, Artificial Sequence
  KIT
tgtttttcttggcaggctcttctcaaccatctgtgagtccaggggaaccgtctccaccatccatccatccaggaaaatcagacttaatagtccgcgtgggcgacgagattaggctgttat

SEQ ID NO: 713 - DNA, 120 bp, Artificial Sequence
  KIT
ccatccatccaggaaaatcagacttaatagtccgcgtgggcgacgagattaggctgttatgcactgatccgggctttgtcaaatggacttttgagatcctggatgaaacgaatgagaata

SEQ ID NO: 714 - DNA, 120 bp, Artificial Sequence
  KIT
gcactgatccgggctttgtcaaatggacttttgagatcctggatgaaacgaatgagaataagcagaatgaatggatcacggaaaaggcagaagccaccaacaccggcaaatacacgtgca

SEQ ID NO: 715 - DNA, 120 bp, Artificial Sequence
  KIT
agcagaatgaatggatcacggaaaaggcagaagccaccaacaccggcaaatacacgtgcaccaacaaacacggcttaagcaattccatttatgtgtttgttagaggtaaatgcttggctt

SEQ ID NO: 716 - DNA, 120 bp, Artificial Sequence
  KIT
cagccattccaactactgattttggatatgcttctatagatcctgccaagcttttccttgttgaccgctccttgtatgggaaagaagacaacgacacgctggtccgctgtcctctcacag

SEQ ID NO: 717 - DNA, 120 bp, Artificial Sequence
  KIT
ttgaccgctccttgtatgggaaagaagacaacgacacgctggtccgctgtcctctcacagacccagaagtgaccaattattccctcaaggggtgccaggggaagcctcttcccaaggact

SEQ ID NO: 718 - DNA, 120 bp, Artificial Sequence
  KIT
acccagaagtgaccaattattccctcaaggggtgccaggggaagcctcttcccaaggacttgaggtttattcctgaccccaaggcgggcatcatgatcaaaagtgtgaaacgcgcctacc

SEQ ID NO: 719 - DNA, 120 bp, Artificial Sequence
  KIT
tgaggtttattcctgaccccaaggcgggcatcatgatcaaaagtgtgaaacgcgcctaccatcggctctgtctgcattgttctgtggaccaggagggcaagtcagtgctgtcggaaaaat

SEQ ID NO: 720 - DNA, 120 bp, Artificial Sequence
  KIT
atcggctctgtctgcattgttctgtggaccaggagggcaagtcagtgctgtcggaaaaattcatcctgaaagtgaggccaggtactggctctttcttatctgcctctgggagttgagaac

SEQ ID NO: 721 - DNA, 120 bp, Artificial Sequence
  KIT
tttcatgctataatacaaattatttgaggggccacatttcttttcattctagccttcaaagctgtgcctgttgtgtctgtgtccaaagcaagctatcttcttagggaaggggaagaattc

SEQ ID NO: 722 - DNA, 120 bp, Artificial Sequence
  KIT
gctgtgcctgttgtgtctgtgtccaaagcaagctatcttcttagggaaggggaagaattcacagtgacgtgcacaataaaagatgtgtctagttctgtgtactcaacgtggaaaagagaa

SEQ ID NO: 723 - DNA, 120 bp, Artificial Sequence
  KIT
acagtgacgtgcacaataaaagatgtgtctagttctgtgtactcaacgtggaaaagagaaaacagtcaggtgagtgaatcgcttcattcttctcatgttctgtctctgtgggagatgata

SEQ ID NO: 724 - DNA, 120 bp, Artificial Sequence
  KIT
tcttcatttttttttctccttttctgaaaccagcagactaaactacaggagaaatataatagctggcatcacggtgacttcaattatgaacgtcaggcaacgttgactatcagttcagcg

SEQ ID NO: 725 - DNA, 120 bp, Artificial Sequence
  KIT
agctggcatcacggtgacttcaattatgaacgtcaggcaacgttgactatcagttcagcgagagttaatgattctggagtgttcatgtgttatgccaataatacttttggatcagcaaat

SEQ ID NO: 726 - DNA, 120 bp, Artificial Sequence
  KIT
agagttaatgattctggagtgttcatgtgttatgccaataatacttttggatcagcaaatgtcacaacaaccttggaagtagtaggtaaatacctctatgggaatgtttaaattactggc

SEQ ID NO: 727 - DNA, 120 bp, Artificial Sequence
  KIT
ttctgtcttatttcattctaattagataaaggattcattaatatcttccccatgataaacactacagtatttgtaaacgatggagaaaatgtagatttgattgttgaatatgaagcattc

SEQ ID NO: 728 - DNA, 120 bp, Artificial Sequence
  KIT
actacagtatttgtaaacgatggagaaaatgtagatttgattgttgaatatgaagcattccccaaacctgaacaccagcagtggatctatatgaacagaaccttcactgataaatgggaa

SEQ ID NO: 729 - DNA, 120 bp, Artificial Sequence
  KIT
cccaaacctgaacaccagcagtggatctatatgaacagaaccttcactgataaatgggaagattatcccaagtctgagaatgaaagtaatatcaggtaagaaatggaccttgccctgggg

SEQ ID NO: 730 - DNA, 120 bp, Artificial Sequence
  KIT
aaagacatgccttccaaggcatgctatccacaggtgattgactagttgtcttttctttgtagatacgtaagtgaacttcatctaacgagattaaaaggcaccgaaggaggcacttacaca

SEQ ID NO: 731 - DNA, 120 bp, Artificial Sequence
  KIT
agatacgtaagtgaacttcatctaacgagattaaaaggcaccgaaggaggcacttacacattcctagtgtccaattctgacgtcaatgctgccatagcatttaatgtttatgtgaatagt

SEQ ID NO: 732 - DNA, 120 bp, Artificial Sequence
  KIT
ttcctagtgtccaattctgacgtcaatgctgccatagcatttaatgtttatgtgaatagtaagtaacatgaagggctccttttaattttttattcttttaaagttgtggctcgtgtttgt

SEQ ID NO: 733 - DNA, 120 bp, Artificial Sequence
  KIT
tgaagtgaatgttgctgaggttttccagcactctgacatatggccatttctgttttcctgtagcaaaaccagaaatcctgacttacgacaggctcgtgaatggcatgctccaatgtgtgg

SEQ ID NO: 734 - DNA, 120 bp, Artificial Sequence
  KIT
tagcaaaaccagaaatcctgacttacgacaggctcgtgaatggcatgctccaatgtgtggcagcaggattcccagagcccacaatagattggtatttttgtccaggaactgagcagaggt

SEQ ID NO: 735 - DNA, 120 bp, Artificial Sequence
  KIT
cagcaggattcccagagcccacaatagattggtatttttgtccaggaactgagcagaggtgagatgattatttttggcactgcttataatgcagaggggaaggactgcaattcacttgaa

SEQ ID NO: 736 - DNA, 120 bp, Artificial Sequence
  KIT
ggcttttgttttcttccctttagatgctctgcttctgtactgccagtggatgtgcagacactaaactcatctgggccaccgtttggaaagctagtggttcagagttctatagattctagt

SEQ ID NO: 737 - DNA, 120 bp, Artificial Sequence
  KIT
ctaaactcatctgggccaccgtttggaaagctagtggttcagagttctatagattctagtgcattcaagcacaatggcacggttgaatgtaaggcttacaacgatgtgggcaagacttct

SEQ ID NO: 738 - DNA, 120 bp, Artificial Sequence
  KIT
gcattcaagcacaatggcacggttgaatgtaaggcttacaacgatgtgggcaagacttctgcctattttaactttgcatttaaaggtaacaacaaaggtatatttctttttaatccaatt

SEQ ID NO: 739 - DNA, 120 bp, Artificial Sequence
  KIT
ctgagtggctgtggtagagatcccatcctgccaaagtttgtgattccacatttctcttccattgtagagcaaatccatccccacaccctgttcactcctttgctgattggtttcgtaatc

SEQ ID NO: 740 - DNA, 120 bp, Artificial Sequence
  KIT
attgtagagcaaatccatccccacaccctgttcactcctttgctgattggtttcgtaatcgtagctggcatgatgtgcattattgtgatgattctgacctacaaatatttacaggtaacc

SEQ ID NO: 741 - DNA, 120 bp, Artificial Sequence
  KIT
gtagctggcatgatgtgcattattgtgatgattctgacctacaaatatttacaggtaaccatttatttgttctctctccagagtgctctaatgactgagacaataattattaaaaggtga

SEQ ID NO: 742 - DNA, 120 bp, Artificial Sequence
  KIT
taatgactgagacaataattattaaaaggtgatctatttttccctttctccccacagaaacccatgtatgaagtacagtggaaggttgttgaggagataaatggaaacaattatgtttac

SEQ ID NO: 743 - DNA, 120 bp, Artificial Sequence
  KIT
cccatgtatgaagtacagtggaaggttgttgaggagataaatggaaacaattatgtttacatagacccaacacaacttccttatgatcacaaatgggagtttcccagaaacaggctgagt

SEQ ID NO: 744 - DNA, 120 bp, Artificial Sequence
  KIT
atagacccaacacaacttccttatgatcacaaatgggagtttcccagaaacaggctgagttttggtcagtatgaaacaggggctttccatgtcacctttttgggtacacataacagtgac

SEQ ID NO: 745 - DNA, 120 bp, Artificial Sequence
  KIT
gcacaaatggtccttcaattccaccaccagcaccatcaccacttaccttgttgtcttccttcctacagggaaaaccctgggtgctggagctttcgggaaggttgttgaggcaactgctta

SEQ ID NO: 746 - DNA, 120 bp, Artificial Sequence
  KIT
tcctacagggaaaaccctgggtgctggagctttcgggaaggttgttgaggcaactgcttatggcttaattaagtcagatgcggccatgactgtcgctgtaaagatgctcaagcgtaagtt

SEQ ID NO: 747 - DNA, 120 bp, Artificial Sequence
  KIT
tggcttaattaagtcagatgcggccatgactgtcgctgtaaagatgctcaagcgtaagttcctgtatggtactgcatgcgcttgacatcagtttgccagttgtgctttttgctaaaatgc

SEQ ID NO: 748 - DNA, 120 bp, Artificial Sequence
  KIT
ctgcatgcgcttgacatcagtttgccagttgtgctttttgctaaaatgcatgtttccaattttagcgagtgcccatttgacagaacgggaagccctcatgtctgaactcaaagtcctgag

SEQ ID NO: 749 - DNA, 120 bp, Artificial Sequence; identical to SEQ ID NO: 33
  KIT

SEQ ID NO: 750 - DNA, 120 bp, Artificial Sequence
  KIT
ttaccttggtaatcacatgaatattgtgaatctacttggagcctgcaccattggaggtaaagccgtgtccaagctgccttttattgtctgtcaggttatcaaaacatgacattttaatat

SEQ ID NO: 751 - DNA, 120 bp, Artificial Sequence
  KIT
catgtcccacttgattcagtcatgacttgtttcatctctcccagcagcgatagtactaatgagtacatggacatgaaacctggagtttcttatgttgtcccaaccaaggccgacaaaagg

SEQ ID NO: 752 - DNA, 120 bp, Artificial Sequence
  KIT
gagtacatggacatgaaacctggagtttcttatgttgtcccaaccaaggccgacaaaaggagatctgtgagaataggtgagtacctacctatcaagcaaccaagagtaactttacagaga

SEQ ID NO: 753 - DNA, 120 bp, Artificial Sequence
  KIT
cttttcctttcctgacctttatggttgtaattgctaagaaaaatcctctcttcctcacaggctcatacatagaaagagatgtgactcccgccatcatggaggatgacgagttggccctag

SEQ ID NO: 754 - DNA, 120 bp, Artificial Sequence
  KIT
gctcatacatagaaagagatgtgactcccgccatcatggaggatgacgagttggccctagacttagaagacttgctgagcttttcttaccaggtggcaaagggcatggctttcctcgcct

SEQ ID NO: 755 - DNA, 120 bp, Artificial Sequence
  KIT
acttagaagacttgctgagcttttcttaccaggtggcaaagggcatggctttcctcgcctccaagaatgtaagtgggagtgattctctaaagagttttgtgttttgtttttttgattttt

SEQ ID NO: 756 - DNA, 120 bp, Artificial Sequence
  KIT
tcactctttacaagttaaaatgaatttaaatggttttcttttctcctccaacctaatagtgtattcacagagacttggcagccagaaatatcctccttactcatggtcggatcacaaaga

SEQ ID NO: 757 - DNA, 120 bp, Artificial Sequence
  KIT
gtattcacagagacttggcagccagaaatatcctccttactcatggtcggatcacaaagatttgtgattttggtctagccagagacatcaagaatgattctaattatgtggttaaaggaa

SEQ ID NO: 758 - DNA, 120 bp, Artificial Sequence
  KIT
tttgtgattttggtctagccagagacatcaagaatgattctaattatgtggttaaaggaaacgtgagtacccattctctgcttgacagtcctgcaaaggatttttagtttcaactttcga

SEQ ID NO: 759 - DNA, 120 bp, Artificial Sequence
  KIT
cttctgttcaattttgttgagcttctgaattaacattattgactctgttgtgcttctattacaggctcgactacctgtgaagtggatggcacctgaaagcattttcaactgtgtatacac

SEQ ID NO: 760 - DNA, 120 bp, Artificial Sequence
  KIT
acaggctcgactacctgtgaagtggatggcacctgaaagcattttcaactgtgtatacacgtttgaaagtgacgtctggtcctatgggatttttctttgggagctgttctctttaggtaa

SEQ ID NO: 761 - DNA, 120 bp, Artificial Sequence
  KIT
gtttgaaagtgacgtctggtcctatgggatttttctttgggagctgttctctttaggtaaaatgatccttgccaaagacaacttcattagactcagagcatcttcttgaagtttcattgg

SEQ ID NO: 762 - DNA, 120 bp, Artificial Sequence
  KIT
cttccttgtgattaacactgctttgcaaactgtgtctcaggaagcagcccctatcctggaatgccggtcgattctaagttctacaagatgatcaaggaaggcttccggatgctcagccct

SEQ ID NO: 763 - DNA, 120 bp, Artificial Sequence
  KIT
atgccggtcgattctaagttctacaagatgatcaaggaaggcttccggatgctcagccctgaacacgcacctgctgaaatgtaagagccaaaaaatttttcctttaggtcacgttttccc

SEQ ID NO: 764 - DNA, 120 bp, Artificial Sequence
  KIT
atgcccatacatttgaaaacaagctgagggcattgaggagggatagtaaatggcccttgtcttgcaggtatgacataatgaagacttgctgggatgcagatcccctaaaaagaccaacat

SEQ ID NO: 765 - DNA, 120 bp, Artificial Sequence
  KIT
cttgcaggtatgacataatgaagacttgctgggatgcagatcccctaaaaagaccaacattcaagcaaattgttcagctaattgagaagcagatttcagagagcaccaatcatgtgagta

SEQ ID NO: 766 - DNA, 120 bp, Artificial Sequence
  KIT
tcaagcaaattgttcagctaattgagaagcagatttcagagagcaccaatcatgtgagtataccctggccaggcatagaatcccccttctcccagttccaggtgtgtcctcctcctcagg

SEQ ID NO: 767 - DNA, 120 bp, Artificial Sequence
  KIT
tgttgctatgttcgttgtagggactgctgtattgactatgggcttgttttctccagatttactccaacttagcaaactgcagccccaaccgacagaagcccgtggtagaccattctgtgc

SEQ ID NO: 768 - DNA, 120 bp, Artificial Sequence
  KIT
actccaacttagcaaactgcagccccaaccgacagaagcccgtggtagaccattctgtgcggatcaattctgtcggcagcaccgcttcctcctcccagcctctgcttgtgcacgacgatg

SEQ ID NO: 769 - DNA, 120 bp, Artificial Sequence
  KIT
ggatcaattctgtcggcagcaccgcttcctcctcccagcctctgcttgtgcacgacgatgtctgagcagaatcagtgtttgggtcacccctccaggaatgatctcttcttttggcttcca

SEQ ID NO: 770 - DNA, 120 bp, Artificial Sequence; identical to SEQ ID NO: 742
  KIT-E11

SEQ ID NO: 771 - DNA, 120 bp, Artificial Sequence
  KIT-E11
aaaggtgatctatttttccctttctccccacagaaacccatgtatgaagtacagtggaaggttgttgaggagataaatggaaacaattatgtttacatagacccaacacaacttccttat

SEQ ID NO: 772 - DNA, 120 bp, Artificial Sequence
  KIT-E11
ataaatggaaacaattatgtttacatagacccaacacaacttccttatgatcacaaatgggagtttcccagaaacaggctgagttttggtcagtatgaaacaggggctttccatgtcacc

SEQ ID NO: 773 - DNA, 120 bp, Artificial Sequence; identical to SEQ ID NO: 744
  KIT-E11

SEQ ID NO: 774 - DNA, 120 bp, Artificial Sequence
  KIT-E13
ctgtaaagatgctcaagcgtaagttcctgtatggtactgcatgcgcttgacatcagtttgccagttgtgctttttgctaaaatgcatgtttccaattttagcgagtgcccatttgacaga

SEQ ID NO: 775 - DNA, 120 bp, Artificial Sequence
  KIT-E13
tcctgtatggtactgcatgcgcttgacatcagtttgccagttgtgctttttgctaaaatgcatgtttccaattttagcgagtgcccatttgacagaacgggaagccctcatgtctgaact

SEQ ID NO: 776 - DNA, 120 bp, Artificial Sequence
  KIT-E13
gacatcagtttgccagttgtgctttttgctaaaatgcatgtttccaattttagcgagtgcccatttgacagaacgggaagccctcatgtctgaactcaaagtcctgagttaccttggtaa

SEQ ID NO: 777 - DNA, 120 bp, Artificial Sequence
  KIT-E13
tttgctaaaatgcatgtttccaattttagcgagtgcccatttgacagaacgggaagccctcatgtctgaactcaaagtcctgagttaccttggtaatcacatgaatattgtgaatctact

SEQ ID NO: 778 - DNA, 120 bp, Artificial Sequence
  KIT-E13
acgggaagccctcatgtctgaactcaaagtcctgagttaccttggtaatcacatgaatattgtgaatctacttggagcctgcaccattggaggtaaagccgtgtccaagctgccttttat

SEQ ID NO: 779 - DNA, 120 bp, Artificial Sequence
  KIT-E13
caaagtcctgagttaccttggtaatcacatgaatattgtgaatctacttggagcctgcaccattggaggtaaagccgtgtccaagctgccttttattgtctgtcaggttatcaaaacatg

SEQ ID NO: 780 - DNA, 120 bp, Artificial Sequence
  KIT-E13
tcacatgaatattgtgaatctacttggagcctgcaccattggaggtaaagccgtgtccaagctgccttttattgtctgtcaggttatcaaaacatgacattttaatatgattttggcaat

SEQ ID NO: 781 - DNA, 120 bp, Artificial Sequence
  KIT-E13
tggagcctgcaccattggaggtaaagccgtgtccaagctgccttttattgtctgtcaggttatcaaaacatgacattttaatatgattttggcaatgctagattataaactgcttggaag

SEQ ID NO: 782 - DNA, 120 bp, Artificial Sequence
  KIT-E14
ttacagaatattgttgctatggtgatcttttgaattttttgagaagaaaacgtgattcatttatttgttcaaagcaggaagatcatgcagaagctgcactttataagaatcttctgcatt

SEQ ID NO: 783 - DNA, 120 bp, Artificial Sequence; identical to SEQ ID NO: 756
  KIT-E17

SEQ ID NO: 784 - DNA, 120 bp, Artificial Sequence
  KIT-E17
tttaaatggttttcttttctcctccaacctaatagtgtattcacagagacttggcagccagaaatatcctccttactcatggtcggatcacaaagatttgtgattttggtctagccagag

SEQ ID NO: 785 - DNA, 120 bp, Artificial Sequence
  KIT-E17
ttactcatggtcggatcacaaagatttgtgattttggtctagccagagacatcaagaatgattctaattatgtggttaaaggaaacgtgagtacccattctctgcttgacagtcctgcaa

SEQ ID NO: 786 - DNA, 120 bp, Artificial Sequence; identical to SEQ ID NO: 758
  KIT-E17

SEQ ID NO: 787 - DNA, 120 bp, Artificial Sequence
  KIT-E18
tccacatttcagcaacagcagcatctataagaatatcttctgttcaattttgttgagcttctgaattaacattattgactctgttgtgcttctattacaggctcgactacctgtgaagtg

SEQ ID NO: 788 - DNA, 120 bp, Artificial Sequence
  KIT-E18
ctataagaatatcttctgttcaattttgttgagcttctgaattaacattattgactctgttgtgcttctattacaggctcgactacctgtgaagtggatggcacctgaaagcattttcaa

SEQ ID NO: 789 - DNA, 120 bp, Artificial Sequence
  KIT-E18
tttgttgagcttctgaattaacattattgactctgttgtgcttctattacaggctcgactacctgtgaagtggatggcacctgaaagcattttcaactgtgtatacacgtttgaaagtga

SEQ ID NO: 790 - DNA, 120 bp, Artificial Sequence
  KIT-E18
tattgactctgttgtgcttctattacaggctcgactacctgtgaagtggatggcacctgaaagcattttcaactgtgtatacacgtttgaaagtgacgtctggtcctatgggatttttct

SEQ ID NO: 791 - DNA, 120 bp, Artificial Sequence; identical to SEQ ID NO: 760
  KIT-E18

SEQ ID NO: 792 - DNA, 120 bp, Artificial Sequence
  KIT-E18
gatggcacctgaaagcattttcaactgtgtatacacgtttgaaagtgacgtctggtcctatgggatttttctttgggagctgttctctttaggtaaaatgatccttgccaaagacaactt

SEQ ID NO: 793 - DNA, 120 bp, Artificial Sequence
  KIT-E18
ctgtgtatacacgtttgaaagtgacgtctggtcctatgggatttttctttgggagctgttctctttaggtaaaatgatccttgccaaagacaacttcattagactcagagcatcttcttg

SEQ ID NO: 794 - DNA, 120 bp, Artificial Sequence
  KIT-E18
cgtctggtcctatgggatttttctttgggagctgttctctttaggtaaaatgatccttgccaaagacaacttcattagactcagagcatcttcttgaagtttcattggtgtcctgcttcc

SEQ ID NO: 795 - DNA, 120 bp, Artificial Sequence
  KIT-E18
ttgggagctgttctctttaggtaaaatgatccttgccaaagacaacttcattagactcagagcatcttcttgaagtttcattggtgtcctgcttccttgtgattaacactgctttgcaaa

SEQ ID NO: 796 - DNA, 120 bp, Artificial Sequence
  KIT-E8
gcagcctcaggaaggttgtagggattagagagggagtgaagtgaatgttgctgaggttttccagcactctgacatatggccatttctgttttcctgtagcaaaaccagaaatcctgactt

SEQ ID NO: 797 - DNA, 120 bp, Artificial Sequence
  KIT-E8
ttagagagggagtgaagtgaatgttgctgaggttttccagcactctgacatatggccatttctgttttcctgtagcaaaaccagaaatcctgacttacgacaggctcgtgaatggcatgc

SEQ ID NO: 798 - DNA, 120 bp, Artificial Sequence
  KIT-E8
tgctgaggttttccagcactctgacatatggccatttctgttttcctgtagcaaaaccagaaatcctgacttacgacaggctcgtgaatggcatgctccaatgtgtggcagcaggattcc

SEQ ID NO: 799 - DNA, 120 bp, Artificial Sequence
  KIT-E8
catatggccatttctgttttcctgtagcaaaaccagaaatcctgacttacgacaggctcgtgaatggcatgctccaatgtgtggcagcaggattcccagagcccacaatagattggtatt

SEQ ID NO: 800 - DNA, 120 bp, Artificial Sequence; identical to SEQ ID NO: 734
  KIT-E8

SEQ ID NO: 801 - DNA, 120 bp, Artificial Sequence
  KIT-E8
acgacaggctcgtgaatggcatgctccaatgtgtggcagcaggattcccagagcccacaatagattggtatttttgtccaggaactgagcagaggtgagatgattatttttggcactgct

SEQ ID NO: 802 - DNA, 120 bp, Artificial Sequence
  KIT-E8
tccaatgtgtggcagcaggattcccagagcccacaatagattggtatttttgtccaggaactgagcagaggtgagatgattatttttggcactgcttataatgcagaggggaaggactgc

SEQ ID NO: 803 - DNA, 120 bp, Artificial Sequence
  KIT-E8
cagagcccacaatagattggtatttttgtccaggaactgagcagaggtgagatgattatttttggcactgcttataatgcagaggggaaggactgcaattcacttgaatttcaaatatgt

SEQ ID NO: 804 - DNA, 120 bp, Artificial Sequence
  KIT-E8
tttgtccaggaactgagcagaggtgagatgattatttttggcactgcttataatgcagaggggaaggactgcaattcacttgaatttcaaatatgttttctgattttttttaaaaaagct

SEQ ID NO: 805 - DNA, 120 bp, Artificial Sequence
  KIT-E9
ttttatgtatttatttattttcctagagtaagccagggcttttgttttcttccctttagatgctctgcttctgtactgccagtggatgtgcagacactaaactcatctgggccaccgttt

SEQ ID NO: 806 - DNA, 120 bp, Artificial Sequence
  KIT-E9
agagtaagccagggcttttgttttcttccctttagatgctctgcttctgtactgccagtggatgtgcagacactaaactcatctgggccaccgtttggaaagctagtggttcagagttct

SEQ ID NO: 807 - DNA, 120 bp, Artificial Sequence
  KIT-E9
gtactgccagtggatgtgcagacactaaactcatctgggccaccgtttggaaagctagtggttcagagttctatagattctagtgcattcaagcacaatggcacggttgaatgtaaggct

SEQ ID NO: 808 - DNA, 120 bp, Artificial Sequence; identical to SEQ ID NO: 737
  KIT-E9

SEQ ID NO: 809 - DNA, 120 bp, Artificial Sequence
  KIT-E9
ggaaagctagtggttcagagttctatagattctagtgcattcaagcacaatggcacggttgaatgtaaggcttacaacgatgtgggcaagacttctgcctattttaactttgcatttaaa

SEQ ID NO: 810 - DNA, 120 bp, Artificial Sequence
  KIT-E9
aatggcacggttgaatgtaaggcttacaacgatgtgggcaagacttctgcctattttaactttgcatttaaaggtaacaacaaaggtatatttctttttaatccaatttaaggggatgtt

SEQ ID NO: 811 - DNA, 120 bp, Artificial Sequence
  KIT-E9
tacaacgatgtgggcaagacttctgcctattttaactttgcatttaaaggtaacaacaaaggtatatttctttttaatccaatttaaggggatgtttaggctctgtctaccatatcagtc

SEQ ID NO: 812 - DNA, 120 bp, Artificial Sequence; identical to SEQ ID NO: 805
  KIT-E9

SEQ ID NO: 813 - DNA, 120 bp, Artificial Sequence; identical to SEQ ID NO: 806
  KIT-E9

SEQ ID NO: 814 - DNA, 120 bp, Artificial Sequence; identical to SEQ ID NO: 29
  KIT-E9

SEQ ID NO: 815 - DNA, 120 bp, Artificial Sequence; identical to SEQ ID NO: 807
  KIT-E9

SEQ ID NO: 816 - DNA, 120 bp, Artificial Sequence; identical to SEQ ID NO: 737
  KIT-E9

SEQ ID NO: 817 - DNA, 120 bp, Artificial Sequence; identical to SEQ ID NO: 809
  KIT-E9

SEQ ID NO: 818 - DNA, 120 bp, Artificial Sequence; identical to SEQ ID NO: 30
  KIT-E9

SEQ ID NO: 819 - DNA, 120 bp, Artificial Sequence; identical to SEQ ID NO: 810
  KIT-E9

SEQ ID NO: 820 - DNA, 120 bp, Artificial Sequence; identical to SEQ ID NO: 811
  KIT-E9

SEQ ID NO: 821 - DNA, 120 bp, Artificial Sequence
  KRAS
gtgtaatgtacaaaaattaccacttgtactagtatgccttaagaaaaaagtacaaattgtatttacataattacacactttgtctttgacttctttttcttctttttaccatctttgctc

SEQ ID NO: 822 - DNA, 120 bp, Artificial Sequence
  KRAS
atttacataattacacactttgtctttgacttctttttcttctttttaccatctttgctcatcttttctttatgttttcgaatttctcgaactaatgtatagaaggcatcatcaacaccc

SEQ ID NO: 823 - DNA, 120 bp, Artificial Sequence
  KRAS
atcttttctttatgttttcgaatttctcgaactaatgtatagaaggcatcatcaacaccctgaaatacataaaaagtattaaaatgtgaatatatacgatggcttcatgtgtacaggtaa

SEQ ID NO: 824 - DNA, 120 bp, Artificial Sequence
  KRAS
tacctttaaaagacatctgctttctgccaaaattaatgtgctgaacttaaacttaccagattacattataatgcattttttaattttcacacagccaggagtcttttcttctttgctgat

SEQ ID NO: 825 - DNA, 120 bp, Artificial Sequence
  KRAS
ttacattataatgcattttttaattttcacacagccaggagtcttttcttctttgctgatttttttcaatctgtattgtcggatctccctcaccaatgtataaaaagcatcctccactct

SEQ ID NO: 826 - DNA, 120 bp, Artificial Sequence
  KRAS
ttttttcaatctgtattgtcggatctccctcaccaatgtataaaaagcatcctccactctctgcattgtaaaacacaacttctttaaagtctgttgcattggtaagagtaatttactggg

SEQ ID NO: 827 - DNA, 120 bp, Artificial Sequence
  KRAS
ttgcagaaaacagatctgtatttatttcagtgttacttacctgtcttgtctttgctgatgtttcaataaaaggaattccataacttcttgctaagtcctgagcctgttttgtgtctactg

SEQ ID NO: 828 - DNA, 120 bp, Artificial Sequence
  KRAS
tttcaataaaaggaattccataacttcttgctaagtcctgagcctgttttgtgtctactgttctagaaggcaaatcacatttatttcctactaggaccataggtacatcttcagagtcct

SEQ ID NO: 829 - DNA, 120 bp, Artificial Sequence
  KRAS
ttctagaaggcaaatcacatttatttcctactaggaccataggtacatcttcagagtccttaactcttttaatttgttctctgggaaagaaaaaaaagttatagcacagtcattagtaac

SEQ ID NO: 830 - DNA, 120 bp, Artificial Sequence
  KRAS
tgtcagcttattatattcaatttaaacccacctataatggtgaatatcttcaaatgatttagtattatttatggcaaatacacaaagaaagccctccccagtcctcatgtactggtccct

SEQ ID NO: 831 - DNA, 120 bp, Artificial Sequence
  KRAS
agtattatttatggcaaatacacaaagaaagccctccccagtcctcatgtactggtccctcattgcactgtactcctcttgacctgctgtgtcgagaatatccaagagacaggtttctcc

SEQ ID NO: 832 - DNA, 120 bp, Artificial Sequence
  KRAS
cattgcactgtactcctcttgacctgctgtgtcgagaatatccaagagacaggtttctccatcaattactacttgcttcctgtaggaatcctgagaagggagaaacacagtctggattat

SEQ ID NO: 833 - DNA, 120 bp, Artificial Sequence
  KRAS
aaatgtcaataatgtattactcggggatttcctcttgaaattgtatgttttcttaatgtattaagtattgtaaggactttttacatactgcttaataacacctgtaggaaaagatgagaa

SEQ ID NO: 834 - DNA, 120 bp, Artificial Sequence
  KRAS
ttaagtattgtaaggactttttacatactgcttaataacacctgtaggaaaagatgagaaacttttactcaattaatgctcaagtactttacgttactcttccgaaaggttatttaaatt

SEQ ID NO: 835 - DNA, 120 bp, Artificial Sequence
  KRAS
gaaacctttatctgtatcaaagaatggtcctgcaccagtaatatgcatattaaaacaagatttacctctattgttggatcatattcgtccacaaaatgattctgaattagctgtatcgtc

SEQ ID NO: 836 - DNA, 120 bp, Artificial Sequence
  KRAS
tttacctctattgttggatcatattcgtccacaaaatgattctgaattagctgtatcgtcaaggcactcttgcctacgccaccagctccaactaccacaagtttatattcagtcattttc

SEQ ID NO: 837 - DNA, 120 bp, Artificial Sequence
  KRAS
aaggcactcttgcctacgccaccagctccaactaccacaagtttatattcagtcattttcagcaggccttataataaaaataatgaaaatgtgactatattagaacatgtcacacataag

SEQ ID NO: 838 - DNA, 120 bp, Artificial Sequence
  KRAS-E2
tttatctgtatcaaagaatggtcctgcaccagtaatatgcatattaaaacaagatttacctctattgttggatcatattcgtccacaaaatgattctgaattagctgtatcgtcaaggca

SEQ ID NO: 839 - DNA, 120 bp, Artificial Sequence
  KRAS-E2
tgcaccagtaatatgcatattaaaacaagatttacctctattgttggatcatattcgtccacaaaatgattctgaattagctgtatcgtcaaggcactcttgcctacgccaccagctcca

SEQ ID NO: 840 - DNA, 120 bp, Artificial Sequence
  KRAS-E2
tcatattcgtccacaaaatgattctgaattagctgtatcgtcaaggcactcttgcctacgccaccagctccaactaccacaagtttatattcagtcattttcagcaggccttataataaa

SEQ ID NO: 841 - DNA, 120 bp, Artificial Sequence
  KRAS-E2
tgaattagctgtatcgtcaaggcactcttgcctacgccaccagctccaactaccacaagtttatattcagtcattttcagcaggccttataataaaaataatgaaaatgtgactatatta

SEQ ID NO: 842 - DNA, 120 bp, Artificial Sequence
  KRAS-E2
ctcttgcctacgccaccagctccaactaccacaagtttatattcagtcattttcagcaggccttataataaaaataatgaaaatgtgactatattagaacatgtcacacataaggttaat

SEQ ID NO: 843 - DNA, 120 bp, Artificial Sequence
  KRAS-E3
ataaaaactataattactccttaatgtcagcttattatattcaatttaaacccacctataatggtgaatatcttcaaatgatttagtattatttatggcaaatacacaaagaaagccctc

SEQ ID NO: 844 - DNA, 120 bp, Artificial Sequence; identical to SEQ ID NO: 830
  KRAS-E3

SEQ ID NO: 845 - DNA, 120 bp, Artificial Sequence
  KRAS-E3
aacccacctataatggtgaatatcttcaaatgatttagtattatttatggcaaatacacaaagaaagccctccccagtcctcatgtactggtccctcattgcactgtactcctcttgacc

SEQ ID NO: 846 - DNA, 120 bp, Artificial Sequence
  KRAS-E3
ttcaaatgatttagtattatttatggcaaatacacaaagaaagccctccccagtcctcatgtactggtccctcattgcactgtactcctcttgacctgctgtgtcgagaatatccaagag

SEQ ID NO: 847 - DNA, 120 bp, Artificial Sequence
  KRAS-E3
cccagtcctcatgtactggtccctcattgcactgtactcctcttgacctgctgtgtcgagaatatccaagagacaggtttctccatcaattactacttgcttcctgtaggaatcctgaga

SEQ ID NO: 848 - DNA, 120 bp, Artificial Sequence; identical to SEQ ID NO: 832
  KRAS-E3

SEQ ID NO: 849 - DNA, 120 bp, Artificial Sequence
  KRAS-E3
tgctgtgtcgagaatatccaagagacaggtttctccatcaattactacttgcttcctgtaggaatcctgagaagggagaaacacagtctggattattacagtgcaccttttacttcaaaa

SEQ ID NO: 850 - DNA, 120 bp, Artificial Sequence
  KRAS-E4
acagttatgattttgcagaaaacagatctgtatttatttcagtgttacttacctgtcttgtctttgctgatgtttcaataaaaggaattccataacttcttgctaagtcctgagcctgtt

SEQ ID NO: 851 - DNA, 120 bp, Artificial Sequence
  KRAS-E4
gatctgtatttatttcagtgttacttacctgtcttgtctttgctgatgtttcaataaaaggaattccataacttcttgctaagtcctgagcctgttttgtgtctactgttctagaaggca

SEQ ID NO: 852 - DNA, 120 bp, Artificial Sequence; identical to SEQ ID NO: 828
  KRAS-E4

SEQ ID NO: 853 - DNA, 120 bp, Artificial Sequence
  KRAS-E4
ttcttgctaagtcctgagcctgttttgtgtctactgttctagaaggcaaatcacatttatttcctactaggaccataggtacatcttcagagtccttaactcttttaatttgttctctgg

SEQ ID NO: 854 - DNA, 120 bp, Artificial Sequence
  KRAS-E4
ttgtgtctactgttctagaaggcaaatcacatttatttcctactaggaccataggtacatcttcagagtccttaactcttttaatttgttctctgggaaagaaaaaaaagttatagcaca

SEQ ID NO: 855 - DNA, 120 bp, Artificial Sequence
  KRAS-E4
aatcacatttatttcctactaggaccataggtacatcttcagagtccttaactcttttaatttgttctctgggaaagaaaaaaaagttatagcacagtcattagtaacacaaatatcttt

SEQ ID NO: 856 - DNA, 120 bp, Artificial Sequence
  MAP2K1
agaggtgctgccctccccccggagttggaagcgcgttacccgggtccaaaatgcccaagaagaagccgacgcccatccagctgaacccggcccccgacggctctgcagttaacgggacca

SEQ ID NO: 857 - DNA, 120 bp, Artificial Sequence
  MAP2K1
agaagccgacgcccatccagctgaacccggcccccgacggctctgcagttaacgggaccagctctgcggagtaagtatggggcgggcggtgaacctcggggcccggctggggaggcccga

SEQ ID NO: 858 - DNA, 120 bp, Artificial Sequence
  MAP2K1
cccactttggaacaggaccaacttggaggccttgcagaagaagctggaggagctagagcttgatgagcagcagcgaaagcgccttgaggcctttcttacccagaagcagaaggtgggaga

SEQ ID NO: 859 - DNA, 120 bp, Artificial Sequence
  MAP2K1
tgatgagcagcagcgaaagcgccttgaggcctttcttacccagaagcagaaggtgggagaactgaaggatgacgactttgagaagatcagtgagctgggggctggcaatggcggtgtggt

SEQ ID NO: 860 - DNA, 120 bp, Artificial Sequence
  MAP2K1
actgaaggatgacgactttgagaagatcagtgagctgggggctggcaatggcggtgtggtgttcaaggtctcccacaagccttctggcctggtcatggccagaaaggtgagtttgccttg

SEQ ID NO: 861 - DNA, 120 bp, Artificial Sequence
  MAP2K1
ctccctctttctttcataaaacctctctttcttccacctttctccagctaattcatctggagatcaaacccgcaatccggaaccagatcataagggagctgcaggttctgcatgagtgca

SEQ ID NO: 862 - DNA, 120 bp, Artificial Sequence
  MAP2K1
agatcaaacccgcaatccggaaccagatcataagggagctgcaggttctgcatgagtgcaactctccgtacatcgtgggcttctatggtgcgttctacagcgatggcgagatcagtatct

SEQ ID NO: 863 - DNA, 120 bp, Artificial Sequence
  MAP2K1
actctccgtacatcgtgggcttctatggtgcgttctacagcgatggcgagatcagtatctgcatggagcacatggtatgtgacaccctctcagcctctggagcaatggccttaagagttg

SEQ ID NO: 864 - DNA, 120 bp, Artificial Sequence
  MAP2K1
aaagaatagttagaacattgtcactaactggtctggtattctcgatcttaggatggaggttctctggatcaagtcctgaagaaagctggaagaattcctgaacaaattttaggaaaagtt

SEQ ID NO: 865 - DNA, 120 bp, Artificial Sequence
  MAP2K1
tctctggatcaagtcctgaagaaagctggaagaattcctgaacaaattttaggaaaagttagcattgctgtgagtatgttatgaagtttttcttctaagttcctcattgataagttaatg

SEQ ID NO: 866 - DNA, 120 bp, Artificial Sequence
  MAP2K1
aaatagattgagtatttttcttatcaccagtattttcttttcttttacattccctttcctctaggtaataaaaggcctgacatatctgagggagaagcacaagatcatgcacagaggtaa

SEQ ID NO: 867 - DNA, 120 bp, Artificial Sequence
  MAP2K1
ctaggtaataaaaggcctgacatatctgagggagaagcacaagatcatgcacagaggtaagaagttatttgctagttattttgctttgaattttagatataatccaaaggctgttgcttc

SEQ ID NO: 868 - DNA, 120 bp, Artificial Sequence
  MAP2K1
cagactcctgttgtttacaagtcttctccagaagccctggaagaatgaactgtaaggcctggactatggaatggtacctgtgcaccagcaattcctgagcaagcagcacagtgagtaggt

SEQ ID NO: 869 - DNA, 120 bp, Artificial Sequence
  MAP2K1
ggactatggaatggtacctgtgcaccagcaattcctgagcaagcagcacagtgagtaggtgattcctggaaacctgagttcaggtgaaaatgagagagagcagtctccttgtccctgcct

SEQ ID NO: 870 - DNA, 120 bp, Artificial Sequence
  MAP2K1
tctcttccccaatctacctgtgtcagttccctccttttctattttctcttccctgcagatgtcaagccctccaacatcctagtcaactcccgtggggagatcaagctctgtgactttggg

SEQ ID NO: 871 - DNA, 120 bp, Artificial Sequence
  MAP2K1
gtcaagccctccaacatcctagtcaactcccgtggggagatcaagctctgtgactttggggtcagcgggcagctcatcgactccatggccaactccttcgtgggcacaaggtcctacatg

SEQ ID NO: 872 - DNA, 120 bp, Artificial Sequence
  MAP2K1
gtcagcgggcagctcatcgactccatggccaactccttcgtgggcacaaggtcctacatgtcggtatgaacagaagtttccattgcttgagcttcttgtacggtcagggagaggagccca

SEQ ID NO: 873 - DNA, 120 bp, Artificial Sequence
  MAP2K1
ctgtctgtctctcctgcagccagaaagactccaggggactcattactctgtgcagtcagacatctggagcatgggactgtctctggtagagatggcggttgggaggtatcccatccctcc

SEQ ID NO: 874 - DNA, 120 bp, Artificial Sequence
  MAP2K1
catctggagcatgggactgtctctggtagagatggcggttgggaggtatcccatccctcctccagatgccaaggagctggagctgatgtttgggtgccaggtggaaggagatgcggctga

SEQ ID NO: 875 - DNA, 120 bp, Artificial Sequence
  MAP2K1
tccagatgccaaggagctggagctgatgtttgggtgccaggtggaaggagatgcggctgagaccccacccaggccaaggacccccgggaggccccttagctgtgagtagcctggtgtgtc

SEQ ID NO: 876 - DNA, 120 bp, Artificial Sequence
  MAP2K1
tcatattaacaagtaatctgtttctgagaagtattttttctttttataaaatttgtagcatacggaatggacagccgacctcccatggcaatttttgagttgttggattacatagtcaac

SEQ ID NO: 877 - DNA, 120 bp, Artificial Sequence
  MAP2K1
tacggaatggacagccgacctcccatggcaatttttgagttgttggattacatagtcaacgaggtaagtactgcctggtttccttcaccttggaatttacttgctcatcttaagaaaaca

SEQ ID NO: 878 - DNA, 120 bp, Artificial Sequence
  MAP2K1
agaggagatggctggagcaaggagccaggcatttttcttatctcaacatgtgtttgcagcctcctccaaaactgcccagtggagtgttcagtctggaatttcaagattttgtgaataaat

SEQ ID NO: 879 - DNA, 120 bp, Artificial Sequence
  MAP2K1
ctcctccaaaactgcccagtggagtgttcagtctggaatttcaagattttgtgaataaatggtaagttggctccttgttctctggaagcgtatactctggatttgtcaggctccccaccc

SEQ ID NO: 880 - DNA, 120 bp, Artificial Sequence
  MAP2K1
caaacatgttatttgagctagaaccagtgccaggcaacagctcttaccttgtctttcttcctttaagcttaataaaaaaccccgcagagagagcagatttgaagcaactcatggtgagtc

SEQ ID NO: 881 - DNA, 120 bp, Artificial Sequence
  MAP2K1
ctttaagcttaataaaaaaccccgcagagagagcagatttgaagcaactcatggtgagtctatttattccggattcttacagtacctgtttattcatttgttcttctctgtcagtcatct

SEQ ID NO: 882 - DNA, 120 bp, Artificial Sequence
  MAP2K1
cctggtgggttttgtttttttgtttctttttaacaccacgtcctctcgtttccttacatgcaggttcatgcttttatcaagagatctgatgctgaggaagtggattttgcaggttggctc

SEQ ID NO: 883 - DNA, 120 bp, Artificial Sequence
  MAP2K1
caggttcatgcttttatcaagagatctgatgctgaggaagtggattttgcaggttggctctgctccaccatcggccttaaccagcccagcacaccaacccatgctgctggcgtctaagtg

SEQ ID NO: 884 - DNA, 120 bp, Artificial Sequence
  MAP2K1
tgctccaccatcggccttaaccagcccagcacaccaacccatgctgctggcgtctaagtgtttgggaagcaacaaagagcgagtcccctgcccggtggtttgccatgtcgcttttgggcc

SEQ ID NO: 885 - DNA, 120 bp, Artificial Sequence
  MAP2K1-E2
ggttgacttctctggtgacagtattgacttgtgctccccactttggaacaggaccaacttggaggccttgcagaagaagctggaggagctagagcttgatgagcagcagcgaaagcgcct

SEQ ID NO: 886 - DNA, 120 bp, Artificial Sequence
  MAP2K1-E2
tgacttgtgctccccactttggaacaggaccaacttggaggccttgcagaagaagctggaggagctagagcttgatgagcagcagcgaaagcgccttgaggcctttcttacccagaagca

SEQ ID NO: 887 - DNA, 120 bp, Artificial Sequence
  MAP2K1-E2
caggaccaacttggaggccttgcagaagaagctggaggagctagagcttgatgagcagcagcgaaagcgccttgaggcctttcttacccagaagcagaaggtgggagaactgaaggatga

SEQ ID NO: 888 - DNA, 120 bp, Artificial Sequence; identical to SEQ ID NO: 859
  MAP2K1-E2

SEQ ID NO: 889 - DNA, 120 bp, Artificial Sequence
  MAP2K1-E2
tgaggcctttcttacccagaagcagaaggtgggagaactgaaggatgacgactttgagaagatcagtgagctgggggctggcaatggcggtgtggtgttcaaggtctcccacaagccttc

SEQ ID NO: 890 - DNA, 120 bp, Artificial Sequence
  MAP2K1-E2
gaaggtgggagaactgaaggatgacgactttgagaagatcagtgagctgggggctggcaatggcggtgtggtgttcaaggtctcccacaagccttctggcctggtcatggccagaaaggt

SEQ ID NO: 891 - DNA, 120 bp, Artificial Sequence
  MAP2K1-E2
cgactttgagaagatcagtgagctgggggctggcaatggcggtgtggtgttcaaggtctcccacaagccttctggcctggtcatggccagaaaggtgagtttgccttgattaacaggtaa

SEQ ID NO: 892 - DNA, 120 bp, Artificial Sequence
  MAP2K1-E2
gggggctggcaatggcggtgtggtgttcaaggtctcccacaagccttctggcctggtcatggccagaaaggtgagtttgccttgattaacaggtaattggattatttctcagggtactta

SEQ ID NO: 893 - DNA, 120 bp, Artificial Sequence; identical to SEQ ID NO: 885
  MAP2K1-E2

SEQ ID NO: 894 - DNA, 120 bp, Artificial Sequence; identical to SEQ ID NO: 886
  MAP2K1-E2

SEQ ID NO: 895 - DNA, 120 bp, Artificial Sequence; identical to SEQ ID NO: 887
  MAP2K1-E2

SEQ ID NO: 896 - DNA, 120 bp, Artificial Sequence; identical to SEQ ID NO: 44
  MAP2K1-E2

SEQ ID NO: 897 - DNA, 120 bp, Artificial Sequence; identical to SEQ ID NO: 859
  MAP2K1-E2

SEQ ID NO: 898 - DNA, 120 bp, Artificial Sequence; identical to SEQ ID NO: 889
  MAP2K1-E2

SEQ ID NO: 899 - DNA, 120 bp, Artificial Sequence; identical to SEQ ID NO: 890
  MAP2K1-E2

SEQ ID NO: 900 - DNA, 120 bp, Artificial Sequence; identical to SEQ ID NO: 891
  MAP2K1-E2

SEQ ID NO: 901 - DNA, 120 bp, Artificial Sequence; identical to SEQ ID NO: 892
  MAP2K1-E2

SEQ ID NO: 902 - DNA, 120 bp, Artificial Sequence
  MET
tcgccttgaacctgttttggcagataaacctctcataatgaaggcccccgctgtgcttgcacctggcatcctcgtgctcctgtttaccttggtgcagaggagcaatggggagtgtaaaga

SEQ ID NO: 903 - DNA, 120 bp, Artificial Sequence
  MET
acctggcatcctcgtgctcctgtttaccttggtgcagaggagcaatggggagtgtaaagaggcactagcaaagtccgagatgaatgtgaatatgaagtatcagcttcccaacttcaccgc

SEQ ID NO: 904 - DNA, 120 bp, Artificial Sequence
  MET
ggcactagcaaagtccgagatgaatgtgaatatgaagtatcagcttcccaacttcaccgcggaaacacccatccagaatgtcattctacatgagcatcacattttccttggtgccactaa

SEQ ID NO: 905 - DNA, 120 bp, Artificial Sequence
  MET
ggaaacacccatccagaatgtcattctacatgagcatcacattttccttggtgccactaactacatttatgttttaaatgaggaagaccttcagaaggttgctgagtacaagactgggcc

SEQ ID NO: 906 - DNA, 120 bp, Artificial Sequence
  MET
ctacatttatgttttaaatgaggaagaccttcagaaggttgctgagtacaagactgggcctgtgctggaacacccagattgtttcccatgtcaggactgcagcagcaaagccaatttatc

SEQ ID NO: 907 - DNA, 120 bp, Artificial Sequence
  MET
tgtgctggaacacccagattgtttcccatgtcaggactgcagcagcaaagccaatttatcaggaggtgtttggaaagataacatcaacatggctctagttgtcgacacctactatgatga

SEQ ID NO: 908 - DNA, 120 bp, Artificial Sequence
  MET
aggaggtgtttggaaagataacatcaacatggctctagttgtcgacacctactatgatgatcaactcattagctgtggcagcgtcaacagagggacctgccagcgacatgtctttcccca

SEQ ID NO: 909 - DNA, 120 bp, Artificial Sequence
  MET
tcaactcattagctgtggcagcgtcaacagagggacctgccagcgacatgtctttccccacaatcatactgctgacatacagtcggaggttcactgcatattctccccacagatagaaga

SEQ ID NO: 910 - DNA, 120 bp, Artificial Sequence
  MET
caatcatactgctgacatacagtcggaggttcactgcatattctccccacagatagaagagcccagccagtgtcctgactgtgtggtgagcgccctgggagccaaagtcctttcatctgt

SEQ ID NO: 911 - DNA, 120 bp, Artificial Sequence
  MET
gcccagccagtgtcctgactgtgtggtgagcgccctgggagccaaagtcctttcatctgtaaaggaccggttcatcaacttctttgtaggcaataccataaattcttcttatttcccaga

SEQ ID NO: 912 - DNA, 120 bp, Artificial Sequence
  MET
aaaggaccggttcatcaacttctttgtaggcaataccataaattcttcttatttcccagatcatccattgcattcgatatcagtgagaaggctaaaggaaacgaaagatggttttatgtt

SEQ ID NO: 913 - DNA, 120 bp, Artificial Sequence
  MET
tcatccattgcattcgatatcagtgagaaggctaaaggaaacgaaagatggttttatgtttttgacggaccagtcctacattgatgttttacctgagttcagagattcttaccccattaa

SEQ ID NO: 914 - DNA, 120 bp, Artificial Sequence
  MET
tttgacggaccagtcctacattgatgttttacctgagttcagagattcttaccccattaagtatgtccatgcctttgaaagcaacaattttatttacttcttgacggtccaaagggaaac

SEQ ID NO: 915 - DNA, 120 bp, Artificial Sequence
  MET
gtatgtccatgcctttgaaagcaacaattttatttacttcttgacggtccaaagggaaactctagatgctcagacttttcacacaagaataatcaggttctgttccataaactctggatt

SEQ ID NO: 916 - DNA, 120 bp, Artificial Sequence
  MET
tctagatgctcagacttttcacacaagaataatcaggttctgttccataaactctggattgcattcctacatggaaatgcctctggagtgtattctcacagaaaagagaaaaaagagatc

SEQ ID NO: 917 - DNA, 120 bp, Artificial Sequence
  MET
gcattcctacatggaaatgcctctggagtgtattctcacagaaaagagaaaaaagagatccacaaagaaggaagtgtttaatatacttcaggctgcgtatgtcagcaagcctggggccca

SEQ ID NO: 918 - DNA, 120 bp, Artificial Sequence
  MET
cacaaagaaggaagtgtttaatatacttcaggctgcgtatgtcagcaagcctggggcccagcttgctagacaaataggagccagcctgaatgatgacattcttttcggggtgttcgcaca

SEQ ID NO: 919 - DNA, 120 bp, Artificial Sequence
  MET
gcttgctagacaaataggagccagcctgaatgatgacattcttttcggggtgttcgcacaaagcaagccagattctgccgaaccaatggatcgatctgccatgtgtgcattccctatcaa

SEQ ID NO: 920 - DNA, 120 bp, Artificial Sequence
  MET
aagcaagccagattctgccgaaccaatggatcgatctgccatgtgtgcattccctatcaaatatgtcaacgacttcttcaacaagatcgtcaacaaaaacaatgtgagatgtctccagca

SEQ ID NO: 921 - DNA, 120 bp, Artificial Sequence
  MET
atatgtcaacgacttcttcaacaagatcgtcaacaaaaacaatgtgagatgtctccagcatttttacggacccaatcatgagcactgctttaatagggtaagtcacatcagttccccact

SEQ ID NO: 922 - DNA, 120 bp, Artificial Sequence
  MET
ctctatgaccatattttattccagacacttctgagaaattcatcaggctgtgaagcgcgccgtgatgaatatcgaacagagtttaccacagctttgcagcgcgttgacttattcatgggt

SEQ ID NO: 923 - DNA, 120 bp, Artificial Sequence
  MET
cgtgatgaatatcgaacagagtttaccacagctttgcagcgcgttgacttattcatgggtcaattcagcgaagtcctcttaacatctatatccaccttcattaaaggagacctcaccata

SEQ ID NO: 924 - DNA, 120 bp, Artificial Sequence
  MET
caattcagcgaagtcctcttaacatctatatccaccttcattaaaggagacctcaccatagctaatcttgggacatcagagggtcgcttcatgcaggtaagtgctttctgagagtagctg

SEQ ID NO: 925 - DNA, 120 bp, Artificial Sequence
  MET
tatttaaactgagcttgttggaataaggatgttataacttttttgctgtttaggttgtggtttctcgatcaggaccatcaacccctcatgtgaattttctcctggactcccatccagtgt

SEQ ID NO: 926 - DNA, 120 bp, Artificial Sequence
  MET
tttctcgatcaggaccatcaacccctcatgtgaattttctcctggactcccatccagtgtctccagaagtgattgtggagcatacattaaaccaaaatggctacacactggttatcactg

SEQ ID NO: 927 - DNA, 120 bp, Artificial Sequence
  MET
ctccagaagtgattgtggagcatacattaaaccaaaatggctacacactggttatcactgggaagaaggtaagctgttcccacagggaatttccatagacgtggtttttcccaaatgcat

SEQ ID NO: 928 - DNA, 120 bp, Artificial Sequence
  MET
tctggaagctctttccaccccttctcttcacagatcacgaagatcccattgaatggcttgggctgcagacatttccagtcctgcagtcaatgcctctctgccccaccctttgttcagtgt

SEQ ID NO: 929 - DNA, 120 bp, Artificial Sequence
  MET
ggctgcagacatttccagtcctgcagtcaatgcctctctgccccaccctttgttcagtgtggctggtgccacgacaaatgtgtgcgatcggaggaatgcctgagcgggacatggactcaa

SEQ ID NO: 930 - DNA, 120 bp, Artificial Sequence
  MET
ggctggtgccacgacaaatgtgtgcgatcggaggaatgcctgagcgggacatggactcaacagatctgtctgcctgcaatctacaaggtaggaatctctaacagctggcatacatgtttt

SEQ ID NO: 931 - DNA, 120 bp, Artificial Sequence
  MET
tatattgggtttttttaaaagttctatgttgtccttgtaggttttcccaaatagtgcaccccttgaaggagggacaaggctgaccatatgtggctgggactttggatttcggaggaataa

SEQ ID NO: 932 - DNA, 120 bp, Artificial Sequence
  MET
ccttgaaggagggacaaggctgaccatatgtggctgggactttggatttcggaggaataataaatttgatttaaagaaaactagagttctccttggaaatgagagctgcaccttgacttt

SEQ ID NO: 933 - DNA, 120 bp, Artificial Sequence
  MET
taaatttgatttaaagaaaactagagttctccttggaaatgagagctgcaccttgactttaagtgagagcacgatgaatacgtaaggatcttaaaatgctttgctggggtgtgcttggaa

SEQ ID NO: 934 - DNA, 120 bp, Artificial Sequence
  MET
cctataaaacaacctaaccagaaaattccttggatttgtcatgtattaaactttgggttttttttccagattgaaatgcacagttggtcctgccatgaataagcatttcaatatgtccat

SEQ ID NO: 935 - DNA, 120 bp, Artificial Sequence
  MET
tttttccagattgaaatgcacagttggtcctgccatgaataagcatttcaatatgtccataattatttcaaatggccacgggacaacacaatacagtacattctcctatgtggtaaggaa

SEQ ID NO: 936 - DNA, 120 bp, Artificial Sequence
  MET
aattatttcaaatggccacgggacaacacaatacagtacattctcctatgtggtaaggaagattctatcctatcatgtttgatttttacttaatctatttaaattataagatgaacaagt

SEQ ID NO: 937 - DNA, 120 bp, Artificial Sequence
  MET
ttaaattataagatgaacaagttactttgttttgtttttatctcccctccaggatcctgtaataacaagtatttcgccgaaatacggtcctatggctggtggcactttacttactttaac

SEQ ID NO: 938 - DNA, 120 bp, Artificial Sequence
  MET
aataacaagtatttcgccgaaatacggtcctatggctggtggcactttacttactttaactggaaattacctaaacagtgggaattctagacacatttcaattggtggaaaaacatgtac

SEQ ID NO: 939 - DNA, 120 bp, Artificial Sequence
  MET
tggaaattacctaaacagtgggaattctagacacatttcaattggtggaaaaacatgtactttaaaaaggtgttgtaaatttattttttgttgcatctgtcaatttgaattaatatctgt

SEQ ID NO: 940 - DNA, 120 bp, Artificial Sequence
  MET
taatagctaaaattcacttccttaattttttttgttcagtgtgtcaaacagtattcttgaatgttataccccagcccaaaccatttcaactgagtttgctgttaaattgaaaattgactt

SEQ ID NO: 941 - DNA, 120 bp, Artificial Sequence
  MET
atgttataccccagcccaaaccatttcaactgagtttgctgttaaattgaaaattgacttagccaaccgagagacaagcatcttcagttaccgtgaagatcccattgtctatgaaattca

SEQ ID NO: 942 - DNA, 120 bp, Artificial Sequence
  MET
agccaaccgagagacaagcatcttcagttaccgtgaagatcccattgtctatgaaattcatccaaccaaatcttttattaggtaagtagaagcttctgatgggtataagaaaacaatgaa

SEQ ID NO: 943 - DNA, 120 bp, Artificial Sequence
  MET
ctgtaatcagtgcaggtgattaaattgaatccctctcttacagtacttggtggaaagaacctctcaacattgtcagttttctattttgctttgccagtggtgggagcacaataacaggtg

SEQ ID NO: 944 - DNA, 120 bp, Artificial Sequence
  MET
ctctcaacattgtcagttttctattttgctttgccagtggtgggagcacaataacaggtgttgggaaaaacctgaattcagttagtgtcccgagaatggtcataaatgtgcatgaagcag

SEQ ID NO: 945 - DNA, 120 bp, Artificial Sequence
  MET
ttgggaaaaacctgaattcagttagtgtcccgagaatggtcataaatgtgcatgaagcaggaaggaactttacagtggtaagtcctttgagcaatggttctactcagagctctgcatctt

SEQ ID NO: 946 - DNA, 120 bp, Artificial Sequence
  MET
tctttctctaggcatgtcaacatcgctctaattcagagataatctgttgtaccactccttccctgcaacagctgaatctgcaactccccctgaaaaccaaagcctttttcatgttagatg

SEQ ID NO: 947 - DNA, 120 bp, Artificial Sequence
  MET
ccctgcaacagctgaatctgcaactccccctgaaaaccaaagcctttttcatgttagatgggatcctttccaaatactttgatctcatttatgtacataatcctgtgtttaagccttttg

SEQ ID NO: 948 - DNA, 120 bp, Artificial Sequence
  MET
ggatcctttccaaatactttgatctcatttatgtacataatcctgtgtttaagccttttgaaaagccagtgatgatctcaatgggcaatgaaaatgtactggaaattaaggtaagaaatg

SEQ ID NO: 949 - DNA, 120 bp, Artificial Sequence
  MET
tgaagtgttaacaacctttttttttttttttcctttcagggaaatgatattgaccctgaagcagttaaaggtgaagtgttaaaagttggaaataagagctgtgagaatatacacttacat

SEQ ID NO: 950 - DNA, 120 bp, Artificial Sequence
  MET
gcagttaaaggtgaagtgttaaaagttggaaataagagctgtgagaatatacacttacattctgaagccgttttatgcacggtccccaatgacctgctgaaattgaacagcgagctaaat

SEQ ID NO: 951 - DNA, 120 bp, Artificial Sequence
  MET
tctgaagccgttttatgcacggtccccaatgacctgctgaaattgaacagcgagctaaatatagaggtgggattcctgcattcctctcatgatgtaaataaggaagccagtgtaattatg

SEQ ID NO: 952 - DNA, 120 bp, Artificial Sequence
  MET
atagaggtgggattcctgcattcctctcatgatgtaaataaggaagccagtgtaattatgttattctcaggcttaaaataaatcattaaagctcatttatgtgtgggttttggctcatca

SEQ ID NO: 953 - DNA, 120 bp, Artificial Sequence
  MET
atcatggctaaatgctgacttttctttatttgtcatttttagtggaagcaagcaatttcttcaaccgtccttggaaaagtaatagttcaaccagatcagaatttcacaggattgattgct

SEQ ID NO: 954 - DNA, 120 bp, Artificial Sequence
  MET
tcaaccgtccttggaaaagtaatagttcaaccagatcagaatttcacaggattgattgctggtgttgtctcaatatcaacagcactgttattactacttgggtttttcctgtggctgaaa

SEQ ID NO: 955 - DNA, 120 bp, Artificial Sequence
  MET
ggtgttgtctcaatatcaacagcactgttattactacttgggtttttcctgtggctgaaaaagagaaagcaaattaaaggtgcatttttgttactgttcatttttagaagttaccttaag

SEQ ID NO: 956 - DNA, 120 bp, Artificial Sequence
  MET
ggcccatgatagccgtctttaacaagctctttctttctctctgttttaagatctgggcagtgaattagttcgctacgatgcaagagtacacactcctcatttggataggcttgtaagtgc

SEQ ID NO: 957 - DNA, 120 bp, Artificial Sequence
  MET
tgaattagttcgctacgatgcaagagtacacactcctcatttggataggcttgtaagtgcccgaagtgtaagcccaactacagaaatggtttcaaatgaatctgtagactaccgagctac

SEQ ID NO: 958 - DNA, 120 bp, Artificial Sequence
  MET
ccgaagtgtaagcccaactacagaaatggtttcaaatgaatctgtagactaccgagctacttttccagaaggtatatttcagtttattgttctgagaaatacctatacatatacctcagt

SEQ ID NO: 959 - DNA, 120 bp, Artificial Sequence
  MET
ctgttgttctttaataattttccttcatcttacagatcagtttcctaattcatctcagaacggttcatgccgacaagtgcagtatcctctgacagacatgtcccccatcctaactagtgg

SEQ ID NO: 960 - DNA, 120 bp, Artificial Sequence
  MET
cggttcatgccgacaagtgcagtatcctctgacagacatgtcccccatcctaactagtggggactctgatatatccagtccattactgcaaaatactgtccacattgacctcagtgctct

SEQ ID NO: 961 - DNA, 120 bp, Artificial Sequence
  MET
ggactctgatatatccagtccattactgcaaaatactgtccacattgacctcagtgctctaaatccagagctggtccaggcagtgcagcatgtagtgattgggcccagtagcctgattgt

SEQ ID NO: 962 - DNA, 120 bp, Artificial Sequence
  MET
aaatccagagctggtccaggcagtgcagcatgtagtgattgggcccagtagcctgattgtgcatttcaatgaagtcataggaagaggtaagtatttccactcagctttttgttaaatacg

SEQ ID NO: 963 - DNA, 120 bp, Artificial Sequence
  MET
ttcataattaaatgttacgcagtgctaaccaagttctttcttttgcacagggcattttggttgtgtatatcatgggactttgttggacaatgatggcaagaaaattcactgtgctgtgaa

SEQ ID NO: 964 - DNA, 120 bp, Artificial Sequence
  MET
ttgtgtatatcatgggactttgttggacaatgatggcaagaaaattcactgtgctgtgaaatccttgaacagtaagtggcattttatttaaccatggagtatacttttgtggtttgcaac

SEQ ID NO: 965 - DNA, 120 bp, Artificial Sequence
  MET
gttaatgtctccaccactggatttctcaggaatcactgacataggagaagtttcccaatttctgaccgagggaatcatcatgaaagattttagtcatcccaatgtcctctcgctcctggg

SEQ ID NO: 966 - DNA, 120 bp, Artificial Sequence
  MET
tctgaccgagggaatcatcatgaaagattttagtcatcccaatgtcctctcgctcctgggaatctgcctgcgaagtgaagggtctccgctggtggtcctaccatacatgaaacatggaga

SEQ ID NO: 967 - DNA, 120 bp, Artificial Sequence
  MET
aatctgcctgcgaagtgaagggtctccgctggtggtcctaccatacatgaaacatggagatcttcgaaatttcattcgaaatgagactcatgtaagttgactgccaagcttactaactgg

SEQ ID NO: 968 - DNA, 120 bp, Artificial Sequence
  MET
ttctaaggtcaaaattagaacagtagatgcttagtttatgcttttctaactctctttgactgcagaatccaactgtaaaagatcttattggctttggtcttcaagtagccaaaggcatga

SEQ ID NO: 969 - DNA, 120 bp, Artificial Sequence
  MET
tgcagaatccaactgtaaaagatcttattggctttggtcttcaagtagccaaaggcatgaaatatcttgcaagcaaaaagtttgtccacagagacttggctgcaagaaactgtatgtaag

SEQ ID NO: 970 - DNA, 120 bp, Artificial Sequence
  MET
aatatcttgcaagcaaaaagtttgtccacagagacttggctgcaagaaactgtatgtaagtatcagaatctctgtgccacaatccaaattaagtgacaaggaggaatctgtttcccactg

SEQ ID NO: 971 - DNA, 120 bp, Artificial Sequence
  MET
tttcagccacgggtaataatttttgtcctttctgtaggctggatgaaaaattcacagtcaaggttgctgattttggtcttgccagagacatgtatgataaagaatactatagtgtacaca

SEQ ID NO: 972 - DNA, 120 bp, Artificial Sequence
  MET
aggttgctgattttggtcttgccagagacatgtatgataaagaatactatagtgtacacaacaaaacaggtgcaaagctgccagtgaagtggatggctttggaaagtctgcaaactcaaa

SEQ ID NO: 973 - DNA, 120 bp, Artificial Sequence
  MET
acaaaacaggtgcaaagctgccagtgaagtggatggctttggaaagtctgcaaactcaaaagtttaccaccaagtcagatgtggtaatgtattggttatctctgagtttctcctctttta

SEQ ID NO: 974 - DNA, 120 bp, Artificial Sequence
  MET
atatgtatggtcacatctctcacctcatctgtcctgtttcttgttttactagtggtcctttggcgtgctcctctgggagctgatgacaagaggagccccaccttatcctgacgtaaacac

SEQ ID NO: 975 - DNA, 120 bp, Artificial Sequence
  MET
tggcgtgctcctctgggagctgatgacaagaggagccccaccttatcctgacgtaaacacctttgatataactgtttacttgttgcaagggagaagactcctacaacccgaatactgccc

SEQ ID NO: 976 - DNA, 120 bp, Artificial Sequence
  MET
ctttgatataactgtttacttgttgcaagggagaagactcctacaacccgaatactgcccagaccccttgtaagtagtctttctgtacctcttacgttctttacttttacagaaatgcct

SEQ ID NO: 977 - DNA, 120 bp, Artificial Sequence
  MET
ctcttacagcatgtctttctttttggaacagatatgaagtaatgctaaaatgctggcaccctaaagccgaaatgcgcccatccttttctgaactggtgtcccggatatcagcgatcttct

SEQ ID NO: 978 - DNA, 120 bp, Artificial Sequence
  MET
ctaaagccgaaatgcgcccatccttttctgaactggtgtcccggatatcagcgatcttctctactttcattggggagcactatgtccatgtgaacgctacttatgtgaacgtaaaatgtg

SEQ ID NO: 979 - DNA, 120 bp, Artificial Sequence
  MET
ctactttcattggggagcactatgtccatgtgaacgctacttatgtgaacgtaaaatgtgtcgctccgtatccttctctgttgtcatcagaagataacgctgatgatgaggtggacacac

SEQ ID NO: 980 - DNA, 120 bp, Artificial Sequence
  MET
tcgctccgtatccttctctgttgtcatcagaagataacgctgatgatgaggtggacacacgaccagcctccttctgggagacatcatagtgctagtactatgtcaaagcaacagtccaca

SEQ ID NO: 981 - DNA, 120 bp, Artificial Sequence
  MET-E14
cccatgagttctgggcactgggtcaaagtctcctggggcccatgatagccgtctttaacaagctctttctttctctctgttttaagatctgggcagtgaattagttcgctacgatgcaag

SEQ ID NO: 982 - DNA, 120 bp, Artificial Sequence
  MET-E14
aaagtctcctggggcccatgatagccgtctttaacaagctctttctttctctctgttttaagatctgggcagtgaattagttcgctacgatgcaagagtacacactcctcatttggatag

SEQ ID NO: 983 - DNA, 120 bp, Artificial Sequence
  MET-E14
ccgtctttaacaagctctttctttctctctgttttaagatctgggcagtgaattagttcgctacgatgcaagagtacacactcctcatttggataggcttgtaagtgcccgaagtgtaag

SEQ ID NO: 984 - DNA, 120 bp, Artificial Sequence
  MET-E14
ctctctgttttaagatctgggcagtgaattagttcgctacgatgcaagagtacacactcctcatttggataggcttgtaagtgcccgaagtgtaagcccaactacagaaatggtttcaaa

SEQ ID NO: 985 - DNA, 120 bp, Artificial Sequence; identical to SEQ ID NO: 957
  MET-E14

SEQ ID NO: 986 - DNA, 120 bp, Artificial Sequence
  MET-E14
agtacacactcctcatttggataggcttgtaagtgcccgaagtgtaagcccaactacagaaatggtttcaaatgaatctgtagactaccgagctacttttccagaaggtatatttcagtt

SEQ ID NO: 987 - DNA, 120 bp, Artificial Sequence
  MET-E14
gcttgtaagtgcccgaagtgtaagcccaactacagaaatggtttcaaatgaatctgtagactaccgagctacttttccagaaggtatatttcagtttattgttctgagaaatacctatac

SEQ ID NO: 988 - DNA, 120 bp, Artificial Sequence
  MET-E14
cccaactacagaaatggtttcaaatgaatctgtagactaccgagctacttttccagaaggtatatttcagtttattgttctgagaaatacctatacatatacctcagtgggttgtgacat

SEQ ID NO: 989 - DNA, 120 bp, Artificial Sequence
  MET-E14
tgaatctgtagactaccgagctacttttccagaaggtatatttcagtttattgttctgagaaatacctatacatatacctcagtgggttgtgacattgttgtttatttttggttttgcat

SEQ ID NO: 990 - DNA, 120 bp, Artificial Sequence
  MET-E15
ccattaaatgaggttttactgttgttctttaataattttccttcatcttacagatcagtttcctaattcatctcagaacggttcatgccgacaagtgcagtatcctctgacagacatgtc

SEQ ID NO: 991 - DNA, 120 bp, Artificial Sequence
  MET-E15
ttctttaataattttccttcatcttacagatcagtttcctaattcatctcagaacggttcatgccgacaagtgcagtatcctctgacagacatgtcccccatcctaactagtggggactc

SEQ ID NO: 992 - DNA, 120 bp, Artificial Sequence
  MET-E15
tacagatcagtttcctaattcatctcagaacggttcatgccgacaagtgcagtatcctctgacagacatgtcccccatcctaactagtggggactctgatatatccagtccattactgca

SEQ ID NO: 993 - DNA, 120 bp, Artificial Sequence
  MET-E15
tcagaacggttcatgccgacaagtgcagtatcctctgacagacatgtcccccatcctaactagtggggactctgatatatccagtccattactgcaaaatactgtccacattgacctcag

SEQ ID NO: 994 - DNA, 120 bp, Artificial Sequence
  MET-E15
gcagtatcctctgacagacatgtcccccatcctaactagtggggactctgatatatccagtccattactgcaaaatactgtccacattgacctcagtgctctaaatccagagctggtcca

SEQ ID NO: 995 - DNA, 120 bp, Artificial Sequence
  MET-E15
ccccatcctaactagtggggactctgatatatccagtccattactgcaaaatactgtccacattgacctcagtgctctaaatccagagctggtccaggcagtgcagcatgtagtgattgg

SEQ ID NO: 996 - DNA, 120 bp, Artificial Sequence
  MET-E15
tgatatatccagtccattactgcaaaatactgtccacattgacctcagtgctctaaatccagagctggtccaggcagtgcagcatgtagtgattgggcccagtagcctgattgtgcattt

SEQ ID NO: 997 - DNA, 120 bp, Artificial Sequence
  MET-E15
aaatactgtccacattgacctcagtgctctaaatccagagctggtccaggcagtgcagcatgtagtgattgggcccagtagcctgattgtgcatttcaatgaagtcataggaagaggtaa

SEQ ID NO: 998 - DNA, 120 bp, Artificial Sequence
  MET-E15
tgctctaaatccagagctggtccaggcagtgcagcatgtagtgattgggcccagtagcctgattgtgcatttcaatgaagtcataggaagaggtaagtatttccactcagctttttgtta

SEQ ID NO: 999 - DNA, 120 bp, Artificial Sequence
  MET-E15
ggcagtgcagcatgtagtgattgggcccagtagcctgattgtgcatttcaatgaagtcataggaagaggtaagtatttccactcagctttttgttaaatacgattttccagtaagcattt

SEQ ID NO: 1000 - DNA, 120 bp, Artificial Sequence
  MET-E16
atagaaagaagaaagaataaaatgaagctcataaagggtttgataaataattatttcataattaaatgttacgcagtgctaaccaagttctttcttttgcacagggcattttggttgtgt

SEQ ID NO: 1001 - DNA, 120 bp, Artificial Sequence
  MET-E16
aagctcataaagggtttgataaataattatttcataattaaatgttacgcagtgctaaccaagttctttcttttgcacagggcattttggttgtgtatatcatgggactttgttggacaa

SEQ ID NO: 1002 - DNA, 120 bp, Artificial Sequence
  MET-E16
aattatttcataattaaatgttacgcagtgctaaccaagttctttcttttgcacagggcattttggttgtgtatatcatgggactttgttggacaatgatggcaagaaaattcactgtgc

SEQ ID NO: 1003 - DNA, 120 bp, Artificial Sequence
  MET-E16
gcagtgctaaccaagttctttcttttgcacagggcattttggttgtgtatatcatgggactttgttggacaatgatggcaagaaaattcactgtgctgtgaaatccttgaacagtaagtg

SEQ ID NO: 1004 - DNA, 120 bp, Artificial Sequence
  MET-E16
ttgcacagggcattttggttgtgtatatcatgggactttgttggacaatgatggcaagaaaattcactgtgctgtgaaatccttgaacagtaagtggcattttatttaaccatggagtat

SEQ ID NO: 1005 - DNA, 120 bp, Artificial Sequence
  MET-E16
atatcatgggactttgttggacaatgatggcaagaaaattcactgtgctgtgaaatccttgaacagtaagtggcattttatttaaccatggagtatacttttgtggtttgcaacctaata

SEQ ID NO: 1006 - DNA, 120 bp, Artificial Sequence
  MET-E16
tgatggcaagaaaattcactgtgctgtgaaatccttgaacagtaagtggcattttatttaaccatggagtatacttttgtggtttgcaacctaataaatagcttataataaaacgttgat

SEQ ID NO: 1007 - DNA, 120 bp, Artificial Sequence
  MET-E16
tgtgaaatccttgaacagtaagtggcattttatttaaccatggagtatacttttgtggtttgcaacctaataaatagcttataataaaacgttgatttacactttccccttgtggaaaaa

SEQ ID NO: 1008 - DNA, 120 bp, Artificial Sequence
  MET-E17
aagtattcactgttccataatgaagttaatgtctccaccactggatttctcaggaatcactgacataggagaagtttcccaatttctgaccgagggaatcatcatgaaagattttagtca

SEQ ID NO: 1009 - DNA, 120 bp, Artificial Sequence; identical to SEQ ID NO: 965
  MET-E17

SEQ ID NO: 1010 - DNA, 120 bp, Artificial Sequence
  MET-E17
agtttcccaatttctgaccgagggaatcatcatgaaagattttagtcatcccaatgtcctctcgctcctgggaatctgcctgcgaagtgaagggtctccgctggtggtcctaccatacat

SEQ ID NO: 1011 - DNA, 120 bp, Artificial Sequence
  MET-E17
aatcatcatgaaagattttagtcatcccaatgtcctctcgctcctgggaatctgcctgcgaagtgaagggtctccgctggtggtcctaccatacatgaaacatggagatcttcgaaattt

SEQ ID NO: 1012 - DNA, 120 bp, Artificial Sequence; identical to SEQ ID NO: 967
  MET-E17

SEQ ID NO: 1013 - DNA, 120 bp, Artificial Sequence
  MET-E17
tccgctggtggtcctaccatacatgaaacatggagatcttcgaaatttcattcgaaatgagactcatgtaagttgactgccaagcttactaactggcaaactagctgtaagccagccatc

SEQ ID NO: 1014 - DNA, 120 bp, Artificial Sequence
  MET-E18
tttttataaataaatatttcagaattctaaggtcaaaattagaacagtagatgcttagtttatgcttttctaactctctttgactgcagaatccaactgtaaaagatcttattggctttg

SEQ ID NO: 1015 - DNA, 120 bp, Artificial Sequence; identical to SEQ ID NO: 968
  MET-E18

SEQ ID NO: 1016 - DNA, 120 bp, Artificial Sequence
  MET-E18
agatgcttagtttatgcttttctaactctctttgactgcagaatccaactgtaaaagatcttattggctttggtcttcaagtagccaaaggcatgaaatatcttgcaagcaaaaagtttg

SEQ ID NO: 1017 - DNA, 120 bp, Artificial Sequence
  MET-E18
gtcttcaagtagccaaaggcatgaaatatcttgcaagcaaaaagtttgtccacagagacttggctgcaagaaactgtatgtaagtatcagaatctctgtgccacaatccaaattaagtga

SEQ ID NO: 1018 - DNA, 120 bp, Artificial Sequence; identical to SEQ ID NO: 970
  MET-E18

SEQ ID NO: 1019 - DNA, 120 bp, Artificial Sequence
  MET-E18
tccacagagacttggctgcaagaaactgtatgtaagtatcagaatctctgtgccacaatccaaattaagtgacaaggaggaatctgtttcccactgttcaatgctagttaagctgttttc

SEQ ID NO: 1020 - DNA, 120 bp, Artificial Sequence
  MET-E18
actgtatgtaagtatcagaatctctgtgccacaatccaaattaagtgacaaggaggaatctgtttcccactgttcaatgctagttaagctgttttctcttcttatgcaaaagtcctttat

SEQ ID NO: 1021 - DNA, 120 bp, Artificial Sequence
  MET-E19
tcagcatcattgtaaattattctatttcagccacgggtaataatttttgtcctttctgtaggctggatgaaaaattcacagtcaaggttgctgattttggtcttgccagagacatgtatg

SEQ ID NO: 1022 - DNA, 120 bp, Artificial Sequence; identical to SEQ ID NO: 971
  MET-E19

SEQ ID NO: 1023 - DNA, 120 bp, Artificial Sequence
  MET-E19
aattcacagtcaaggttgctgattttggtcttgccagagacatgtatgataaagaatactatagtgtacacaacaaaacaggtgcaaagctgccagtgaagtggatggctttggaaagtc

SEQ ID NO: 1024 - DNA, 120 bp, Artificial Sequence
  MET-E19
ttggtcttgccagagacatgtatgataaagaatactatagtgtacacaacaaaacaggtgcaaagctgccagtgaagtggatggctttggaaagtctgcaaactcaaaagtttaccacca

SEQ ID NO: 1025 - DNA, 120 bp, Artificial Sequence; identical to SEQ ID NO: 973
  MET-E19

SEQ ID NO: 1026 - DNA, 120 bp, Artificial Sequence
  MET-E19
tgaagtggatggctttggaaagtctgcaaactcaaaagtttaccaccaagtcagatgtggtaatgtattggttatctctgagtttctcctcttttactttcatatccaactttttttgaa

SEQ ID NO: 1027 - DNA, 120 bp, Artificial Sequence
  MET-E2
ttctcttcatttctgacaactgaactgctctcgccttgaacctgttttggcagataaacctctcataatgaaggcccccgctgtgcttgcacctggcatcctcgtgctcctgtttacctt

SEQ ID NO: 1028 - DNA, 120 bp, Artificial Sequence
  MET-E2
ctgctctcgccttgaacctgttttggcagataaacctctcataatgaaggcccccgctgtgcttgcacctggcatcctcgtgctcctgtttaccttggtgcagaggagcaatggggagtg

SEQ ID NO: 1029 - DNA, 120 bp, Artificial Sequence
  MET-E2
ggcagataaacctctcataatgaaggcccccgctgtgcttgcacctggcatcctcgtgctcctgtttaccttggtgcagaggagcaatggggagtgtaaagaggcactagcaaagtccga

SEQ ID NO: 1030 - DNA, 120 bp, Artificial Sequence
  MET-E2
ggcccccgctgtgcttgcacctggcatcctcgtgctcctgtttaccttggtgcagaggagcaatggggagtgtaaagaggcactagcaaagtccgagatgaatgtgaatatgaagtatca

SEQ ID NO: 1031 - DNA, 120 bp, Artificial Sequence
  MET-E2
catcctcgtgctcctgtttaccttggtgcagaggagcaatggggagtgtaaagaggcactagcaaagtccgagatgaatgtgaatatgaagtatcagcttcccaacttcaccgcggaaac

SEQ ID NO: 1032 - DNA, 120 bp, Artificial Sequence
  MET-E2
ggtgcagaggagcaatggggagtgtaaagaggcactagcaaagtccgagatgaatgtgaatatgaagtatcagcttcccaacttcaccgcggaaacacccatccagaatgtcattctaca

SEQ ID NO: 1033 - DNA, 120 bp, Artificial Sequence
  MET-E2
taaagaggcactagcaaagtccgagatgaatgtgaatatgaagtatcagcttcccaacttcaccgcggaaacacccatccagaatgtcattctacatgagcatcacattttccttggtgc

SEQ ID NO: 1034 - DNA, 120 bp, Artificial Sequence
  MET-E2
gatgaatgtgaatatgaagtatcagcttcccaacttcaccgcggaaacacccatccagaatgtcattctacatgagcatcacattttccttggtgccactaactacatttatgttttaaa

SEQ ID NO: 1035 - DNA, 120 bp, Artificial Sequence
  MET-E2
gcttcccaacttcaccgcggaaacacccatccagaatgtcattctacatgagcatcacattttccttggtgccactaactacatttatgttttaaatgaggaagaccttcagaaggttgc

SEQ ID NO: 1036 - DNA, 120 bp, Artificial Sequence
  MET-E2
acccatccagaatgtcattctacatgagcatcacattttccttggtgccactaactacatttatgttttaaatgaggaagaccttcagaaggttgctgagtacaagactgggcctgtgct

SEQ ID NO: 1037 - DNA, 120 bp, Artificial Sequence
  MET-E2
tgagcatcacattttccttggtgccactaactacatttatgttttaaatgaggaagaccttcagaaggttgctgagtacaagactgggcctgtgctggaacacccagattgtttcccatg

SEQ ID NO: 1038 - DNA, 120 bp, Artificial Sequence
  MET-E2
cactaactacatttatgttttaaatgaggaagaccttcagaaggttgctgagtacaagactgggcctgtgctggaacacccagattgtttcccatgtcaggactgcagcagcaaagccaa

SEQ ID NO: 1039 - DNA, 120 bp, Artificial Sequence
  MET-E2
tgaggaagaccttcagaaggttgctgagtacaagactgggcctgtgctggaacacccagattgtttcccatgtcaggactgcagcagcaaagccaatttatcaggaggtgtttggaaaga

SEQ ID NO: 1040 - DNA, 120 bp, Artificial Sequence
  MET-E2
tgagtacaagactgggcctgtgctggaacacccagattgtttcccatgtcaggactgcagcagcaaagccaatttatcaggaggtgtttggaaagataacatcaacatggctctagttgt

SEQ ID NO: 1041 - DNA, 120 bp, Artificial Sequence
  MET-E2
ggaacacccagattgtttcccatgtcaggactgcagcagcaaagccaatttatcaggaggtgtttggaaagataacatcaacatggctctagttgtcgacacctactatgatgatcaact

SEQ ID NO: 1042 - DNA, 120 bp, Artificial Sequence
  MET-E2
tcaggactgcagcagcaaagccaatttatcaggaggtgtttggaaagataacatcaacatggctctagttgtcgacacctactatgatgatcaactcattagctgtggcagcgtcaacag

SEQ ID NO: 1043 - DNA, 120 bp, Artificial Sequence
  MET-E2
tttatcaggaggtgtttggaaagataacatcaacatggctctagttgtcgacacctactatgatgatcaactcattagctgtggcagcgtcaacagagggacctgccagcgacatgtctt

SEQ ID NO: 1044 - DNA, 120 bp, Artificial Sequence
  MET-E2
taacatcaacatggctctagttgtcgacacctactatgatgatcaactcattagctgtggcagcgtcaacagagggacctgccagcgacatgtctttccccacaatcatactgctgacat

SEQ ID NO: 1045 - DNA, 120 bp, Artificial Sequence
  MET-E2
cgacacctactatgatgatcaactcattagctgtggcagcgtcaacagagggacctgccagcgacatgtctttccccacaatcatactgctgacatacagtcggaggttcactgcatatt

SEQ ID NO: 1046 - DNA, 120 bp, Artificial Sequence
  MET-E2
cattagctgtggcagcgtcaacagagggacctgccagcgacatgtctttccccacaatcatactgctgacatacagtcggaggttcactgcatattctccccacagatagaagagcccag

SEQ ID NO: 1047 - DNA, 120 bp, Artificial Sequence
  MET-E2
agggacctgccagcgacatgtctttccccacaatcatactgctgacatacagtcggaggttcactgcatattctccccacagatagaagagcccagccagtgtcctgactgtgtggtgag

SEQ ID NO: 1048 - DNA, 120 bp, Artificial Sequence
  MET-E2
tccccacaatcatactgctgacatacagtcggaggttcactgcatattctccccacagatagaagagcccagccagtgtcctgactgtgtggtgagcgccctgggagccaaagtcctttc

SEQ ID NO: 1049 - DNA, 120 bp, Artificial Sequence
  MET-E2
acagtcggaggttcactgcatattctccccacagatagaagagcccagccagtgtcctgactgtgtggtgagcgccctgggagccaaagtcctttcatctgtaaaggaccggttcatcaa

SEQ ID NO: 1050 - DNA, 120 bp, Artificial Sequence
  MET-E2
ctccccacagatagaagagcccagccagtgtcctgactgtgtggtgagcgccctgggagccaaagtcctttcatctgtaaaggaccggttcatcaacttctttgtaggcaataccataaa

SEQ ID NO: 1051 - DNA, 120 bp, Artificial Sequence
  MET-E2
ccagtgtcctgactgtgtggtgagcgccctgggagccaaagtcctttcatctgtaaaggaccggttcatcaacttctttgtaggcaataccataaattcttcttatttcccagatcatcc

SEQ ID NO: 1052 - DNA, 120 bp, Artificial Sequence
  MET-E2
cgccctgggagccaaagtcctttcatctgtaaaggaccggttcatcaacttctttgtaggcaataccataaattcttcttatttcccagatcatccattgcattcgatatcagtgagaag

SEQ ID NO: 1053 - DNA, 120 bp, Artificial Sequence
  MET-E2
atctgtaaaggaccggttcatcaacttctttgtaggcaataccataaattcttcttatttcccagatcatccattgcattcgatatcagtgagaaggctaaaggaaacgaaagatggttt

SEQ ID NO: 1054 - DNA, 120 bp, Artificial Sequence
  MET-E2
cttctttgtaggcaataccataaattcttcttatttcccagatcatccattgcattcgatatcagtgagaaggctaaaggaaacgaaagatggttttatgtttttgacggaccagtccta

SEQ ID NO: 1055 - DNA, 120 bp, Artificial Sequence
  MET-E2
ttcttcttatttcccagatcatccattgcattcgatatcagtgagaaggctaaaggaaacgaaagatggttttatgtttttgacggaccagtcctacattgatgttttacctgagttcag

SEQ ID NO: 1056 - DNA, 120 bp, Artificial Sequence
  MET-E2
attgcattcgatatcagtgagaaggctaaaggaaacgaaagatggttttatgtttttgacggaccagtcctacattgatgttttacctgagttcagagattcttaccccattaagtatgt

SEQ ID NO: 1057 - DNA, 120 bp, Artificial Sequence
  MET-E2
gctaaaggaaacgaaagatggttttatgtttttgacggaccagtcctacattgatgttttacctgagttcagagattcttaccccattaagtatgtccatgcctttgaaagcaacaattt

SEQ ID NO: 1058 - DNA, 120 bp, Artificial Sequence
  MET-E2
tatgtttttgacggaccagtcctacattgatgttttacctgagttcagagattcttaccccattaagtatgtccatgcctttgaaagcaacaattttatttacttcttgacggtccaaag

SEQ ID NO: 1059 - DNA, 120 bp, Artificial Sequence
  MET-E2
cattgatgttttacctgagttcagagattcttaccccattaagtatgtccatgcctttgaaagcaacaattttatttacttcttgacggtccaaagggaaactctagatgctcagacttt

SEQ ID NO: 1060 - DNA, 120 bp, Artificial Sequence
  MET-E2
agattcttaccccattaagtatgtccatgcctttgaaagcaacaattttatttacttcttgacggtccaaagggaaactctagatgctcagacttttcacacaagaataatcaggttctg

SEQ ID NO: 1061 - DNA, 120 bp, Artificial Sequence
  MET-E2
ccatgcctttgaaagcaacaattttatttacttcttgacggtccaaagggaaactctagatgctcagacttttcacacaagaataatcaggttctgttccataaactctggattgcattc

SEQ ID NO: 1062 - DNA, 120 bp, Artificial Sequence
  MET-E2
tatttacttcttgacggtccaaagggaaactctagatgctcagacttttcacacaagaataatcaggttctgttccataaactctggattgcattcctacatggaaatgcctctggagtg

SEQ ID NO: 1063 - DNA, 120 bp, Artificial Sequence
  MET-E2
ggaaactctagatgctcagacttttcacacaagaataatcaggttctgttccataaactctggattgcattcctacatggaaatgcctctggagtgtattctcacagaaaagagaaaaaa

SEQ ID NO: 1064 - DNA, 120 bp, Artificial Sequence
  MET-E2
tcacacaagaataatcaggttctgttccataaactctggattgcattcctacatggaaatgcctctggagtgtattctcacagaaaagagaaaaaagagatccacaaagaaggaagtgtt

SEQ ID NO: 1065 - DNA, 120 bp, Artificial Sequence
  MET-E2
ttccataaactctggattgcattcctacatggaaatgcctctggagtgtattctcacagaaaagagaaaaaagagatccacaaagaaggaagtgtttaatatacttcaggctgcgtatgt

SEQ ID NO: 1066 - DNA, 120 bp, Artificial Sequence
  MET-E2
ctacatggaaatgcctctggagtgtattctcacagaaaagagaaaaaagagatccacaaagaaggaagtgtttaatatacttcaggctgcgtatgtcagcaagcctggggcccagcttgc

SEQ ID NO: 1067 - DNA, 120 bp, Artificial Sequence
  MET-E2
tattctcacagaaaagagaaaaaagagatccacaaagaaggaagtgtttaatatacttcaggctgcgtatgtcagcaagcctggggcccagcttgctagacaaataggagccagcctgaa

SEQ ID NO: 1068 - DNA, 120 bp, Artificial Sequence
  MET-E2
gagatccacaaagaaggaagtgtttaatatacttcaggctgcgtatgtcagcaagcctggggcccagcttgctagacaaataggagccagcctgaatgatgacattcttttcggggtgtt

SEQ ID NO: 1069 - DNA, 120 bp, Artificial Sequence
  MET-E2
taatatacttcaggctgcgtatgtcagcaagcctggggcccagcttgctagacaaataggagccagcctgaatgatgacattcttttcggggtgttcgcacaaagcaagccagattctgc

SEQ ID NO: 1070 - DNA, 120 bp, Artificial Sequence
  MET-E2
cagcaagcctggggcccagcttgctagacaaataggagccagcctgaatgatgacattcttttcggggtgttcgcacaaagcaagccagattctgccgaaccaatggatcgatctgccat

SEQ ID NO: 1071 - DNA, 120 bp, Artificial Sequence
  MET-E2
tagacaaataggagccagcctgaatgatgacattcttttcggggtgttcgcacaaagcaagccagattctgccgaaccaatggatcgatctgccatgtgtgcattccctatcaaatatgt

SEQ ID NO: 1072 - DNA, 120 bp, Artificial Sequence
  MET-E2
tgatgacattcttttcggggtgttcgcacaaagcaagccagattctgccgaaccaatggatcgatctgccatgtgtgcattccctatcaaatatgtcaacgacttcttcaacaagatcgt

SEQ ID NO: 1073 - DNA, 120 bp, Artificial Sequence
  MET-E2
cgcacaaagcaagccagattctgccgaaccaatggatcgatctgccatgtgtgcattccctatcaaatatgtcaacgacttcttcaacaagatcgtcaacaaaaacaatgtgagatgtct

SEQ ID NO: 1074 - DNA, 120 bp, Artificial Sequence
  MET-E2
cgaaccaatggatcgatctgccatgtgtgcattccctatcaaatatgtcaacgacttcttcaacaagatcgtcaacaaaaacaatgtgagatgtctccagcatttttacggacccaatca

SEQ ID NO: 1075 - DNA, 120 bp, Artificial Sequence
  MET-E2
gtgtgcattccctatcaaatatgtcaacgacttcttcaacaagatcgtcaacaaaaacaatgtgagatgtctccagcatttttacggacccaatcatgagcactgctttaatagggtaag

SEQ ID NO: 1076 - DNA, 120 bp, Artificial Sequence
  MET-E2
caacgacttcttcaacaagatcgtcaacaaaaacaatgtgagatgtctccagcatttttacggacccaatcatgagcactgctttaatagggtaagtcacatcagttccccacttataaa

SEQ ID NO: 1077 - DNA, 120 bp, Artificial Sequence
  MET-E2
caacaaaaacaatgtgagatgtctccagcatttttacggacccaatcatgagcactgctttaatagggtaagtcacatcagttccccacttataaactgtgaggtataaattagaaataa

SEQ ID NO: 1078 - DNA, 120 bp, Artificial Sequence; identical to SEQ ID NO: 974
  MET-E20

SEQ ID NO: 1079 - DNA, 120 bp, Artificial Sequence
  MET-E20
tcatctgtcctgtttcttgttttactagtggtcctttggcgtgctcctctgggagctgatgacaagaggagccccaccttatcctgacgtaaacacctttgatataactgtttacttgtt

SEQ ID NO: 1080 - DNA, 120 bp, Artificial Sequence
  MET-E20
ctgggagctgatgacaagaggagccccaccttatcctgacgtaaacacctttgatataactgtttacttgttgcaagggagaagactcctacaacccgaatactgcccagaccccttgta

SEQ ID NO: 1081 - DNA, 120 bp, Artificial Sequence
  MET-E20
cccaccttatcctgacgtaaacacctttgatataactgtttacttgttgcaagggagaagactcctacaacccgaatactgcccagaccccttgtaagtagtctttctgtacctcttacg

SEQ ID NO: 1082 - DNA, 120 bp, Artificial Sequence; identical to SEQ ID NO: 976
  MET-E20

SEQ ID NO: 1083 - DNA, 120 bp, Artificial Sequence
  NRAS
attgcccaatactatatactaagatttgtaattatgccaagaaaccatatgctcaccttgttacatcaccacacatggcaatcccatacaaccctgagtcccatcatcactgctgttgag

SEQ ID NO: 1084 - DNA, 120 bp, Artificial Sequence
  NRAS
ttacatcaccacacatggcaatcccatacaaccctgagtcccatcatcactgctgttgagttttttcattcggtactggcgtatttctcttaccagtgtgtaaaaagcatcttcaacacc

SEQ ID NO: 1085 - DNA, 120 bp, Artificial Sequence
  NRAS
ttttttcattcggtactggcgtatttctcttaccagtgtgtaaaaagcatcttcaacaccctataaaaggaaaaaatgaaaaaaaatgagagagctagctcaacggacacaatccaaatt

SEQ ID NO: 1086 - DNA, 120 bp, Artificial Sequence
  NRAS
gatgcaaactcttgcacaaatgctgaaagctgtaccatacctgtctggtcttggctgaggtttcaatgaatggaatcccgtaactcttggccagttcgtgggcttgttttgtatcaactg

SEQ ID NO: 1087 - DNA, 120 bp, Artificial Sequence
  NRAS
tttcaatgaatggaatcccgtaactcttggccagttcgtgggcttgttttgtatcaactgtccttgttggcaaatcacacttgtttcccactagcaccataggtacatcatccgagtctt

SEQ ID NO: 1088 - DNA, 120 bp, Artificial Sequence
  NRAS
tccttgttggcaaatcacacttgtttcccactagcaccataggtacatcatccgagtcttttactcgcttaatctgctccctaaaaacgggaatatattatcagaacataagaaaaacaa

SEQ ID NO: 1089 - DNA, 120 bp, Artificial Sequence
  NRAS
atcctttcagagaaaataatgctcctagtacctgtagaggttaatatccgcaaatgacttgctattattgatggcaaatacacagaggaagccttcgcctgtcctcatgtattggtctct

SEQ ID NO: 1090 - DNA, 120 bp, Artificial Sequence
  NRAS
gctattattgatggcaaatacacagaggaagccttcgcctgtcctcatgtattggtctctcatggcactgtactcttcttgtccagctgtatccagtatgtccaacaaacaggtttcacc

SEQ ID NO: 1091 - DNA, 120 bp, Artificial Sequence
  NRAS
catggcactgtactcttcttgtccagctgtatccagtatgtccaacaaacaggtttcaccatctataaccacttgttttctgtaagaatcctgggggtgtggagggtaagggggcaggga

SEQ ID NO: 1092 - DNA, 120 bp, Artificial Sequence
  NRAS
atgggtaaagatgatccgacaagtgagagacaggatcaggtcagcgggctaccactgggcctcacctctatggtgggatcatattcatctacaaagtggttctggattagctggattgtc

SEQ ID NO: 1093 - DNA, 120 bp, Artificial Sequence
  NRAS
ctcacctctatggtgggatcatattcatctacaaagtggttctggattagctggattgtcagtgcgcttttcccaacaccacctgctccaaccaccaccagtttgtactcagtcatttca

SEQ ID NO: 1094 - DNA, 120 bp, Artificial Sequence
  NRAS
agtgcgcttttcccaacaccacctgctccaaccaccaccagtttgtactcagtcatttcacaccagcaagaacctgttggaaaccagtaatcagggttaattggcgagccacatctacag

SEQ ID NO: 1095 - DNA, 120 bp, Artificial Sequence
  NRAS-E2
gatgatccgacaagtgagagacaggatcaggtcagcgggctaccactgggcctcacctctatggtgggatcatattcatctacaaagtggttctggattagctggattgtcagtgcgctt

SEQ ID NO: 1096 - DNA, 120 bp, Artificial Sequence
  NRAS-E2
gatcaggtcagcgggctaccactgggcctcacctctatggtgggatcatattcatctacaaagtggttctggattagctggattgtcagtgcgcttttcccaacaccacctgctccaacc

SEQ ID NO: 1097 - DNA, 120 bp, Artificial Sequence
  NRAS-E2
tattcatctacaaagtggttctggattagctggattgtcagtgcgcttttcccaacaccacctgctccaaccaccaccagtttgtactcagtcatttcacaccagcaagaacctgttgga

SEQ ID NO: 1098 - DNA, 120 bp, Artificial Sequence
  NRAS-E2
attagctggattgtcagtgcgcttttcccaacaccacctgctccaaccaccaccagtttgtactcagtcatttcacaccagcaagaacctgttggaaaccagtaatcagggttaattggc

SEQ ID NO: 1099 - DNA, 120 bp, Artificial Sequence
  NRAS-E2
ttcccaacaccacctgctccaaccaccaccagtttgtactcagtcatttcacaccagcaagaacctgttggaaaccagtaatcagggttaattggcgagccacatctacagtactttaaa

SEQ ID NO: 1100 - DNA, 120 bp, Artificial Sequence
  NRAS-E3
ataaagattcagaacacaaagatcatcctttcagagaaaataatgctcctagtacctgtagaggttaatatccgcaaatgacttgctattattgatggcaaatacacagaggaagccttc

SEQ ID NO: 1101 - DNA, 120 bp, Artificial Sequence; identical to SEQ ID NO: 1089
  NRAS-E3

SEQ ID NO: 1102 - DNA, 120 bp, Artificial Sequence
  NRAS-E3
ctagtacctgtagaggttaatatccgcaaatgacttgctattattgatggcaaatacacagaggaagccttcgcctgtcctcatgtattggtctctcatggcactgtactcttcttgtcc

SEQ ID NO: 1103 - DNA, 120 bp, Artificial Sequence
  NRAS-E3
cgcaaatgacttgctattattgatggcaaatacacagaggaagccttcgcctgtcctcatgtattggtctctcatggcactgtactcttcttgtccagctgtatccagtatgtccaacaa

SEQ ID NO: 1104 - DNA, 120 bp, Artificial Sequence
  NRAS-E3
gcctgtcctcatgtattggtctctcatggcactgtactcttcttgtccagctgtatccagtatgtccaacaaacaggtttcaccatctataaccacttgttttctgtaagaatcctgggg

SEQ ID NO: 1105 - DNA, 120 bp, Artificial Sequence; identical to SEQ ID NO: 1091
  NRAS-E3

SEQ ID NO: 1106 - DNA, 120 bp, Artificial Sequence
  NRAS-E3
agctgtatccagtatgtccaacaaacaggtttcaccatctataaccacttgttttctgtaagaatcctgggggtgtggagggtaagggggcagggagggagggaagttcaatttttatta

SEQ ID NO: 1107 - DNA, 120 bp, Artificial Sequence
  NRAS-E4
cagagttaatcaactgatgcaaactcttgcacaaatgctgaaagctgtaccatacctgtctggtcttggctgaggtttcaatgaatggaatcccgtaactcttggccagttcgtgggctt

SEQ ID NO: 1108 - DNA, 120 bp, Artificial Sequence
  NRAS-E4
tcttgcacaaatgctgaaagctgtaccatacctgtctggtcttggctgaggtttcaatgaatggaatcccgtaactcttggccagttcgtgggcttgttttgtatcaactgtccttgttg

SEQ ID NO: 1109 - DNA, 120 bp, Artificial Sequence
  NRAS-E4
aggtttcaatgaatggaatcccgtaactcttggccagttcgtgggcttgttttgtatcaactgtccttgttggcaaatcacacttgtttcccactagcaccataggtacatcatccgagt

SEQ ID NO: 1110 - DNA, 120 bp, Artificial Sequence
  NRAS-E4
aactcttggccagttcgtgggcttgttttgtatcaactgtccttgttggcaaatcacacttgtttcccactagcaccataggtacatcatccgagtcttttactcgcttaatctgctccc

SEQ ID NO: 1111 - DNA, 120 bp, Artificial Sequence
  NRAS-E4
gttttgtatcaactgtccttgttggcaaatcacacttgtttcccactagcaccataggtacatcatccgagtcttttactcgcttaatctgctccctaaaaacgggaatatattatcaga

SEQ ID NO: 1112 - DNA, 120 bp, Artificial Sequence
  NRAS-E4
gcaaatcacacttgtttcccactagcaccataggtacatcatccgagtcttttactcgcttaatctgctccctaaaaacgggaatatattatcagaacataagaaaaacaagattaggct

SEQ ID NO: 1113 - DNA, 120 bp, Artificial Sequence
  PDGFRA
taggctccagggttgtttctatttgctaatgctgtttctgttgacttttgacttttctagtttcccagagctatggggacttcccatccggcgttcctggtcttaggctgtcttctcaca

SEQ ID NO: 1114 - DNA, 120 bp, Artificial Sequence
  PDGFRA
tttcccagagctatggggacttcccatccggcgttcctggtcttaggctgtcttctcacaggtacggagcccagtcctctctgagttccttgtttgggtgtcttgtttttttaagctttg

SEQ ID NO: 1115 - DNA, 120 bp, Artificial Sequence
  PDGFRA
agagcgtgcttccttttgcagggctgagcctaatcctctgccagctttcattaccctctatccttccaaatgaaaatgaaaaggttgtgcagctgaattcatccttttctctgagatgct

SEQ ID NO: 1116 - DNA, 120 bp, Artificial Sequence
  PDGFRA
tccttccaaatgaaaatgaaaaggttgtgcagctgaattcatccttttctctgagatgctttggggagagtgaagtgagctggcagtaccccatgtctgaagaagagagctccgatgtgg

SEQ ID NO: 1117 - DNA, 120 bp, Artificial Sequence
  PDGFRA
ttggggagagtgaagtgagctggcagtaccccatgtctgaagaagagagctccgatgtggaaatcagaaatgaagaaaacaacagcggcctttttgtgacggtcttggaagtgagcagtg

SEQ ID NO: 1118 - DNA, 120 bp, Artificial Sequence
  PDGFRA
aaatcagaaatgaagaaaacaacagcggcctttttgtgacggtcttggaagtgagcagtgcctcggcggcccacacagggttgtacacttgctattacaaccacactcagacagaagaga

SEQ ID NO: 1119 - DNA, 120 bp, Artificial Sequence
  PDGFRA
cctcggcggcccacacagggttgtacacttgctattacaaccacactcagacagaagagaatgagcttgaaggcaggcacatttacatctatgtgccaggtgagttggctgggtctccag

SEQ ID NO: 1120 - DNA, 120 bp, Artificial Sequence
  PDGFRA
gtctaatagagtcttcattcttttttaaaccacagacccagatgtagcctttgtacctctaggaatgacggattatttagtcatcgtggaggatgatgattctgccattataccttgtcg

SEQ ID NO: 1121 - DNA, 120 bp, Artificial Sequence
  PDGFRA
aggaatgacggattatttagtcatcgtggaggatgatgattctgccattataccttgtcgcacaactgatcccgagactcctgtaaccttacacaacagtgagggggtggtacctgcctc

SEQ ID NO: 1122 - DNA, 120 bp, Artificial Sequence
  PDGFRA
cacaactgatcccgagactcctgtaaccttacacaacagtgagggggtggtacctgcctcctacgacagcagacagggctttaatgggaccttcactgtagggccctatatctgtgaggc

SEQ ID NO: 1123 - DNA, 120 bp, Artificial Sequence
  PDGFRA
ctacgacagcagacagggctttaatgggaccttcactgtagggccctatatctgtgaggccaccgtcaaaggaaagaagttccagaccatcccatttaatgtttatgctttaaaaggtac

SEQ ID NO: 1124 - DNA, 120 bp, Artificial Sequence
  PDGFRA
caccgtcaaaggaaagaagttccagaccatcccatttaatgtttatgctttaaaaggtacttgtatcatctccttccttctttaaataagagtaacaggcaaaatcataaggtgcgtgta

SEQ ID NO: 1125 - DNA, 120 bp, Artificial Sequence
  PDGFRA
aacccaaactttataagatcctggctatcctgtggatttttaggcccttgtatttgttcttttttatagcaacatcagagctggatctagaaatggaagctcttaaaaccgtgtataagt

SEQ ID NO: 1126 - DNA, 120 bp, Artificial Sequence
  PDGFRA
tttttatagcaacatcagagctggatctagaaatggaagctcttaaaaccgtgtataagtcaggggaaacgattgtggtcacctgtgctgtttttaacaatgaggtggttgaccttcaat

SEQ ID NO: 1127 - DNA, 120 bp, Artificial Sequence
  PDGFRA
caggggaaacgattgtggtcacctgtgctgtttttaacaatgaggtggttgaccttcaatggacttaccctggagaagtggtaggtaccctcaaaacgtgcaatggcttggagcagagca

SEQ ID NO: 1128 - DNA, 120 bp, Artificial Sequence
  PDGFRA
tttaaaagtcggttttcttccccttttgctgtagaaaggcaaaggcatcacaatgctggaagaaatcaaagtcccatccatcaaattggtgtacactttgacggtccccgaggccacggt

SEQ ID NO: 1129 - DNA, 120 bp, Artificial Sequence
  PDGFRA
agaaatcaaagtcccatccatcaaattggtgtacactttgacggtccccgaggccacggtgaaagacagtggagattacgaatgtgctgcccgccaggctaccagggaggtcaaagaaat

SEQ ID NO: 1130 - DNA, 120 bp, Artificial Sequence
  PDGFRA
gaaagacagtggagattacgaatgtgctgcccgccaggctaccagggaggtcaaagaaatgaagaaagtcactatttctgtccatggtacattccgctttctaaaatgtcagttgtccat

SEQ ID NO: 1131 - DNA, 120 bp, Artificial Sequence
  PDGFRA
ttaatggaaactcttccctgtacagagaaaggtttcattgaaatcaaacccaccttcagccagttggaagctgtcaacctgcatgaagtcaaacattttgttgtagaggtgcgggcctac

SEQ ID NO: 1132 - DNA, 120 bp, Artificial Sequence
  PDGFRA
cagttggaagctgtcaacctgcatgaagtcaaacattttgttgtagaggtgcgggcctacccacctcccaggatatcctggctgaaaaacaatctgactctgattgaaaatctcactgag

SEQ ID NO: 1133 - DNA, 120 bp, Artificial Sequence
  PDGFRA
ccacctcccaggatatcctggctgaaaaacaatctgactctgattgaaaatctcactgagatcaccactgatgtggaaaagattcaggaaataaggtaaagaaactctctgcccaagtat

SEQ ID NO: 1134 - DNA, 120 bp, Artificial Sequence
  PDGFRA
tgtttaaacaattggaacttacttagctactgcttgttgaaacaaaatcctttttttaaaaggtatcgaagcaaattaaagctgatccgtgctaaggaagaagacagtggccattatact

SEQ ID NO: 1135 - DNA, 120 bp, Artificial Sequence
  PDGFRA
aggtatcgaagcaaattaaagctgatccgtgctaaggaagaagacagtggccattatactattgtagctcaaaatgaagatgctgtgaagagctatacttttgaactgttaactcaaggt

SEQ ID NO: 1136 - DNA, 120 bp, Artificial Sequence
  PDGFRA
attgtagctcaaaatgaagatgctgtgaagagctatacttttgaactgttaactcaaggtatgtaaagggagtataaagataatgctagctctgtagatgagtgtcttccaaggaaagcc

SEQ ID NO: 1137 - DNA, 120 bp, Artificial Sequence
  PDGFRA
tctcatatgttctgggacacgagctattccattctgacttctttctgcctcttgcagttccttcatccattctggacttggtcgatgatcaccatggctcaactgggggacagacggtga

SEQ ID NO: 1138 - DNA, 120 bp, Artificial Sequence
  PDGFRA
cttcatccattctggacttggtcgatgatcaccatggctcaactgggggacagacggtgaggtgcacagctgaaggcacgccgcttcctgatattgagtggatgatatgcaaagatatta

SEQ ID NO: 1139 - DNA, 120 bp, Artificial Sequence
  PDGFRA
ggtgcacagctgaaggcacgccgcttcctgatattgagtggatgatatgcaaagatattaagaagtatggaaaacagatgtgtcttcttctttcgtggtcagaatatttctcccttgaca

SEQ ID NO: 1140 - DNA, 120 bp, Artificial Sequence
  PDGFRA
acttaggccctttttctctctagatgtaataatgaaacttcctggactattttggccaacaatgtctcaaacatcatcacggagatccactcccgagacaggagtaccgtggagggccgt

SEQ ID NO: 1141 - DNA, 120 bp, Artificial Sequence
  PDGFRA
aatgtctcaaacatcatcacggagatccactcccgagacaggagtaccgtggagggccgtgtgactttcgccaaagtggaggagaccatcgccgtgcgatgcctggctaagaatctcctt

SEQ ID NO: 1142 - DNA, 120 bp, Artificial Sequence
  PDGFRA
gtgactttcgccaaagtggaggagaccatcgccgtgcgatgcctggctaagaatctccttggagctgagaaccgagagctgaagctggtggctcccagtgagttcctcaacagtcaggac

SEQ ID NO: 1143 - DNA, 120 bp, Artificial Sequence
  PDGFRA
tgccaggaaacttttcattgtgcctctctctcttgtcacgtagccctgcgttctgaactcacggtggctgctgcagtcctggtgctgttggtgattgtgatcatctcacttattgtcctg

SEQ ID NO: 1144 - DNA, 120 bp, Artificial Sequence
  PDGFRA
acggtggctgctgcagtcctggtgctgttggtgattgtgatcatctcacttattgtcctggttgtcatttggaaacaggtagatattttctcataaaactaaagatctttgaagccaatg

SEQ ID NO: 1145 - DNA, 120 bp, Artificial Sequence
  PDGFRA
ctggtgcactgggactttggtaattcaccagttacctgtcctggtcatttatagaaaccgaggtatgaaattcgctggagggtcattgaatcaatcagcccagatggacatgaatatatt

SEQ ID NO: 1146 - DNA, 120 bp, Artificial Sequence
  PDGFRA
aggtatgaaattcgctggagggtcattgaatcaatcagcccagatggacatgaatatatttatgtggacccgatgcagctgccttatgactcaagatgggagtttccaagagatggacta

SEQ ID NO: 1147 - DNA, 120 bp, Artificial Sequence
  PDGFRA
tatgtggacccgatgcagctgccttatgactcaagatgggagtttccaagagatggactagtgcttggtaagttccatggggtaacctcccaagactcccttttcccttgcacacaactt

SEQ ID NO: 1148 - DNA, 120 bp, Artificial Sequence
  PDGFRA
ggctacggtgcagaaagctgaggaggcgtctggagtttttgggtgttaatgattctgcctgcccacaggtcgggtcttggggtctggagcgtttgggaaggtggttgaaggaacagccta

SEQ ID NO: 1149 - DNA, 120 bp, Artificial Sequence
  PDGFRA
gcccacaggtcgggtcttggggtctggagcgtttgggaaggtggttgaaggaacagcctatggattaagccggtcccaacctgtcatgaaagttgcagtgaagatgctaaaacgtaagtg

SEQ ID NO: 1150 - DNA, 120 bp, Artificial Sequence
  PDGFRA
tggattaagccggtcccaacctgtcatgaaagttgcagtgaagatgctaaaacgtaagtgctccttcctggggattttttgagcacggggattttttgagcatggggatattaagggaat

SEQ ID NO: 1151 - DNA, 120 bp, Artificial Sequence
  PDGFRA
tttttttctgagaacaggaagttggtagctcagctggactgatatgtgatttattctttcaacagccacggccagatccagtgaaaaacaagctctcatgtctgaactgaagataatgac

SEQ ID NO: 1152 - DNA, 120 bp, Artificial Sequence; identical to SEQ ID NO: 26
  PDGFRA

SEQ ID NO: 1153 - DNA, 120 bp, Artificial Sequence
  PDGFRA
tcacctggggccacatttgaacattgtaaacttgctgggagcctgcaccaagtcaggtgggctcactgacctggagtgaggattttcactggacacatgtggttgtgaaaactgttcaat

SEQ ID NO: 1154 - DNA, 120 bp, Artificial Sequence
  PDGFRA
cttcattttcatacccatctcctaacggcttttgtccccataggccccatttacatcatcacagagtattgcttctatggagatttggtcaactatttgcataagaatagggatagcttc

SEQ ID NO: 1155 - DNA, 120 bp, Artificial Sequence
  PDGFRA
acagagtattgcttctatggagatttggtcaactatttgcataagaatagggatagcttcctgagccaccacccagagaagccaaagaaagagctggatatctttggattgaaccctgct

SEQ ID NO: 1156 - DNA, 120 bp, Artificial Sequence
  PDGFRA
ctgagccaccacccagagaagccaaagaaagagctggatatctttggattgaaccctgctgatgaaagcacacggaggtgggtgcaaagagagatgttgctgtctatcattatcttacag

SEQ ID NO: 1157 - DNA, 120 bp, Artificial Sequence
  PDGFRA
tgggagctcttctgctatttacatgtgatccacttagacctataaaatgcagctctggccagggatgcttgagttctggaaccttgcaagaactgtctgtggatctccaagctcgaggtc

SEQ ID NO: 1158 - DNA, 120 bp, Artificial Sequence
  PDGFRA
agggatgcttgagttctggaaccttgcaagaactgtctgtggatctccaagctcgaggtccttgctgaacctggacctataaatgacgtcaatgatagtgatccctactgcagaaatcta

SEQ ID NO: 1159 - DNA, 120 bp, Artificial Sequence
  PDGFRA
ggcaccctgggtaagatttctctttctgtttttacagctatgttattttatcttttgaaaacaatggtgactacatggacatgaagcaggctgatactacacagtatgtccccatgctag

SEQ ID NO: 1160 - DNA, 120 bp, Artificial Sequence
  PDGFRA
acaatggtgactacatggacatgaagcaggctgatactacacagtatgtccccatgctagaaaggaaagaggtttctaaatattccgacatccagagatcactctatgatcgtccagcct

SEQ ID NO: 1161 - DNA, 120 bp, Artificial Sequence
  PDGFRA
aaaggaaagaggtttctaaatattccgacatccagagatcactctatgatcgtccagcctcatataagaagaaatctatgttaggtaaaagtgtctatactcactctgggtgttgggact

SEQ ID NO: 1162 - DNA, 120 bp, Artificial Sequence
  PDGFRA
tctgcaacctgatgatttcctgctgcctgccagcaccaatacatttaatttcttttctgcagactcagaagtcaaaaacctcctttcagatgataactcagaaggccttactttattgga

SEQ ID NO: 1163 - DNA, 120 bp, Artificial Sequence
  PDGFRA
agactcagaagtcaaaaacctcctttcagatgataactcagaaggccttactttattggatttgttgagcttcacctatcaagttgcccgaggaatggagtttttggcttcaaaaaatgt

SEQ ID NO: 1164 - DNA, 120 bp, Artificial Sequence
  PDGFRA
tttgttgagcttcacctatcaagttgcccgaggaatggagtttttggcttcaaaaaatgtaagttcaaggaacacagacctttttagacccagatttcagtgagtggagtgtggacggag

SEQ ID NO: 1165 - DNA, 120 bp, Artificial Sequence
  PDGFRA
gtgatgctattcagctacagatggcttgatcctgagtcatttcttccttttccatgcagtgtgtccaccgtgatctggctgctcgcaacgtcctcctggcacaaggaaaaattgtgaaga

SEQ ID NO: 1166 - DNA, 120 bp, Artificial Sequence
  PDGFRA
gtgtccaccgtgatctggctgctcgcaacgtcctcctggcacaaggaaaaattgtgaagatctgtgactttggcctggccagagacatcatgcatgattcgaactatgtgtcgaaaggca

SEQ ID NO: 1167 - DNA, 120 bp, Artificial Sequence
  PDGFRA
tctgtgactttggcctggccagagacatcatgcatgattcgaactatgtgtcgaaaggcagtgtacgtcctcacttccctcactggtcaggctcatcctccttcactttaatctctaaag

SEQ ID NO: 1168 - DNA, 120 bp, Artificial Sequence
  PDGFRA
tttccactgctgtggatcatcagtgagtagacatgggtttaactgtctccctccttccttgcagacctttctgcccgtgaagtggatggctcctgagagcatctttgacaacctctacac

SEQ ID NO: 1169 - DNA, 120 bp, Artificial Sequence
  PDGFRA
gcagacctttctgcccgtgaagtggatggctcctgagagcatctttgacaacctctacaccacactgagtgatgtctggtcttatggcattctgctctgggagatcttttcccttggtat

SEQ ID NO: 1170 - DNA, 120 bp, Artificial Sequence
  PDGFRA
cacactgagtgatgtctggtcttatggcattctgctctgggagatcttttcccttggtatgggcctgacattgctgcttatttgggctgttctgaaacaccactggaaggaaaatgtgtt

SEQ ID NO: 1171 - DNA, 120 bp, Artificial Sequence
  PDGFRA
agcgtttgttagtcctggtgttttattgtttggcttttaggtggcaccccttaccccggcatgatggtggattctactttctacaataagatcaagagtgggtaccggatggccaagcct

SEQ ID NO: 1172 - DNA, 120 bp, Artificial Sequence
  PDGFRA
atgatggtggattctactttctacaataagatcaagagtgggtaccggatggccaagcctgaccacgctaccagtgaagtgtgagctccttccccatcccgggggcctgtgttcacagtc

SEQ ID NO: 1173 - DNA, 120 bp, Artificial Sequence
  PDGFRA
gggtctagggggagggaggggccctgagacttccccctgtgcccactcttgagttctgtccccacagctacgagatcatggtgaaatgctggaacagtgagccggagaagagaccctcct

SEQ ID NO: 1174 - DNA, 120 bp, Artificial Sequence
  PDGFRA
cccacagctacgagatcatggtgaaatgctggaacagtgagccggagaagagaccctccttttaccacctgagtgagattgtggagaatctgctgcctggacaatataaaaaggtgtgtt

SEQ ID NO: 1175 - DNA, 120 bp, Artificial Sequence
  PDGFRA
tttaccacctgagtgagattgtggagaatctgctgcctggacaatataaaaaggtgtgtttggatctgtgggtggaaaggtctggataaagctggaagttataccagtgagctgtgctgt

SEQ ID NO: 1176 - DNA, 120 bp, Artificial Sequence
  PDGFRA
gattaaatatgttcaatgaatgtttatagagttatgaaaaaattcacctggacttcctgaagagtgaccatcctgctgtggcacgcatgcgtgtggactcagacaatgcatacattggtg

SEQ ID NO: 1177 - DNA, 120 bp, Artificial Sequence
  PDGFRA
agagtgaccatcctgctgtggcacgcatgcgtgtggactcagacaatgcatacattggtgtcacctacaaaaacgaggaagacaagctgaaggactgggagggtggtctggatgagcaga

SEQ ID NO: 1178 - DNA, 120 bp, Artificial Sequence
  PDGFRA
tcacctacaaaaacgaggaagacaagctgaaggactgggagggtggtctggatgagcagagactgagcgctgacagtggctacatcattcctctgcctgacattgaccctgtccctgagg

SEQ ID NO: 1179 - DNA, 120 bp, Artificial Sequence
  PDGFRA
gactgagcgctgacagtggctacatcattcctctgcctgacattgaccctgtccctgaggaggaggacctgggcaagaggaacagacacaggtagctgtgggggcagcctcggtgtctca

SEQ ID NO: 1180 - DNA, 120 bp, Artificial Sequence
  PDGFRA
gttctgtgcaggagttgtaatatttgctcttctctccctcctccagctcgcagacctctgaagagagtgccattgagacgggttccagcagttccaccttcatcaagagagaggacgaga

SEQ ID NO: 1181 - DNA, 120 bp, Artificial Sequence
  PDGFRA
aagagagtgccattgagacgggttccagcagttccaccttcatcaagagagaggacgagaccattgaagacatcgacatgatggatgacatcggcatagactcttcagacctggtggaag

SEQ ID NO: 1182 - DNA, 120 bp, Artificial Sequence
  PDGFRA
ccattgaagacatcgacatgatggatgacatcggcatagactcttcagacctggtggaagacagcttcctgtaactggcggattcgaggggttccttccacttctggggccacctctgga

SEQ ID NO: 1183 - DNA, 120 bp, Artificial Sequence; identical to SEQ ID NO: 1145
  PDGFRA-E12

SEQ ID NO: 1184 - DNA, 120 bp, Artificial Sequence
  PDGFRA-E12
tcaccagttacctgtcctggtcatttatagaaaccgaggtatgaaattcgctggagggtcattgaatcaatcagcccagatggacatgaatatatttatgtggacccgatgcagctgcct

SEQ ID NO: 1185 - DNA, 120 bp, Artificial Sequence
  PDGFRA-E12
agcccagatggacatgaatatatttatgtggacccgatgcagctgccttatgactcaagatgggagtttccaagagatggactagtgcttggtaagttccatggggtaacctcccaagac

SEQ ID NO: 1186 - DNA, 120 bp, Artificial Sequence; identical to SEQ ID NO: 1147
  PDGFRA-E12

SEQ ID NO: 1187 - DNA, 120 bp, Artificial Sequence
  PDGFRA-E14
aatgatatccaatcacaggattagtcatattcttggtttttttctgagaacaggaagttggtagctcagctggactgatatgtgatttattctttcaacagccacggccagatccagtga

SEQ ID NO: 1188 - DNA, 120 bp, Artificial Sequence
  PDGFRA-E14
tcatattcttggtttttttctgagaacaggaagttggtagctcagctggactgatatgtgatttattctttcaacagccacggccagatccagtgaaaaacaagctctcatgtctgaact

SEQ ID NO: 1189 - DNA, 120 bp, Artificial Sequence
  PDGFRA-E14
aacaggaagttggtagctcagctggactgatatgtgatttattctttcaacagccacggccagatccagtgaaaaacaagctctcatgtctgaactgaagataatgactcacctggggcc

SEQ ID NO: 1190 - DNA, 120 bp, Artificial Sequence
  PDGFRA-E14
gactgatatgtgatttattctttcaacagccacggccagatccagtgaaaaacaagctctcatgtctgaactgaagataatgactcacctggggccacatttgaacattgtaaacttgct

SEQ ID NO: 1191 - DNA, 120 bp, Artificial Sequence
  PDGFRA-E14
aaaacaagctctcatgtctgaactgaagataatgactcacctggggccacatttgaacattgtaaacttgctgggagcctgcaccaagtcaggtgggctcactgacctggagtgaggatt

SEQ ID NO: 1192 - DNA, 120 bp, Artificial Sequence
  PDGFRA-E14
gaagataatgactcacctggggccacatttgaacattgtaaacttgctgggagcctgcaccaagtcaggtgggctcactgacctggagtgaggattttcactggacacatgtggttgtga

SEQ ID NO: 1193 - DNA, 120 bp, Artificial Sequence
  PDGFRA-E14
acatttgaacattgtaaacttgctgggagcctgcaccaagtcaggtgggctcactgacctggagtgaggattttcactggacacatgtggttgtgaaaactgttcaatcaggcttaaatc

SEQ ID NO: 1194 - DNA, 120 bp, Artificial Sequence
  PDGFRA-E14
gggagcctgcaccaagtcaggtgggctcactgacctggagtgaggattttcactggacacatgtggttgtgaaaactgttcaatcaggcttaaatcctccactctccatccccacacatg

SEQ ID NO: 1195 - DNA, 120 bp, Artificial Sequence; identical to SEQ ID NO: 1165
  PDGFRA-E18

SEQ ID NO: 1196 - DNA, 120 bp, Artificial Sequence
  PDGFRA-E18
cttgatcctgagtcatttcttccttttccatgcagtgtgtccaccgtgatctggctgctcgcaacgtcctcctggcacaaggaaaaattgtgaagatctgtgactttggcctggccagag

SEQ ID NO: 1197 - DNA, 120 bp, Artificial Sequence
  PDGFRA-E18
tggcacaaggaaaaattgtgaagatctgtgactttggcctggccagagacatcatgcatgattcgaactatgtgtcgaaaggcagtgtacgtcctcacttccctcactggtcaggctcat

SEQ ID NO: 1198 - DNA, 120 bp, Artificial Sequence; identical to SEQ ID NO: 1167
  PDGFRA-E18

SEQ ID NO: 1199 - DNA, 120 bp, Artificial Sequence
  TP53
gagagatgggggtgggaggctgtcagtggggaacaagaagtggagaatgtcagtctgagtcaggcccttctgtcttgaacatgagttttttatggcgggaggtagactgaccctttttgg

SEQ ID NO: 1200 - DNA, 120 bp, Artificial Sequence
  TP53
caggcccttctgtcttgaacatgagttttttatggcgggaggtagactgaccctttttggacttcaggtggctgtaggagacagaagcagggaggagagatgacatcacatgagtgagag

SEQ ID NO: 1201 - DNA, 120 bp, Artificial Sequence
  TP53
gatgagaatggaatcctatggctttccaacctaggaaggcaggggagtagggccaggaaggggctgaggtcactcacctggagtgagccctgctcccccctggctccttcccagcctggg

SEQ ID NO: 1202 - DNA, 120 bp, Artificial Sequence
  TP53
gggctgaggtcactcacctggagtgagccctgctcccccctggctccttcccagcctgggcatccttgagttccaaggcctcattcagctctcggaacatctcgaagcgctcacgcccac

SEQ ID NO: 1203 - DNA, 120 bp, Artificial Sequence
  TP53
catccttgagttccaaggcctcattcagctctcggaacatctcgaagcgctcacgcccacggatctgcagcaacagaggagggggagaagtaagtatatacacagtacctgagttaaaag

SEQ ID NO: 1204 - DNA, 120 bp, Artificial Sequence
  TP53
gtaagtcaagtagcatctgtatcaggcaaagtcatagaaccattttcatgctctctttaacaattttctttttgaaagctggtctggtcctttaaaatatatattatggtataagttggt

SEQ ID NO: 1205 - DNA, 120 bp, Artificial Sequence
  TP53
caattttctttttgaaagctggtctggtcctttaaaatatatattatggtataagttggtgttctgaagttagttagctacaaccaggagccattgtctttgaggcatcactgccccctg

SEQ ID NO: 1206 - DNA, 120 bp, Artificial Sequence; identical to SEQ ID NO: 1204
  TP53

SEQ ID NO: 1207 - DNA, 120 bp, Artificial Sequence; identical to SEQ ID NO: 1205
  TP53

SEQ ID NO: 1208 - DNA, 120 bp, Artificial Sequence
  TP53
tgagtgttagactggaaactttccacttgataagaggtcccaagacttagtacctgaagggtgaaatattctccatccagtggtttcttctttggctggggagaggagctggtgttgttg

SEQ ID NO: 1209 - DNA, 120 bp, Artificial Sequence
  TP53
gtgaaatattctccatccagtggtttcttctttggctggggagaggagctggtgttgttgggcagtgctaggaaagaggcaaggaaaggtgataaaagtgaatctgaggcataactgcac

SEQ ID NO: 1210 - DNA, 120 bp, Artificial Sequence
  TP53
ggcataactgcacccttggtctcctccaccgcttcttgtcctgcttgcttacctcgcttagtgctccctgggggcagctcgtggtgaggctcccctttcttgcggagattctcttcctct

SEQ ID NO: 1211 - DNA, 120 bp, Artificial Sequence
  TP53
gtgctccctgggggcagctcgtggtgaggctcccctttcttgcggagattctcttcctctgtgcgccggtctctcccaggacaggcacaaacacgcacctcaaagctgttccgtcccagt

SEQ ID NO: 1212 - DNA, 120 bp, Artificial Sequence
  TP53
gtgcgccggtctctcccaggacaggcacaaacacgcacctcaaagctgttccgtcccagtagattaccactactcaggataggaaaagagaagcaagaggcagtaaggaaatcaggtcct

SEQ ID NO: 1213 - DNA, 120 bp, Artificial Sequence
  TP53
ggtcagaggcaagcagaggctggggcacagcaggccagtgtgcagggtggcaagtggctcctgacctggagtcttccagtgtgatgatggtgaggatgggcctccggttcatgccgccca

SEQ ID NO: 1214 - DNA, 120 bp, Artificial Sequence
  TP53
ctgacctggagtcttccagtgtgatgatggtgaggatgggcctccggttcatgccgcccatgcaggaactgttacacatgtagttgtagtggatggtggtacagtcagagccaacctagg

SEQ ID NO: 1215 - DNA, 120 bp, Artificial Sequence
  TP53
tgcaggaactgttacacatgtagttgtagtggatggtggtacagtcagagccaacctaggagataacacaggcccaagatgaggccagtgcgccttggggagacctgtggcaagcagggg

SEQ ID NO: 1216 - DNA, 120 bp, Artificial Sequence
  TP53
cctggagggccactgacaaccacccttaacccctcctcccagagaccccagttgcaaaccagacctcaggcggctcatagggcaccaccacactatgtcgaaaagtgtttctgtcatcca

SEQ ID NO: 1217 - DNA, 120 bp, Artificial Sequence
  TP53
agacctcaggcggctcatagggcaccaccacactatgtcgaaaagtgtttctgtcatccaaatactccacacgcaaatttccttccactcggataagatgctgaggaggggccagaccta

SEQ ID NO: 1218 - DNA, 120 bp, Artificial Sequence
  TP53
aatactccacacgcaaatttccttccactcggataagatgctgaggaggggccagacctaagagcaatcagtgaggaatcagaggcctggggaccctgggcaaccagccctgtcgtctct

SEQ ID NO: 1219 - DNA, 120 bp, Artificial Sequence
  TP53
tgtcgtctctccagccccagctgctcaccatcgctatctgagcagcgctcatggtgggggcagcgcctcacaacctccgtcatgtgctgtgactgcttgtagatggccatggcgcggacg

SEQ ID NO: 1220 - DNA, 120 bp, Artificial Sequence
  TP53
cagcgcctcacaacctccgtcatgtgctgtgactgcttgtagatggccatggcgcggacgcgggtgccgggcgggggtgtggaatcaacccacagctgcacagggcaggtcttggccagt

SEQ ID NO: 1221 - DNA, 120 bp, Artificial Sequence
  TP53
cgggtgccgggcgggggtgtggaatcaacccacagctgcacagggcaggtcttggccagttggcaaaacatcttgttgagggcaggggagtactgtaggaagaggaaggagacagagttg

SEQ ID NO: 1222 - DNA, 120 bp, Artificial Sequence
  TP53
gggcaactgaccgtgcaagtcacagacttggctgtcccagaatgcaagaagcccagacggaaaccgtagctgccctggtaggttttctgggaagggacagaagatgacaggggccaggag

SEQ ID NO: 1223 - DNA, 120 bp, Artificial Sequence; identical to SEQ ID NO: 1222
  TP53

SEQ ID NO: 1224 - DNA, 120 bp, Artificial Sequence
  TP53
ggggctggtgcaggggccgccggtgtaggagctgctggtgcaggggccacggggggagcagcctctggcattctgggagcttcatctggacctgggtcttcagtgaaccattgttcaata

SEQ ID NO: 1225 - DNA, 120 bp, Artificial Sequence
  TP53
gcctctggcattctgggagcttcatctggacctgggtcttcagtgaaccattgttcaatatcgtccggggacagcatcaaatcatccattgcttgggacggcaagggggactgtagatgg

SEQ ID NO: 1226 - DNA, 120 bp, Artificial Sequence
  TP53
ccctccaggtccccagcccaacccttgtccttaccagaacgttgttttcaggaagtctgaaagacaagagcagaaagtcagtcccatggaattttcgcttcccacaggtctctgctaggg

SEQ ID NO: 1227 - DNA, 120 bp, Artificial Sequence
  TP53
aagacaagagcagaaagtcagtcccatggaattttcgcttcccacaggtctctgctagggggctggggttggggtgggggtggtgggcctgcccttccaatggatccactcacagtttcc

SEQ ID NO: 1228 - DNA, 120 bp, Artificial Sequence
  TP53
ggctggggttggggtgggggtggtgggcctgcccttccaatggatccactcacagtttccataggtctgaaaatgtttcctgactcagagggggctcgacgctaggatctgactgcggct

SEQ ID NO: 1229 - DNA, 120 bp, Artificial Sequence
  TP53
ataggtctgaaaatgtttcctgactcagagggggctcgacgctaggatctgactgcggctcctccatggcagtgacccggaaggcagtctggctgctgcaagaggaaaagtggggatcca